European Patent Application EP 4 389 762 A1, published June 26, 2024. Title: PEPTIDES AND USES THEREOF. Applicant: Ospedale San Raffaele S.r.l. The sequence listing filed with the application follows.

SEQUENCE LISTING (129 sequences)

SEQ ID NO: 1 - protein, 288 aa, Homo sapiens
MSKSFQQSSLSRDSQGHGRDLSAAGIGLLAAATQSLSMPASLGRMNQGTARLASLMNLGMSSSLNQQGAHSALSSASTSSHNLQSIFNIGSRGPLPLSSQHRGDADQASNILASFGLSARDLDELSRYPEDKITPENLPQILLQLKRRRTEEGPTLSYGRDGRSATREPPYRVPRDDWEEKRHFRRDSFDDRGPSLNPVLDYDHGSRSQESGYYDRMDYEDDRLRDGERCRDDSFFGETSHNYHKFDSEYERMGRGPGPLQERSLFEKKRGAPPSSNIEDFHGLLPKG

SEQ ID NO: 2 - protein, 60 aa, synthetic construct
RTEEGPTLSYGRDGRSATREPPYRVPRDDWEEKRHFRRDSFDDRGPSLNPVLDYDHGSRS

SEQ ID NO: 3 - protein, 61 aa, synthetic construct
SFDDRGPSLNPVLDYDHGSRSQESGYYDRMDYEDDRLRDGERCRDDSFFGETSHNYHKFDS

SEQ ID NO: 4 - protein, 60 aa, synthetic construct
ERCRDDSFFGETSHNYHKFDSEYERMGRGPGPLQERSLFEKKRGAPPSSNIEDFHGLLPK

SEQ ID NO: 5 - protein, 46 aa, synthetic construct
ESGYYDRMDYEDDRLRDGERCRDDSFFGETSHNYHKFDSEYERMGR

SEQ ID NO: 6 - protein, 101 aa, synthetic construct
SFDDRGPSLNPVLDYDHGSRSQESGYYDRMDYEDDRLRDGERCRDDSFFGETSHNYHKFDSEYERMGRGPGPLQERSLFEKKRGAPPSSNIEDFHGLLPKG

SEQ ID NO: 7 - protein, 80 aa, synthetic construct
QESGYYDRMDYEDDRLRDGERCRDDSFFGETSHNYHKFDSEYERMGRGPGPLQERSLFEKKRGAPPSSNIEDFHGLLPKG

SEQ ID NO: 8 - protein, 79 aa, synthetic construct
ESGYYDRMDYEDDRLRDGERCRDDSFFGETSHNYHKFDSEYERMGRGPGPLQERSLFEKKRGAPPSSNIEDFHGLLPKG

SEQ ID NO: 9 - protein, 609 aa, synthetic construct [sequence omitted]

SEQ ID NO: 10 - protein, 585 aa, synthetic construct [sequence omitted]

SEQ ID NO: 11 - protein, 137 aa, synthetic construct
EEGPTLSYGRDGRSATREPPYRVPRDDWEEKRHFRRDSFDDRGPSLNPVLDYDHGSRSQESGYYDRMDYEDDRLRDGERCRDDSFFGETSHNYHKFDSEYERMGRGPGPLQERSLFEKKRGAPPSSNIEDFHGLLPK

SEQ ID NO: 12 - protein, 79 aa, synthetic construct
QESGYYDRMDYEDDRLRDGERCRDDSFFGETSHNYHKFDSEYERMGRGPGPLQERSLFEKKRGAPPSSNIEDFHGLLPK

SEQ ID NO: 13 - protein, 78 aa, synthetic construct
ESGYYDRMDYEDDRLRDGERCRDDSFFGETSHNYHKFDSEYERMGRGPGPLQERSLFEKKRGAPPSSNIEDFHGLLPK

SEQ ID NO: 14 - protein, 100 aa, synthetic construct
SFDDRGPSLNPVLDYDHGSRSQESGYYDRMDYEDDRLRDGERCRDDSFFGETSHNYHKFDSEYERMGRGPGPLQERSLFEKKRGAPPSSNIEDFHGLLPK

SEQ ID NO: 15 - protein, 139 aa, synthetic construct
RTEEGPTLSYGRDGRSATREPPYRVPRDDWEEKRHFRRDSFDDRGPSLNPVLDYDHGSRSQESGYYDRMDYEDDRLRDGERCRDDSFFGETSHNYHKFDSEYERMGRGPGPLQERSLFEKKRGAPPSSNIEDFHGLLPK

SEQ ID NO: 16 - protein, 138 aa, synthetic construct
EEGPTLSYGRDGRSATREPPYRVPRDDWEEKRHFRRDSFDDRGPSLNPVLDYDHGSRSQESGYYDRMDYEDDRLRDGERCRDDSFFGETSHNYHKFDSEYERMGRGPGPLQERSLFEKKRGAPPSSNIEDFHGLLPKG

SEQ ID NO: 17 - protein, 287 aa, synthetic construct
MSKSFQQSSLSRDSQGHGRDLSAAGIGLLAAATQSLSMPASLGRMNQGTARLASLMNLGMSSSLNQQGAHSALSSASTSSHNLQSIFNIGSRGPLPLSSQHRGDADQASNILASFGLSARDLDELSRYPEDKITPENLPQILLQLKRRRTEEGPTLSYGRDGRSATREPPYRVPRDDWEEKRHFRRDSFDDRGPSLNPVLDYDHGSRSQESGYYDRMDYEDDRLRDGERCRDDSFFGETSHNYHKFDSEYERMGRGPGPLQERSLFEKKRGAPPSSNIEDFHGLLPK

SEQ ID NO: 18 - protein, 287 aa, synthetic construct
SKSFQQSSLSRDSQGHGRDLSAAGIGLLAAATQSLSMPASLGRMNQGTARLASLMNLGMSSSLNQQGAHSALSSASTSSHNLQSIFNIGSRGPLPLSSQHRGDADQASNILASFGLSARDLDELSRYPEDKITPENLPQILLQLKRRRTEEGPTLSYGRDGRSATREPPYRVPRDDWEEKRHFRRDSFDDRGPSLNPVLDYDHGSRSQESGYYDRMDYEDDRLRDGERCRDDSFFGETSHNYHKFDSEYERMGRGPGPLQERSLFEKKRGAPPSSNIEDFHGLLPKG

SEQ ID NO: 19 - protein, 286 aa, synthetic construct
SKSFQQSSLSRDSQGHGRDLSAAGIGLLAAATQSLSMPASLGRMNQGTARLASLMNLGMSSSLNQQGAHSALSSASTSSHNLQSIFNIGSRGPLPLSSQHRGDADQASNILASFGLSARDLDELSRYPEDKITPENLPQILLQLKRRRTEEGPTLSYGRDGRSATREPPYRVPRDDWEEKRHFRRDSFDDRGPSLNPVLDYDHGSRSQESGYYDRMDYEDDRLRDGERCRDDSFFGETSHNYHKFDSEYERMGRGPGPLQERSLFEKKRGAPPSSNIEDFHGLLPK

SEQ ID NO: 20 - protein, 5 aa, synthetic construct
GPPGS

SEQ ID NO: 21 - protein, 5 aa, synthetic construct
GGGGS

SEQ ID NO: 22 - protein, 4 aa, synthetic construct
GGGS

SEQ ID NO: 23 - DNA, 21 bp, synthetic construct
  source 1..21: mol_type = other DNA
tcaagaaggtggtgaagcagg

SEQ ID NO: 24 - protein, 5 aa, synthetic construct
SGGGG

SEQ ID NO: 25 - protein, 4 aa, synthetic construct
SGGG

SEQ ID NO: 26 - DNA, 22 bp, synthetic construct
  source 1..22: mol_type = other DNA
accaggaaatgagcttgacaaa

SEQ ID NO: 27 - DNA, 26 bp, synthetic construct
  source 1..26: mol_type = other DNA
gcccgccagaataacggcgaaagcgg

SEQ ID NO: 28 - DNA, 26 bp, synthetic construct
  source 1..26: mol_type = other DNA
ccgctttcgccgttattctggcgggc

SEQ ID NO: 29 - protein, 5 aa, synthetic construct
GGGGA

SEQ ID NO: 30 - protein, 321 aa, synthetic construct
SKSFQQSSLSRDSQGHGRDLSAAGIGLLAAATQSLSMPASLGRMNQGTARLASLMNLGMSSSLNQQGAHSALSSASTSSHNLQSIFNIGSRGPLPLSSQHRGDADQASNILASFGLSARDLDELSRYPEDKITPENLPQILLQLKRRRTEEGPTLSYGRDGRSATREPPYRVPRDDWEEKRHFRRDSFDDRGPSLNPVLDYDHGSRSQESGYYDRMDYEDDRLRDGERCRDDSFFGETSHNYHKFDSEYERMGRGPGPLQERSLFEKKRGAPPSSNIEDFHGLLPKGYPHLCSICDLPVHSNKEWSQHINGASHSRRCQLL

SEQ ID NO: 31 - protein, 797 aa, synthetic construct
SKSFQQSSLSRDSQGHGRDLSAAGIGLLAAATQSLSMPASLGRMNQGTARLASLMNLGMSSSLNQQGAHSALSSASTSSHNLQSIFNIGSRGPLPLSSQHRGDADQASNILASFGLSARDLDELSRYPEDKITPENLPQILLQLKRRRTEEGPTLSYGRDGRSATREPPYRVPRDDWEEKRHFRRDSFDDRGPSLNPVLDYDHGSRSQESGYYDRMDYEDDRLRDGERCRDDSFFGETSHNYHKFDSEYERMGRGPGPLQERSLFEKKRGAPPSSNIEDFHGLLPKGYPHLCSICDLPVHSNKEWSQHINGASHSRRCQLLLEIYPEWNPDNDTGHTMGDPFMLQQSTNPAPGILGPPPPSFHLGGPAVGPRGNLGAGNGNLQGPRHMQKGRVETSRVVHIMDFQRGKNLRYQLLQLVEPFGVISNHLILNKINEAFIEMATTEDAQAAVDYYTTTPALVFGKPVRVHLSQKYKRIKKPEGKPDQKFDQKQELGRVIHLSNLPHSGYSDSAVLKLAEPYGKIKNYILMRMKSQAFIEMETREDAMAMVDHCLKKALWFQGRCVKVDLSEKYKKLVLRIPNRGIDLLKKDKSRKRSYSPDGKESPSDKKSKTDGSQKTESSTEGKEQEEKSGEDGEKDTKDDQTEQEPNMLLESEDELLVDEEEAAALLESGSSVGDETDLANLGDVASDGKKEPSDKAVKKDGSASAAAKKKLKKVDKIEELDQENEAALENGIKNEENTEPGAESSENADDPNKDTSENADGQSDENKDDYTIPDEYRIGPYQPNVPVGIDYVIPK

SEQ ID NO: 32 - protein, 23 aa, synthetic construct
GGSSEAAEAAEAAEAAEAAEAAE

SEQ ID NO: 33 - DNA, 6163 bp, synthetic construct
  source 1..6163: mol_type = other DNA
gacggatcgggagatctcccgatcccctatggtgcactctcagtacaatctgctctgatgccgcatagttaagccagtatctgctccctgcttgtgtgttggaggtcgctgagtagtgcgcgagcaaaatttaagctacaacaaggcaaggcttgaccgacaattgcatgaagaatctgcttagggttaggcgttttgcgctgcttcgcgatgtacgggccagatatacgcgttgacattgattattgactagttattaatagtaatcaattacggggtcattagttcatagcccatatatggagttccgcgttacataacttacggtaaatggcccgcctggctgaccgcccaacgacccccgcccattgacgtcaataatgacgtatgttcccatagtaacgccaatagggactttccattgacgtcaatgggtggagtatttacggtaaactgcccacttggcagtacatcaagtgtatcatatgccaagtacgccccctattgacgtcaatgacggtaaatggcccgcctggcattatgcccagtacatgaccttatgggactttcctacttggcagtacatctacgtattagtcatcgctattaccatggtgatgcggttttggcagtacatcaatgggcgtggatagcggtttgactcacggggatttccaagtctccaccccattgacgtcaatgggagtttgttttggcaccaaaatcaacgggactttccaaaatgtcgtaacaactccgccccattgacgcaaatgggcggtaggcgtgtacggtgggaggtctatataagcagagctctccctatcagtgatagagatctccctatcagtgatagagatcgtcgacgagctcgtttagtgaaccgtcagatcgcctggagacgccatccacgctgttttgacctccatagaagacaccgggaccgatccagcctccggactctagcgtttaaacttaagcttggtaccgagctcggatccactagtccagtgtggtggaattctgcagatatcacaagtttgtacaaaaaagcaggctccatggattacaaggatgacgacgataagagcccgggcggatcctccaagtcattccagcagtcatctctcagtagggactcacagggtcatgggcgtgacctgtctgcggcaggaataggccttcttgctgctgctacccagtctttaagtatgccagcatctcttggaaggatgaaccagggtactgcacgccttgctagtttaatgaatcttggaatgagttcttcattgaatcaacaaggagctcatagtgcactgtcttctgctagtacttcttcccataatttgcagtctatatttaacattggaagtagaggtccactccctttatcttctcaacaccgtggagatgcagaccaggccagtaacattttggccagctttggtctgtctgctagagacttagatgaactgagtcgttatccagaggacaagattactcctgagaatttgccccaaatccttctacagcttaaaaggaggagaactgaagaaggccctaccttgagttatggtagagatggcagatctgctacacgggagccaccatacagagtacctagggatgattgggaagaaaaaaggcactttagaagagatagttttgatgatcgtggtcctagtctcaacccagtgcttgattatgaccatggaagtcgttctcaagaatctggttattatgacagaatggattatgaagatgacagattaagagatggagaaaggtgtagggatgattctttttttggtgagacctcgcataactatcataaatttgacagtgagtatgagagaatgggacgtggtcctggccccttacaagagagatctctctttgagaaaaagagaggcgctcctccaagtagcaatattgaagacttccatggactcttaccgaagggtagggatcccaagaaaaaacgcaaggtggaagatcctaagaaaaagcggaaagtggaagacccaaaaaagaagagaaaggtagactgagacccagctttcttgtacaaagtggtgacgtaagctaggggcccgtttaaacccgctgatcagcctcgactgtgccttctagttgccagccatctgttgtttgcccctcccccgtgccttccttgaccctggaaggtgccactcccactgtcctttcctaataaaatgaggaaattgcatcgcattgtctgagtaggtgtcattctattctggggggtggggtggggcaggacagcaagggggaggattgggaagacaatagcaggcatgctggggatgcggtgggctctatggcttctgaggcggaaagaaccagctggggctctagggggtatccccacgcgccctgtagcggcgcattaagcgcggcgggtgtggtggttacgcgcagcgtgaccgctacacttgccagcgccctagcgcccgctcctttcgctttcttcccttcctttctcgccacgttcgccggctttccccgtcaagctctaaatcgggggctccctttagggttccgatttagtgctttacggcacctcgaccccaaaaaacttgattagggtgatggttcacgtacctagaagttcctattccgaagttcctattctctagaaagtataggaacttccttggccaaaaagcctgaactcaccgcgacgtctgtcgagaagtttctgatcgaaaagttcgacagcgtctccgacctgatgcagctctcggagggcgaagaatctcgtgctttcagcttcgatgtaggagggcgtggatatgtcctgcgggtaaatagctgcgccgatggtttctacaaagatcgttatgtttatcggcactttgcatcggccgcgctcccgattccggaagtgcttgacattggggaattcagcgagagcctgacctattgcatctcccgccgtgcacagggtgtcacgttgcaagacctgcctgaaaccgaactgcccgctgttctgcagccggtcgcggaggccatggatgcgatcgctgcggccgatcttagccagacgagcgggttcggcccattcggaccgcaaggaatcggtcaatacactacatggcgtgatttcatatgcgcgattgctgatccccatgtgtatcactggcaaactgtgatggacgacaccgtcagtgcgtccgtcgcgcaggctctcgatgagctgatgctttgggccgaggactgccccgaagtccggcacctcgtgcacgcggatttcggctccaacaatgtcctgacggacaatggccgcataacagcggtcattgactggagcgaggcgatgttcggggattcccaatacgaggtcgccaacatcttcttctggaggccgtggttggcttgtatggagcagcagacgcgctacttcgagcggaggcatccggagcttgcaggatcgccgcggctccgggcgtatatgctccgcattggtcttgaccaactctatcagagcttggttgacggcaatttcgatgatgcagcttgggcgcagggtcgatgcgacgcaatcgtccgatccggagccgggactgtcgggcgtacacaaatcgcccgcagaagcgcggccgtctggaccgatggctgtgtagaagtactcgccgatagtggaaaccgacgccccagcactcgtccgagggcaaaggaatagcacgtactacgagatttcgattccaccgccgccttctatgaaaggttgggcttcggaatcgttttccgggacgccggctggatgatcctccagcgcggggatctcatgctggagttcttcgcccaccccaacttgtttattgcagcttataatggttacaaataaagcaatagcatcacaaatttcacaaataaagcatttttttcactgcattctagttgtggtttgtccaaactcatcaatgtatcttatcatgtctgtataccgtcgacctctagctagagcttggcgtaatcatggtcatagctgtttcctgtgtgaaattgttatccgctcacaattccacacaacatacgagccggaagcataaagtgtaaagcctggggtgcctaatgagtgagctaactcacattaattgcgttgcgctcactgcccgctttccagtcgggaaacctgtcgtgccagctgcattaatgaatcggccaacgcgcggggagaggcggtttgcgtattgggcgctcttccgcttcctcgctcactgactcgctgcgctcggtcgttcggctgcggcgagcggtatcagctcactcaaaggcggtaatacggttatccacagaatcaggggataacgcaggaaagaacatgtgagcaaaaggccagcaaaaggccaggaaccgtaaaaaggccgcgttgctggcgtttttccataggctccgcccccctgacgagcatcacaaaaatcgacgctcaagtcagaggtggcgaaacccgacaggactataaagataccaggcgtttccccctggaagctccctcgtgcgctctcctgttccgaccctgccgcttaccggatacctgtccgcctttctcccttcgggaagcgtggcgctttctcatagctcacgctgtaggtatctcagttcggtgtaggtcgttcgctccaagctgggctgtgtgcacgaaccccccgttcagcccgaccgctgcgccttatccggtaactatcgtcttgagtccaacccggtaagacacgacttatcgccactggcagcagccactggtaacaggattagcagagcgaggtatgtaggcggtgctacagagttcttgaagtggtggcctaactacggctacactagaagaacagtatttggtatctgcgctctgctgaagccagttaccttcggaaaaagagttggtagctcttgatccggcaaacaaaccaccgctggtagcggtggtttttttgtttgcaagcagcagattacgcgcagaaaaaaaggatctcaagaagatcctttgatcttttctacggggtctgacgctcagtggaacgaaaactcacgttaagggattttggtcatgagattatcaaaaaggatcttcacctagatccttttaaattaaaaatgaagttttaaatcaatctaaagtatatatgagtaaacttggtctgacagttaccaatgcttaatcagtgaggcacctatctcagcgatctgtctatttcgttcatccatagttgcctgactccccgtcgtgtagataactacgatacgggagggcttaccatctggccccagtgctgcaatgataccgcgagacccacgctcaccggctccagatttatcagcaataaaccagccagccggaagggccgagcgcagaagtggtcctgcaactttatccgcctccatccagtctattaattgttgccgggaagctagagtaagtagttcgccagttaatagtttgcgcaacgttgttgccattgctacaggcatcgtggtgtcacgctcgtcgtttggtatggcttcattcagctccggttcccaacgatcaaggcgagttacatgatcccccatgttgtgcaaaaaagcggttagctccttcggtcctccgatcgttgtcagaagtaagttggccgcagtgttatcactcatggttatggcagcactgcataattctcttactgtcatgccatccgtaagatgcttttctgtgactggtgagtactcaaccaagtcattctgagaatagtgtatgcggcgaccgagttgctcttgcccggcgtcaatacgggataataccgcgccacatagcagaactttaaaagtgctcatcattggaaaacgttcttcggggcgaaaactctcaaggatcttaccgctgttgagatccagttcgatgtaacccactcgtgcacccaactgatcttcagcatcttttactttcaccagcgtttctgggtgagcaaaaacaggaaggcaaaatgccgcaaaaaagggaataagggcgacacggaaatgttgaatactcatactcttcctttttcaatattattgaagcatttatcagggttattgtctcatgagcggatacatatttgaatgtatttagaaaaataaacaaataggggttccgcgcacatttccccgaaaagtgccacctgacgtc

SEQ ID NO: 34 - protein, 329 aa, synthetic construct
MDYKDDDDKSPGGSSKSFQQSSLSRDSQGHGRDLSAAGIGLLAAATQSLSMPASLGRMNQGTARLASLMNLGMSSSLNQQGAHSALSSASTSSHNLQSIFNIGSRGPLPLSSQHRGDADQASNILASFGLSARDLDELSRYPEDKITPENLPQILLQLKRRRTEEGPTLSYGRDGRSATREPPYRVPRDDWEEKRHFRRDSFDDRGPSLNPVLDYDHGSRSQESGYYDRMDYEDDRLRDGERCRDDSFFGETSHNYHKFDSEYERMGRGPGPLQERSLFEKKRGAPPSSNIEDFHGLLPKGRDPKKKRKVEDPKKKRKVEDPKKKRKVD

SEQ ID NO: 35 - DNA, 10910 bp, synthetic construct
  source 1..10910: mol_type = other DNA
gtcgacggatcgggagatctcccgatcccctatggtgcactctcagtacaatctgctctgatgccgcatagttaagccagtatctgctccctgcttgtgtgttggaggtcgctgagtagtgcgcgagcaaaatttaagctacaacaaggcaaggcttgaccgacaattgcatgaagaatctgcttagggttaggcgttttgcgctgcttcgcgatgtacgggccagatatacgcgttgacattgattattgactagttattaatagtaatcaattacggggtcattagttcatagcccatatatggagttccgcgttacataacttacggtaaatggcccgcctggctgaccgcccaacgacccccgcccattgacgtcaataatgacgtatgttcccatagtaacgccaatagggactttccattgacgtcaatgggtggagtatttacggtaaactgcccacttggcagtacatcaagtgtatcatatgccaagtacgccccctattgacgtcaatgacggtaaatggcccgcctggcattatgcccagtacatgaccttatgggactttcctacttggcagtacatctacgtattagtcatcgctattaccatggtgatgcggttttggcagtacatcaatgggcgtggatagcggtttgactcacggggatttccaagtctccaccccattgacgtcaatgggagtttgttttggcaccaaaatcaacgggactttccaaaatgtcgtaacaactccgccccattgacgcaaatgggcggtaggcgtgtacggtgggaggtctatataagcagcgcgttttgcctgtactgggtctctctggttagaccagatctgagcctgggagctctctggctaactagggaacccactgcttaagcctcaataaagcttgccttgagtgcttcaagtagtgtgtgcccgtctgttgtgtgactctggtaactagagatccctcagacccttttagtcagtgtggaaaatctctagcagtggcgcccgaacagggacttgaaagcgaaagggaaaccagaggagctctctcgacgcaggactcggcttgctgaagcgcgcacggcaagaggcgaggggcggcgactggtgagtacgccaaaaattttgactagcggaggctagaaggagagagatgggtgcgagagcgtcagtattaagcgggggagaattagatcgcgatgggaaaaaattcggttaaggccagggggaaagaaaaaatataaattaaaacatatagtatgggcaagcagggagctagaacgattcgcagttaatcctggcctgttagaaacatcagaaggctgtagacaaatactgggacagctacaaccatcccttcagacaggatcagaagaacttagatcattatataatacagtagcaaccctctattgtgtgcatcaaaggatagagataaaagacaccaaggaagctttagacaagatagaggaagagcaaaacaaaagtaagaccaccgcacagcaagcggccgctgatcttcagacctggaggaggagatatgagggacaattggagaagtgaattatataaatataaagtagtaaaaattgaaccattaggagtagcacccaccaaggcaaagagaagagtggtgcagagagaaaaaagagcagtgggaataggagctttgttccttgggttcttgggagcagcaggaagcactatgggcgcagcgtcaatgacgctgacggtacaggccagacaattattgtctggtatagtgcagcagcagaacaatttgctgagggctattgaggcgcaacagcatctgttgcaactcacagtctggggcatcaagcagctccaggcaagaatcctggctgtggaaagatacctaaaggatcaacagctcctggggatttggggttgctctggaaaactcatttgcaccactgctgtgccttggaatgctagttggagtaataaatctctggaacagatttggaatcacacgacctggatggagtgggacagagaaattaacaattacacaagcttaatacactccttaattgaagaatcgcaaaaccagcaagaaaagaatgaacaagaattattggaattagataaatgggcaagtttgtggaattggtttaacataacaaattggctgtggtatataaaattattcataatgatagtaggaggcttggtaggtttaagaatagtttttgctgtactttctatagtgaatagagttaggcagggatattcaccattatcgtttcagacccacctcccaaccccgaggggacccgacaggcccgaaggaatagaagaagaaggtggagagagagacagagacagatccattcgattagtgaacggatcggcactgcgtgcgccaattctgcagacaaatggcagtattcatccacaattttaaaagaaaaggggggattggggggtacagtgcaggggaaagaatagtagacataatagcaacagacatacaaactaaagaattacaaaaacaaattacaaaaattcaaaattttcgggtttattacagggacagcagagatccagtttggttaattaacccgtgtcggctccagatctggcctccgcgccgggttttggcgcctcccgcgggcgcccccctcctcacggcgagcgctgccacgtcagacgaagggcgcagcgagcgtcctgatccttccgcccggacgctcaggacagcggcccgctgctcataagactcggccttagaaccccagtatcagcagaaggacattttaggacgggacttgggtgactctagggcactggttttctttccagagagcggaacaggcgaggaaaagtagtcccttctcggcgattctgcggagggatctccgtggggcggtgaacgccgatgattatataaggacgcgccgggtgtggcacagctagttccgtcgcagccgggatttgggtcgcggttcttgtttgtggatcgctgtgatcgtcacttggtgagtagcgggctgctgggctggccggggctttcgtggccgccgggccgctcggtgggacggaagcgtgtggagagaccgccaagggctgtagtctgggtccgcgagcaaggttgccctgaactgggggttggggggagcgcagcaaaatggcggctgttcccgagtcttgaatggaagacgcttgtgaggcgggctgtgaggtcgttgaaacaaggtggggggcatggtgggcggcaagaacccaaggtcttgaggccttcgctaatgcgggaaagctcttattcgggtgagatgggctggggcaccatctggggaccctgacgtgaagtttgtcactgactggagaactcggtttgtcgtctgttgcgggggcggcagttatggcggtgccgttgggcagtgcacccgtacctttgggagcgcgcgccctcgtcgtgtcgtgacgtcacccgttctgttggcttataatgcagggtggggccacctgccggtaggtgtgcggtaggcttttctccgtcgcaggacgcagggttcgggcctagggtaggctctcctgaatcgacaggcgccggacctctggtgaggggagggataagtgaggcgtcagtttctttggtcggttttatgtacctatcttcttaagtagctgaagctccggttttgaactatgcgctcggggttggcgagtgtgttttgtgaagttttttaggcaccttttgaaatgtaatcatttgggtcaatatgtaattttcagtgttagactagtaaattgtccgctaaattctggccgtttttggcttttttgttagacgaagcttgggctgcaggtcgactctagaggatccccgggtaccggtcgccaccatggtgagcaagggcgaggagctgttcaccggggtggtgcccatcctggtcgagctggacggcgacgtaaacggccacaagttcagcgtgtccggcgagggcgagggcgatgccacctacggcaagctgaccctgaagttcatctgcaccaccggcaagctgcccgtgccctggcccaccctcgtgaccaccctgacctacggcgtgcagtgcttcagccgctaccccgaccacatgaagcagcacgacttcttcaagtccgccatgcccgaaggctacgtccaggagcgcaccatcttcttcaaggacgacggcaactacaagacccgcgccgaggtgaagttcgagggcgacaccctggtgaaccgcatcgagctgaagggcatcgacttcaaggaggacggcaacatcctggggcacaagctggagtacaactacaacagccacaacgtctatatcatggccgacaagcagaagaacggcatcaaggtgaacttcaagatccgccacaacatcgaggacggcagcgtgcagctcgccgaccactaccagcagaacacccccatcggcgacggccccgtgctgctgcccgacaaccactacctgagcacccagtccgccctgagcaaagaccccaacgagaagcgcgatcacatggtcctgctggagttcgtgaccgccgccgggatcactctcggcatggacgagctgtactccaagtcattccagcagtcatctctcagtagggactcacagggtcatgggcgtgacctgtctgcggcaggaataggccttcttgctgctgctacccagtctttaagtatgccagcatctcttggaaggatgaaccagggtactgcacgccttgctagtttaatgaatcttggaatgagttcttcattgaatcaacaaggagctcatagtgcactgtcttctgctagtacttcttcccataatttgcagtctatatttaacattggaagtagaggtccactccctttatcttctcaacaccgtggagatgcagaccaggccagtaacattttggccagctttggtctgtctgctagagacttagatgaactgagtcgttatccagaggacaagattactcctgagaatttgccccaaatccttctacagcttaaaaggaggagaactgaagaaggccctaccttgagttatggtagagatggcagatctgctacacgggagccaccatacagagtacctagggatgattgggaagaaaaaaggcactttagaagagatagttttgatgatcgtggtcctagtctcaacccagtgcttgattatgaccatggaagtcgttctcaagaatctggttattatgacagaatggattatgaagatgacagattaagagatggagaaaggtgtagggatgattctttttttggtgagacctcgcataactatcataaatttgacagtgagtatgagagaatgggacgtggtcctggccccttacaagagagatctctctttgagaaaaagagaggcgctcctccaagtagcaatattgaagacttccatggactcttaccgaagggtagggatcccaagaaaaaacgcaaggtggaagatcctaagaaaaagcggaaagtggaagacccaaaaaagaagagaaaggtagactaatgtacaagtaagctagctcgagctagaattaattcgatatcaagcttatcgataatcaacctctggattacaaaatttgtgaaagattgactggtattcttaactatgttgctccttttacgctatgtggatacgctgctttaatgcctttgtatcatgctattgcttcccgtatggctttcattttctcctccttgtataaatcctggttgctgtctctttatgaggagttgtggcccgttgtcaggcaacgtggcgtggtgtgcactgtgtttgctgacgcaacccccactggttggggcattgccaccacctgtcagctcctttccgggactttcgctttccccctccctattgccacggcggaactcatcgccgcctgccttgcccgctgctggacaggggctcggctgttgggcactgacaattccgtggtgttgtcggggaaatcatcgtcctttccttggctgctcgcctgtgttgccacctggattctgcgcgggacgtccttctgctacgtcccttcggccctcaatccagcggaccttccttcccgcggcctgctgccggctctgcggcctcttccgcgtcttcgccttcgccctcagacgagtcggatctccctttgggccgcctccccgcatcgataccgtcgacctcgagacctagaaaaacatggagcaatcacaagtagcaatacagcagctaccaatgctgattgtgcctggctagaagcacaagaggaggaggaggtgggttttccagtcacacctcaggtacctttaagaccaatgacttacaaggcagctgtagatcttagccactttttaaaagaaaaggggggactggaagggctaattcactcccaacgaagacaagatatccttgatctgtggatctaccacacacaaggctacttccctgattggcagaactacacaccagggccagggatcagatatccactgacctttggatggtgctacaagctagtaccagttgagcaagagaaggtagaagaagccaatgaaggagagaacacccgcttgttacaccctgtgagcctgcatgggatggatgacccggagagagaagtattagagtggaggtttgacagccgcctagcatttcatcacatggcccgagagctgcatccggactgtactgggtctctctggttagaccagatctgagcctgggagctctctggctaactagggaacccactgcttaagcctcaataaagcttgccttgagtgcttcaagtagtgtgtgcccgtctgttgtgtgactctggtaactagagatccctcagacccttttagtcagtgtggaaaatctctagcagggcccgtttaaacccgctgatcagcctcgactgtgccttctagttgccagccatctgttgtttgcccctcccccgtgccttccttgaccctggaaggtgccactcccactgtcctttcctaataaaatgaggaaattgcatcgcattgtctgagtaggtgtcattctattctggggggtggggtggggcaggacagcaagggggaggattgggaagacaatagcaggcatgctggggatgcggtgggctctatggcttctgaggcggaaagaaccagctggggctctagggggtatccccacgcgccctgtagcggcgcattaagcgcggcgggtgtggtggttacgcgcagcgtgaccgctacacttgccagcgccctagcgcccgctcctttcgctttcttcccttcctttctcgccacgttcgccggctttccccgtcaagctctaaatcgggggctccctttagggttccgatttagtgctttacggcacctcgaccccaaaaaacttgattagggtgatggttcacgtagtgggccatcgccctgatagacggtttttcgccctttgacgttggagtccacgttctttaatagtggactcttgttccaaactggaacaacactcaaccctatctcggtctattcttttgatttataagggattttgccgatttcggcctattggttaaaaaatgagctgatttaacaaaaatttaacgcgaattaattctgtggaatgtgtgtcagttagggtgtggaaagtccccaggctccccagcaggcagaagtatgcaaagcatgcatctcaattagtcagcaaccaggtgtggaaagtccccaggctccccagcaggcagaagtatgcaaagcatgcatctcaattagtcagcaaccatagtcccgcccctaactccgcccatcccgcccctaactccgcccagttccgcccattctccgccccatggctgactaattttttttatttatgcagaggccgaggccgcctctgcctctgagctattccagaagtagtgaggaggcttttttggaggcctaggcttttgcaaaaagctcccgggagcttgtatatccattttcggatctgatcagcacgtgttgacaattaatcatcggcatagtatatcggcatagtataatacgacaaggtgaggaactaaaccatggccaagttgaccagtgccgttccggtgctcaccgcgcgcgacgtcgccggagcggtcgagttctggaccgaccggctcgggttctcccgggacttcgtggaggacgacttcgccggtgtggtccgggacgacgtgaccctgttcatcagcgcggtccaggaccaggtggtgccggacaacaccctggcctgggtgtgggtgcgcggcctggacgagctgtacgccgagtggtcggaggtcgtgtccacgaacttccgggacgcctccgggccggccatgaccgagatcggcgagcagccgtgggggcgggagttcgccctgcgcgacccggccggcaactgcgtgcacttcgtggccgaggagcaggactgacacgtgctacgagatttcgattccaccgccgccttctatgaaaggttgggcttcggaatcgttttccgggacgccggctggatgatcctccagcgcggggatctcatgctggagttcttcgcccaccccaacttgtttattgcagcttataatggttacaaataaagcaatagcatcacaaatttcacaaataaagcatttttttcactgcattctagttgtggtttgtccaaactcatcaatgtatcttatcatgtctgtataccgtcgacctctagctagagcttggcgtaatcatggtcatagctgtttcctgtgtgaaattgttatccgctcacaattccacacaacatacgagccggaagcataaagtgtaaagcctggggtgcctaatgagtgagctaactcacattaattgcgttgcgctcactgcccgctttccagtcgggaaacctgtcgtgccagctgcattaatgaatcggccaacgcgcggggagaggcggtttgcgtattgggcgctcttccgcttcctcgctcactgactcgctgcgctcggtcgttcggctgcggcgagcggtatcagctcactcaaaggcggtaatacggttatccacagaatcaggggataacgcaggaaagaacatgtgagcaaaaggccagcaaaaggccaggaaccgtaaaaaggccgcgttgctggcgtttttccataggctccgcccccctgacgagcatcacaaaaatcgacgctcaagtcagaggtggcgaaacccgacaggactataaagataccaggcgtttccccctggaagctccctcgtgcgctctcctgttccgaccctgccgcttaccggatacctgtccgcctttctcccttcgggaagcgtggcgctttctcatagctcacgctgtaggtatctcagttcggtgtaggtcgttcgctccaagctgggctgtgtgcacgaaccccccgttcagcccgaccgctgcgccttatccggtaactatcgtcttgagtccaacccggtaagacacgacttatcgccactggcagcagccactggtaacaggattagcagagcgaggtatgtaggcggtgctacagagttcttgaagtggtggcctaactacggctacactagaagaacagtatttggtatctgcgctctgctgaagccagttaccttcggaaaaagagttggtagctcttgatccggcaaacaaaccaccgctggtagcggtggtttttttgtttgcaagcagcagattacgcgcagaaaaaaaggatctcaagaagatcctttgatcttttctacggggtctgacgctcagtggaacgaaaactcacgttaagggattttggtcatgagattatcaaaaaggatcttcacctagatccttttaaattaaaaatgaagttttaaatcaatctaaagtatatatgagtaaacttggtctgacagttaccaatgcttaatcagtgaggcacctatctcagcgatctgtctatttcgttcatccatagttgcctgactccccgtcgtgtagataactacgatacgggagggcttaccatctggccccagtgctgcaatgataccgcgagacccacgctcaccggctccagatttatcagcaataaaccagccagccggaagggccgagcgcagaagtggtcctgcaactttatccgcctccatccagtctattaattgttgccgggaagctagagtaagtagttcgccagttaatagtttgcgcaacgttgttgccattgctacaggcatcgtggtgtcacgctcgtcgtttggtatggcttcattcagctccggttcccaacgatcaaggcgagttacatgatcccccatgttgtgcaaaaaagcggttagctccttcggtcctccgatcgttgtcagaagtaagttggccgcagtgttatcactcatggttatggcagcactgcataattctcttactgtcatgccatccgtaagatgcttttctgtgactggtgagtactcaaccaagtcattctgagaatagtgtatgcggcgaccgagttgctcttgcccggcgtcaatacgggataataccgcgccacatagcagaactttaaaagtgctcatcattggaaaacgttcttcggggcgaaaactctcaaggatcttaccgctgttgagatccagttcgatgtaacccactcgtgcacccaactgatcttcagcatcttttactttcaccagcgtttctgggtgagcaaaaacaggaaggcaaaatgccgcaaaaaagggaataagggcgacacggaaatgttgaatactcatactcttcctttttcaatattattgaagcatttatcagggttattgtctcatgagcggatacatatttgaatgtatttagaaaaataaacaaataggggttccgcgcacatttccccgaaaagtgccacctgac

SEQ ID NO: 36 - protein, 553 aa, unidentified
MVSKGEELFTGVVPILVELDGDVNGHKFSVSGEGEGDATYGKLTLKFICTTGKLPVPWPTLVTTLTYGVQCFSRYPDHMKQHDFFKSAMPEGYVQERTIFFKDDGNYKTRAEVKFEGDTLVNRIELKGIDFKEDGNILGHKLEYNYNSHNVYIMADKQKNGIKVNFKIRHNIEDGSVQLADHYQQNTPIGDGPVLLPDNHYLSTQSALSKDPNEKRDHMVLLEFVTAAGITLGMDELYSKSFQQSSLSRDSQGHGRDLSAAGIGLLAAATQSLSMPASLGRMNQGTARLASLMNLGMSSSLNQQGAHSALSSASTSSHNLQSIFNIGSRGPLPLSSQHRGDADQASNILASFGLSARDLDELSRYPEDKITPENLPQILLQLKRRRTEEGPTLSYGRDGRSATREPPYRVPRDDWEEKRHFRRDSFDDRGPSLNPVLDYDHGSRSQESGYYDRMDYEDDRLRDGERCRDDSFFGETSHNYHKFDSEYERMGRGPGPLQERSLFEKKRGAPPSSNIEDFHGLLPKGRDPKKKRKVEDPKKKRKVEDPKKKRKVD

SEQ ID NO: 37 - DNA, 9459 bp, synthetic construct
  source 1..9459: mol_type = other DNA
aaatttcacaaataaagcatttttttcactgcattctagttgtggtttgtccaaactcatcaatgtatcttatcatgtctggctctagctatcccgcccctaactccgcccagttccgcccattctccgccccatggctgactaattttttttatttatgcagaggccgaggccgcctcggcctctgagctattccagaagtagtgaggaggcttttttggaggcctaggcttttgcgtcgagacgtacccaattcgccctatagtgagtcgtattacgcgcgctcactggccgtcgttttacaacgtcgtgactgggaaaaccctggcgttacccaacttaatcgccttgcagcacatccccctttcgccagctggcgtaatagcgaagaggcccgcaccgatcgcccttcccaacagttgcgcagcctgaatggcgaatggcgcgacgcgccctgtagcggcgcattaagcgcggcgggtgtggtggttacgcgcagcgtgaccgctacacttgccagcgccctagcgcccgctcctttcgctttcttcccttcctttctcgccacgttcgccggctttccccgtcaagctctaaatcgggggctccctttagggttccgatttagtgctttacggcacctcgaccccaaaaaacttgattagggtgatggttcacgtagtgggccatcgccctgatagacggtttttcgccctttgacgttggagtccacgttctttaatagtggactcttgttccaaactggaacaacactcaaccctatctcggtctattcttttgatttataagggattttgccgatttcggcctattggttaaaaaatgagctgatttaacaaaaatttaacgcgaattttaacaaaatattaacgtttacaatttcccaggtggcacttttcggggaaatgtgcgcggaacccctatttgtttatttttctaaatacattcaaatatgtatccgctcatgagacaataaccctgataaatgcttcaataatattgaaaaaggaagagtatgagtattcaacatttccgtgtcgcccttattcccttttttgcggcattttgccttcctgtttttgctcacccagaaacgctggtgaaagtaaaagatgctgaagatcagttgggtgcacgagtgggttacatcgaactggatctcaacagcggtaagatccttgagagttttcgccccgaagaacgttttccaatgatgagcacttttaaagttctgctatgtggcgcggtattatcccgtattgacgccgggcaagagcaactcggtcgccgcatacactattctcagaatgacttggttgagtactcaccagtcacagaaaagcatcttacggatggcatgacagtaagagaattatgcagtgctgccataaccatgagtgataacactgcggccaacttacttctgacaacgatcggaggaccgaaggagctaaccgcttttttgcacaacatgggggatcatgtaactcgccttgatcgttgggaaccggagctgaatgaagccataccaaacgacgagcgtgacaccacgatgcctgtagcaatggcaacaacgttgcgcaaactattaactggcgaactacttactctagcttcccggcaacaattaatagactggatggaggcggataaagttgcaggaccacttctgcgctcggcccttccggctggctggtttattgctgataaatctggagccggtgagcgtgggtctcgcggtatcattgcagcactggggccagatggtaagccctcccgtatcgtagttatctacacgacggggagtcaggcaactatggatgaacgaaatagacagatcgctgagataggtgcctcactgattaagcattggtaactgtcagaccaagtttactcatatatactttagattgatttaaaacttcatttttaatttaaaaggatctaggtgaagatcctttttgataatctcatgaccaaaatcccttaacgtgagttttcgttccactgagcgtcagaccccgtagaaaagatcaaaggatcttcttgagatcctttttttctgcgcgtaatctgctgcttgcaaacaaaaaaaccaccgctaccagcggtggtttgtttgccggatcaagagctaccaactctttttccgaaggtaactggcttcagcagagcgcagataccaaatactgtccttctagtgtagccgtagttaggccaccacttcaagaactctgtagcaccgcctacatacctcgctctgctaatcctgttaccagtggctgctgccagtggcgataagtcgtgtcttaccgggttggactcaagacgatagttaccggataaggcgcagcggtcgggctgaacggggggttcgtgcacacagcccagcttggagcgaacgacctacaccgaactgagatacctacagcgtgagctatgagaaagcgccacgcttcccgaagggagaaaggcggacaggtatccggtaagcggcagggtcggaacaggagagcgcacgagggagcttccagggggaaacgcctggtatctttatagtcctgtcgggtttcgccacctctgacttgagcgtcgatttttgtgatgctcgtcaggggggcggagcctatggaaaaacgccagcaacgcggcctttttacggttcctggccttttgctggccttttgctcacatgttctttcctgcgttatcccctgattctgtggataaccgtattaccgcctttgagtgagctgataccgctcgccgcagccgaacgaccgagcgcagcgagtcagtgagcgaggaagcggaagagcgcccaatacgcaaaccgcctctccccgcgcgttggccgattcattaatgcagctggcacgacaggtttcccgactggaaagcgggcagtgagcgcaacgcaattaatgtgagttagctcactcattaggcaccccaggctttacactttatgcttccggctcgtatgttgtgtggaattgtgagcggataacaatttcacacaggaaacagctatgaccatgattacgccaagcgcgcaattaaccctcactaaagggaacaaaagctggagctgcaagcttggccattgcatacgttgtatccatatcataatatgtacatttatattggctcatgtccaacattaccgccatgttgacattgattattgactagttattaatagtaatcaattacggggtcattagttcatagcccatatatggagttccgcgttacataacttacggtaaatggcccgcctggctgaccgcccaacgacccccgcccattgacgtcaataatgacgtatgttcccatagtaacgccaatagggactttccattgacgtcaatgggtggagtatttacggtaaactgcccacttggcagtacatcaagtgtatcatatgccaagtacgccccctattgacgtcaatgacggtaaatggcccgcctggcattatgcccagtacatgaccttatgggactttcctacttggcagtacatctacgtattagtcatcgctattaccatggtgatgcggttttggcagtacatcaatgggcgtggatagcggtttgactcacggggatttccaagtctccaccccattgacgtcaatgggagtttgttttggcaccaaaatcaacgggactttccaaaatgtcgtaacaactccgccccattgacgcaaatgggcggtaggcgtgtacggtgggaggtctatataagcagagctcgtttagtgaaccggggtctctctggttagaccagatctgagcctgggagctctctggctaactagggaacccactgcttaagcctcaataaagcttgccttgagtgcttcaagtagtgtgtgcccgtctgttgtgtgactctggtaactagagatccctcagacccttttagtcagtgtggaaaatctctagcagtggcgcccgaacagggacctgaaagcgaaagggaaaccagagctctctcgacgcaggactcggcttgctgaagcgcgcacggcaagaggcgaggggcggcgactggtgagtacgccaaaaattttgactagcggaggctagaaggagagagatgggtgcgagagcgtcagtattaagcgggggagaattagatcgcgatgggaaaaaattcggttaaggccagggggaaagaaaaaatataaattaaaacatatagtatgggcaagcagggagctagaacgattcgcagttaatcctggcctgttagaaacatcagaaggctgtagacaaatactgggacagctacaaccatcccttcagacaggatcagaagaacttagatcattatataatacagtagcaaccctctattgtgtgcatcaaaggatagagataaaagacaccaaggaagctttagacaagatagaggaagagcaaaacaaaagtaagaccaccgcacagcaagcggccgctgatcttcagacctggaggaggagatatgagggacaattggagaagtgaattatataaatataaagtagtaaaaattgaaccattaggagtagcacccaccaaggcaaagagaagagtggtgcagagagaaaaaagagcagtgggaataggagctttgttccttgggttcttgggagcagcaggaagcactatgggcgcagcctcaatgacgctgacggtacaggccagacaattattgtctggtatagtgcagcagcagaacaatttgctgagggctattgaggcgcaacagcatctgttgcaactcacagtctggggcatcaagcagctccaggcaagaatcctggctgtggaaagatacctaaaggatcaacagctcctggggatttggggttgctctggaaaactcatttgcaccactgctgtgccttggaatgctagttggagtaataaatctctggaacagattggaatcacacgacctggatggagtgggacagagaaattaacaattacacaagcttaatacactccttaattgaagaatcgcaaaaccagcaagaaaagaatgaacaagaattattggaattagataaatgggcaagtttgtggaattggtttaacataacaaattggctgtggtatataaaattattcataatgatagtaggaggcttggtaggtttaagaatagtttttgctgtactttctatagtgaatagagttaggcagggatattcaccattatcgtttcagacccacctcccaaccccgaggggacccgacaggcccgaaggaatagaagaagaaggtggagagagagacagagacagatccattcgattagtgaacggatctcgacggtatcggttaacttttaaaagaaaaggggggattggggggtacagtgcaggggaaagaatagtagacataatagcaacagacatacaaactaaagaattacaaaaacaaattacaaaaattcaaaattttatcgatcacgagactagcctcgagaagcttgattatatactagtatgaaaccccacctgtaggtttggcaagctagctgcagtaacgccattttgcaaggcatggaaaaataccaaaccaagaatagagaagttcagatcaagggcgggtacatgaaaatagctaacgttgggccaaacaggatatctgcggtgagcagtttcggccccggcccggggccaagaacagatggtcaccgcagtttcggccccggcccgaggccaagaacagatggtccccagatatggcccaaccctcagcagtttcttaagacccatcagatgtttccaggctcccccaaggacctgaaatgaccctgcgccttatttgaattaaccaatcagcctgcttctcgcttctgttcgcgcgcttctgcttcccgagctctataaaagagctcacaacccctcactcggcttaattaaaagctttatataatcagcatcacaagtttgtacaaaaaagcaggctccatggattacaaggatgacgacgataagagcccgggcggatcctccaagtcattccagcagtcatctctcagtagggactcacagggtcatgggcgtgacctgtctgcggcaggaataggccttcttgctgctgctacccagtctttaagtatgccagcatctcttggaaggatgaaccagggtactgcacgccttgctagtttaatgaatcttggaatgagttcttcattgaatcaacaaggagctcatagtgcactgtcttctgctagtacttcttcccataatttgcagtctatatttaacattggaagtagaggtccactccctttatcttctcaacaccgtggagatgcagaccaggccagtaacattttggccagctttggtctgtctgctagagacttagatgaactgagtcgttatccagaggacaagattactcctgagaatttgccccaaatccttctacagcttaaaaggaggagaactgaagaaggccctaccttgagttatggtagagatggcagatctgctacacgggagccaccatacagagtacctagggatgattgggaagaaaaaaggcactttagaagagatagttttgatgatcgtggtcctagtctcaacccagtgcttgattatgaccatggaagtcgttctcaagaatctggttattatgacagaatggattatgaagatgacagattaagagatggagaaaggtgtagggatgattctttttttggtgagacctcgcataactatcataaatttgacagtgagtatgagagaatgggacgtggtcctggccccttacaagagagatctctctttgagaaaaagagaggcgctcctccaagtagcaatattgaagacttccatggactcttaccgaagggtagggatcccaagaaaaaacgcaaggtggaagatcctaagaaaaagcggaaagtggaagacccaaaaaagaagagaaaggtagactaataagacccagctttcttgtacaaagtggtgatgctctagaatgcatgcatgccgtacgatcgccgcctcaggcctgagttcgaagtatacgtcgacaatcaacctctggattacaaaatttgtgaaagattgactggtattcttaactatgttgctccttttacgctatgtggatacgctgctttaatgcctttgtatcatgctattgcttcccgtatggctttcattttctcctccttgtataaatcctggttgctgtctctttatgaggagttgtggcccgttgtcaggcaacgtggcgtggtgtgcactgtgtttgctgacgcaacccccactggttggggcattgccaccacctgtcagctcctttccgggactttcgctttccccctccctattgccacggcggaactcatcgccgcctgccttgcccgctgctggacaggggctcggctgttgggcactgacaattccgtggtgttgtcggggaagctgacgtcctttccatggctgctcgcctgtgttgccacctggattctgcgcgggacgtcttctgctacgtcccttcggcctcaatcagcggacttccttcccgcggcctgctgccggctctgcggcctcttccgcgtcttcgccttcgccctcagacgagtcggatctccctttgggccgcctccccgcctggaattcctgcagcccgggggatcaaggatctgcgatcgctccggtgcccgtcagtgggcagagcgcacatcgcccacagtccccgagaagttggggggaggggtcggcaattgaacgggtgcctagagaaggtggcgcggggtaaactgggaaagtgatgtcgtgtactggctccgcctttttcccgagggtgggggagaaccgtatataagtgcagtagtcgccgtgaacgttctttttcgcaacgggtttgccgccagaacacagctgaagcttcgaggggctcgcatctctccttcacgcgcccgccgccctacctgaggccgccatccacgccggttgagtcgcgttctgccgcctcccgcctgtggtgcctcctgaactgcgtccgccgtctaggtaagtttaaagctcaggtcgagaccgggcctttgtccggcgctcccttggagcctacctagactcagccggctctccacgctttgcctgaccctgcttgctcaactctacgtctttgtttcgttttctgttctgcgccgttacagatccaagctgtgaccggcgcctacgatccaccggtcgccaccatgagcgagctgattaaggagaacatgcacatgaagctgtacatggagggcaccgtggacaaccatcacttcaagtgcacatccgagggcgaaggcaagccctacgagggcacccagaccatgagaatcaaggtggtcgagggcggccctctccccttcgccttcgacatcctggctactagcttcctctacggcagcaagaccttcatcaaccacacccagggcatccccgacttcttcaagcagtccttccctgagggcttcacatgggagagagtcaccacatacgaagacgggggcgtgctgaccgctacccaggacaccagcctccaggacggctgcctcatctacaacgtcaagatcagaggggtgaacttcacatccaacggccctgtgatgcagaagaaaacactcggctgggaggccttcaccgagacgctgtaccccgctgacggcggcctggaaggcagaaacgacatggccctgaagctcgtgggcgggagccatctgatcgcaaacatcaagaccacatatagatccaagaaacccgctaagaacctcaagatgcctggcgtctactatgtggactacagactggaaagaatcaaggaggccaacaacgagacctacgtcgagcagcacgaggtggcagtggccagatactgcgacctccctagcaaactggggcacaagcttaattaaagcggccgcgtcgagagatgggggaggctaactgagctagcttagtcatgcaccgggctgcaggaattcgagctcggtacctttaagaccaatgacttacaaggcagctgtagatcttagccactttttaaaagaaaaggggggactggaagggctaattcactcccaacgaagacaagatctgctttttgcttgtactgggtctctctggttagaccagatctgagcctgggagctctctggctaactagggaacccactgcttaagcctcaataaagcttgccttgagtgcttcaagtagtgtgtgcccgtctgttgtgtgactctggtaactagagatccctcagacccttttagtcagtgtggaaaatctctagcagtagtagttcatgtcatcttattattcagtatttataacttgcaaagaaatgaatatcagagagtgagaggaacttgtttattgcagcttataatggttacaaataaagcaatagcatcac

SEQ ID NO: 38 - protein, 329 aa, synthetic construct; identical to SEQ ID NO: 34

SEQ ID NO: 39 - DNA, 8192 bp, synthetic construct
  source 1..8192: mol_type = other DNA
aatgcagctgcgcgctcgctcgctcactgaggccgcccgggcaaagcccgggcgtcgggcgacctttggtcgcccggcctcagtgagcgagcgagcgcgcagagagggagtggccaactccatcactaggggttccttgtagttaatgattaacccgccatgctacttatctacaaactctagcatgctgcccatgtaaggaggcaaggcctggggacacccgagatgcctggttataattaacccagacatgtggctgcccccccccccccaacacctgctgcctctaaaaataaccctgcatgccatgttcccggcgaagggccagctgtcccccgccagctagactcagcacttagtttaggaaccagtgagcaagtcagcccttggggcagcccatacaaggccatggggctgggcaagctgcacgcctgggtccggggtgggcacggtgcccgggcaacgagctgaaagctcatctgctctcaggggcccctccctggggacagcccctcctggctagtcacaccctgtaggctcctctatataacccaggggcacaggggctgccctcattctaccaccacctccacagcacagacagacactcaggagccagccagcgtcgaggttaaccatggtgagcaagggcgaggaggataacatggccatcatcaaggagttcatgcgcttcaaggtgcacatggagggctccgtgaacggccacgagttcgagatcgagggcgagggcgagggccgcccctacgagggcacccagaccgccaagctgaaggtgaccaagggtggccccctgcccttcgcctgggacatcctgtcccctcagttcatgtacggctccaaggcctacgtgaagcaccccgccgacatccccgactacttgaagctgtccttccccgagggcttcaagtgggagcgcgtgatgaacttcgaggacggcggcgtggtgaccgtgacccaggactcctccctgcaggacggcgagttcatctacaaggtgaagctgcgcggcaccaacttcccctccgacggccccgtaatgcagaagaagaccatgggctgggaggcctcctccgagcggatgtaccccgaggacggcgccctgaagggcgagatcaagcagaggctgaagctgaaggacggcggccactacgacgctgaggtcaagaccacctacaaggccaagaagcccgtgcagctgcccggcgcctacaacgtcaacatcaagttggacatcacctcccacaacgaggactacaccatcgtggaacagtacgaacgcgccgagggccgccactccaccggcggcatggacgagctgtacaagtagggggatccgaccggtgctagcggccgccaattgcaacgtcgtgactgggaaaaccctggcgttacccaacttaatcgccttgcagcacatccccctttcgccagctggcgtaatagcgaagaggcccgcaccgatcgcccttcccaacagttgcgcagcctgaatggcgaatggcgctttgcctggtttccggcaccagaagcggtgccggaaagctggctggagtgcgatcttcctgaggccgatactgtcgtcgtcccctcaaactggcagatgcacggttacgatgcgcccatctacaccaacgtgacctatcccattacggtcaatccgccgtttgttcccacggagaatccgacgggttgttactcgctcacatttaatgttgatgaaagctggctacaggaaggccagacgcgaattatttttgatggcgttaactcggcgtttcatctgtggtgcaacgggcgctgggtcggttacggccaggacagtcgtttgccgtctgaatttgacctgagcgcatttttacgcgccggagaaaaccgcctcgcggtgatggtgctgcgctggagtgacggcagttatctggaagatcaggatatgtggcggatgagcggcattttccgtgacgtctcgttgctgcataaaccgactacacaaatcagcgatttccatgttgccactcgctttaatgatgatttcagccgcgctgtactggaggctgaagttcagatgtgcggcgagttgcgtgactacctacgggtaacagtttctttatggcagggtgaaacgcaggtcgccagcggcaccgcgcctttcggcggtgaaattatcgatgagcgtggtggttatgccgatcgcgtcacactacgtctgaacgtcgaaaacccgaaactgtggagcgccgaaatcccgaatctctatcgtgcggtggttgaactgcacaccgccgacggcacgctgattgaagcagaagcctgcgatgtcggtttccgcgaggtgcggattgaaaatggtctgctgctgctgaacggcaagccgttgctgattcgaggcgttaaccgtcacgagcatcatcctctgcatggtcaggtcatggatgagcagacgatggtgcaggatatcctgctgatgaagcagaacaactttaacgccgtgcgctgttcgcattatccgaaccatccgctgtggtacacgctgtgcgaccgctacggcctgtatgtggtggatgaagccaatattgaaacccacggcatggtgccaatgaatcgtctgaccgatgatccgcgctggctaccggcgatgagcgaacgcgtaacgcgaatggtgcagcgcgatcgtaatcacccgagtgtgatcatctggtcgctggggaatgaatcaggccacggcgctaatcacgacgcgctgtatcgctggatcaaatctgtcgatccttcccgcccggtgcagtatgaaggcggcggagccgacaccacggccaccgatattatttgcccgatgtacgcgcgcgtggatgaagaccagcccttcccggctgtgccgaaatggtccatcaaaaaatggctttcgctacctggagagacgcgcccgctgatcctttgcgaatacgcccacgcgatgggtaacagtcttggcggtttcgctaaatactggcaggcgtttcgtcagtatccccgtttacagggcggcttcgtctgggactgggtggatcagtcgctgattaaatatgatgaaaacggcaacccgtggtcggcttacggcggtgattttggcgatacgccgaacgatcgccagttctgtatgaacggtctggtctttgccgaccgcacgccgcatccagcgctgacggaagcaaaacaccagcagcagtttttccagttccgtttatccgggcaaaccatcgaagtgaccagcgaatacctgttccgtcatagcgataacgagctcctgcactggatggtggcgctggatggtaagccgctggcaagcggtgaagtgcctctggatgtcgctccacaaggtaaacagttgattgaactgcctgaactaccgcagccggagagcgccgggcaactctggctcacagtacgcgtagtgcaaccgaacgcgaccgcatggtcagaagccgggcacatcagcgcctggcagcagtggcgtctggcggaaaacctcagtgtgacgctccccgccgcgtcccacgccatcccgcatctgaccaccagcgaaatggatttttgcatcgagctgggtaataagcgttggcaatttaaccgccagtcaggctttctttcacagatgtggattggcgataaaaaacaactgctgacgccgctgcgcgatcagttcacccgtgcaccgctggataacgacattggcgtaagtgaagcgacccgcattgaccctaacgcctgggtcgaacgctggaaggcggcgggccattaccaggccgaagcagcgttgttgcagtgcacggcagatacacttgctgatgcggtgctgattacgaccgctcacgcgtggcagcatcaggggaaaaccttatttatcagccggaaaacctaccggattgatggtagtggtcaaatggcgattaccgttgatgttgaagtggcgagcgatacaccgcatccggcgcggattggcctgaactgccagctggcgcaggtagcagagcgggtaaactggctcggattagggccgcaagaaaactatcccgaccgccttactgccgcctgttttgaccgctgggatctgccattgtcagacatgtataccccgtacgtcttcccgagcgaaaacggtctgcgctgcgggacgcgcgaattgaattatggcccacaccagtggcgcggcgacttccagttcaacatcagccgctacagtcaacagcaactgatggaaaccagccatcgccatctgctgcacgcggaagaaggcacatggctgaatatcgacggtttccatatggggattggtggcgacgactcctggagcccgtcagtatcggcgttaaccggtggctagtaataaaagatccttattttcattggatctgtgtgttggttttttgtgtgggtaccgtttgtagataagtagcatggcgggttaatcattaactacaaggaacccctagtgatggagttggccactccctctctgcgcgctcgctcgctcactgaggccgggcgaccaaaggtcgcccgacgcccgggctttgcccgggcggcctcagtgagcgagcgagcgcgcagctggcgtaatagcgaagaggcccgcaccgatcgcccttcccaacagttgcgcagcctgaatggcgaatggcgattccgttgcaatggctggcggtaatattgttctggatattaccagcaaggccgatagtttgagttcttctactcaggcaagtgatgttattactaatcaaagaagtattgcgacaacggttaatttgcgtgatggacagactcttttactcggtggcctcactgattataaaaacacttctcaggattctggcgtaccgttcctgtctaaaatccctttaatcggcctcctgtttagctcccgctctgattctaacgaggaaagcacgttatacgtgctcgtcaaagcaaccatagtacgcgccctgtagcggcgcattaagcgcggcgggtgtggtggttacgcgcagcgtgaccgctacacttgccagcgccctagcgcccgctcctttcgctttcttcccttcctttctcgccacgttcgccggctttccccgtcaagctctaaatcgggggctccctttagggttccgatttagtgctttacggcacctcgaccccaaaaaacttgattagggtgatggttcacgtagtgggccatcgccctgatagacggtttttcgccctttgacgttggagtccacgttctttaatagtggactcttgttccaaactggaacaacactcaaccctatctcggtctattcttttgatttataagggattttgccgatttcggcctattggttaaaaaatgagctgatttaacaaaaatttaacgcgaattttaacaaaatattaacgtttacaatttaaatatttgcttatacaatcttcctgtttttggggcttttctgattatcaaccggggtacatatgattgacatgctagttttacgattaccgttcatcgattctcttgtttgctccagactctcaggcaatgacctgatagcctttgtagagacctctcaaaaatagctaccctctccggcatgaatttatcagctagaacggttgaatatcatattgatggtgatttgactgtctccggcctttctcacccgtttgaatctttacctacacattactcaggcattgcatttaaaatatatgagggttctaaaaatttttatccttgcgttgaaataaaggcttctcccgcaaaagtattacagggtcataatgtttttggtacaaccgatttagctttatgctctgaggctttattgcttaattttgctaattctttgccttgcctgtatgatttattggatgttggaattcctgatgcggtattttctccttacgcatctgtgcggtatttcacaccgcatatggtgcactctcagtacaatctgctctgatgccgcatagttaagccagccccgacacccgccaacacccgctgacgcgccctgacgggcttgtctgctcccggcatccgcttacagacaagctgtgaccgtctccgggagctgcatgtgtcagaggttttcaccgtcatcaccgaaacgcgcgagacgaaagggcctcgtgatacgcctatttttataggttaatgtcatgataataatggtttcttagacgtcaggtggcacttttcggggaaatgtgcgcggaacccctatttgtttatttttctaaatacattcaaatatgtatccgctcatgagacaataaccctgataaatgcttcaataatattgaaaaaggaagagtatgagtattcaacatttccgtgtcgcccttattcccttttttgcggcattttgccttcctgtttttgctcacccagaaacgctggtgaaagtaaaagatgctgaagatcagttgggtgcacgagtgggttacatcgaactggatctcaacagcggtaagatccttgagagttttcgccccgaagaacgttttccaatgatgagcacttttaaagttctgctatgtggcgcggtattatcccgtattgacgccgggcaagagcaactcggtcgccgcatacactattctcagaatgacttggttgagtactcaccagtcacagaaaagcatcttacggatggcatgacagtaagagaattatgcagtgctgccataaccatgagtgataacactgcggccaacttacttctgacaacgatcggaggaccgaaggagctaaccgcttttttgcacaacatgggggatcatgtaactcgccttgatcgttgggaaccggagctgaatgaagccataccaaacgacgagcgtgacaccacgatgcctgtagcaatggcaacaacgttgcgcaaactattaactggcgaactacttactctagcttcccggcaacaattaatagactggatggaggcggataaagttgcaggaccacttctgcgctcggcccttccggctggctggtttattgctgataaatctggagccggtgagcgtgggtctcgcggtatcattgcagcactggggccagatggtaagccctcccgtatcgtagttatctacacgacggggagtcaggcaactatggatgaacgaaatagacagatcgctgagataggtgcctcactgattaagcattggtaactgtcagaccaagtttactcatatatactttagattgatttaaaacttcatttttaatttaaaaggatctaggtgaagatcctttttgataatctcatgaccaaaatcccttaacgtgagttttcgttccactgagcgtcagaccccgtagaaaagatcaaaggatcttcttgagatcctttttttctgcgcgtaatctgctgcttgcaaacaaaaaaaccaccgctaccagcggtggtttgtttgccggatcaagagctaccaactctttttccgaaggtaactggcttcagcagagcgcagataccaaatactgtccttctagtgtagccgtagttaggccaccacttcaagaactctgtagcaccgcctacatacctcgctctgctaatcctgttaccagtggctgctgccagtggcgataagtcgtgtcttaccgggttggactcaagacgatagttaccggataaggcgcagcggtcgggctgaacggggggttcgtgcacacagcccagcttggagcgaacgacctacaccgaactgagatacctacagcgtgagctatgagaaagcgccacgcttcccgaagggagaaaggcggacaggtatccggtaagcggcagggtcggaacaggagagcgcacgagggagcttccagggggaaacgcctggtatctttatagtcctgtcgggtttcgccacctctgacttgagcgtcgatttttgtgatgctcgtcaggggggcggagcctatggaaaaacgccagcaacgcggcctttttacggttcctggccttttgctggccttttgctcacatgttctttcctgcgttatcccctgattctgtggataaccgtattaccgcctttgagtgagctgataccgctcgccgcagccgaacgaccgagcgcagcgagtcagtgagcgaggaagcggaagagcgcccaatacgcaaaccgcctctccccgcgcgttggccgattcattaatg

SEQ ID NO: 40 - protein, 236 aa, synthetic construct
MVSKGEEDNMAIIKEFMRFKVHMEGSVNGHEFEIEGEGEGRPYEGTQTAKLKVTKGGPLPFAWDILSPQFMYGSKAYVKHPADIPDYLKLSFPEGFKWERVMNFEDGGVVTVTQDSSLQDGEFIYKVKLRGTNFPSDGPVMQKKTMGWEASSERMYPEDGALKGEIKQRLKLKDGGHYDAEVKTTYKAKKPVQLPGAYNVNIKLDITSHNEDYTIVEQYERAEGRHSTGGMDELYK

SEQ ID NO: 41 - DNA, 8365 bp, synthetic construct
  source 1..8365: mol_type = other DNA
cagctgcgcgctcgctcgctcactgaggccgcccgggcaaagcccgggcgtcgggcgacctttggtcgcccggcctcagtgagcgagcgagcgcgcagagagggagtggccaactccatcactaggggttccttgtagttaatgattaacccgccatgctacttatctacaaactctagcatgctgcccatgtaaggaggcaaggcctggggacacccgagatgcctggttataattaacccagacatgtggctgcccccccccccccaacacctgctgcctctaaaaataaccctgcatgccatgttcccggcgaagggccagctgtcccccgccagctagactcagcacttagtttaggaaccagtgagcaagtcagcccttggggcagcccatacaaggccatggggctgggcaagctgcacgcctgggtccggggtgggcacggtgcccgggcaacgagctgaaagctcatctgctctcaggggcccctccctggggacagcccctcctggctagtcacaccctgtaggctcctctatataacccaggggcacaggggctgccctcattctaccaccacctccacagcacagacagacactcaggagccagccagcgtcgaggttaacgccaccatggtgagcaagggcgaggagctgttcaccggggtggtgcccatcctggtcgagctggacggcgacgtaaacggccacaagttcagcgtgtccggcgagggcgagggcgatgccacctacggcaagctgaccctgaagttcatctgcaccaccggcaagctgcccgtgccctggcccaccctcgtgaccaccctgacctacggcgtgcagtgcttcagccgctaccccgaccacatgaagcagcacgacttcttcaagtccgccatgcccgaaggctacgtccaggagcgcaccatcttcttcaaggacgacggcaactacaagacccgcgccgaggtgaagttcgagggcgacaccctggtgaaccgcatcgagctgaagggcatcgacttcaaggaggacggcaacatcctggggcacaagctggagtacaactacaacagccacaacgtctatatcatggccgacaagcagaagaacggcatcaaggtgaacttcaagatccgccacaacatcgaggacggcagcgtgcagctcgccgaccactaccagcagaacacccccatcggcgacggccccgtgctgctgcccgacaaccactacctgagcacccagtccgccctgagcaaagaccccaacgagaagcgcgatcacatggtcctgctggagttcgtgaccgccgccgggatcactctcggcatggacgagctgtactccaagtcattccagcagtcatctctcagtagggactcacagggtcatgggcgtgacctgtctgcggcaggaataggccttcttgctgctgctacccagtctttaagtatgccagcatctcttggaaggatgaaccagggtactgcacgccttgctagtttaatgaatcttggaatgagttcttcattgaatcaacaaggagctcatagtgcactgtcttctgctagtacttcttcccataatttgcagtctatatttaacattggaagtagaggtccactccctttatcttctcaacaccgtggagatgcagaccaggccagtaacattttggccagctttggtctgtctgctagagacttagatgaactgagtcgttatccagaggacaagattactcctgagaatttgccccaaatccttctacagcttaaaaggaggagaactgaagaaggccctaccttgagttatggtagagatggcagatctgctacacgggagccaccatacagagtacctagggatgattgggaagaaaaaaggcactttagaagagatagttttgatgatcgtggtcctagtctcaacccagtgcttgattatgaccatggaagtcgttctcaagaatctggttattatgacagaatggattatgaagatgacagattaagagatggagaaaggtgtagggatgattctttttttggtgagacctcgcataactatcataaatttgacagtgagtatgagagaatgggacgtggtcctggccccttacaagagagatctctctttgagaaaaagagaggcgctcctccaagtagcaatattgaagacttccatggactcttaccgaagggtagggatcccaagaaaaaacgcaaggtggaagatcctaagaaaaagcggaaagtggaagacccaaaaaagaagagaaaggtataaaccggtgcagggtgaaacgcaggtcgccagcggcaccgcgcctttcggcggtgaaattatcgatgagcgtggtggttatgccgatcgcgtcacactacgtctgaacgtcgaaaacccgaaactgtggagcgccgaaatcccgaatctctatcgtgcggtggttgaactgcacaccgccgacggcacgctgattgaagcagaagcctgcgatgtcggtttccgcgaggtgcggattgaaaatggtctgctgctgctgaacggcaagccgttgctgattcgaggcgttaaccgtcacgagcatcatcctctgcatggtcaggtcatggatgagcagacgatggtgcaggatatcctgctgatgaagcagaacaactttaacgccgtgcgctgttcgcattatccgaaccatccgctgtggtacacgctgtgcgaccgctacggcctgtatgtggtggatgaagccaatattgaaacccacggcatggtgccaatgaatcgtctgaccgatgatccgcgctggctaccggcgatgagcgaacgcgtaacgcgaatggtgcagcgcgatcgtaatcacccgagtgtgatcatctggtcgctggggaatgaatcaggccacggcgctaatcacgacgcgctgtatcgctggatcaaatctgtcgatccttcccgcccggtgcagtatgaaggcggcggagccgacaccacggccaccgatattatttgcccgatgtacgcgcgcgtggatgaagaccagcccttcccggctgtgccgaaatggtccatcaaaaaatggctttcgctacctggagagacgcgcccgctgatcctttgcgaatacgcccacgcgatgggtaacagtcttggcggtttcgctaaatactggcaggcgtttcgtcagtatccccgtttacagggcggcttcgtctgggactgggtggatcagtcgctgattaaatatgatgaaaacggcaacccgtggtcggcttacggcggtgattttggcgatacgccgaacgatcgccagttctgtatgaacggtctggtctttgccgaccgcacgccgcatccagcgctgacggaagcaaaacaccagcagcagtttttccagttccgtttatccgggcaaaccatcgaagtgaccagcgaatacctgttccgtcatagcgataacgagctcctgcactggatggtggcgctggatggtaagccgctggcaagcggtgaagtgcctctggatgtcgctccacaaggtaaacagttgattgaactgcctgaactaccgcagccggagagcgccgggcaactctggctcacagtacgcgtagtgcaaccgaacgcgaccgcatggtcagaagccgggcacatcagcgcctggcagcagtggcgtctggcggaaaacctcagtgtgacgctccccgccgcgtcccacgccatcccgcatctgaccaccagcgaaatggatttttgcatcgagctgggtaataagcgttggcaatttaaccgccagtcaggctttctttcacagatgtggattggcgataaaaaacaactgctgacgccgctgcgcgatcagttcacccgtgcaccgctggataacgacattggcgtaagtgaagcgacccgcattgaccctaacgcctgggtcgaacgctggaaggcggcgggccattaccaggccgaagcagcgttgttgcagtgcacggcagatacacttgctgatgcggtgctgattacgaccgctcacgcgtggcagcatcaggggaaaaccttatttatcagccggaaaacctaccggattgatggtagtggtcaaatggcgattaccgttgatgttgaagtggcgagcgatacaccgcatccggcgcggattggcctgaactgccagctggcgcaggtagcagagcgggtaaactggctcggattagggccgcaagaaaactatcccgaccgccttactgccgcctgttttgaccgctgggatctgccattgtcagacatgtataccccgtacgtcttcccgagcgaaaacggtctgcgctgcgggacgcgcgaattgaattatggcccacaccagtggcgcggcgacttccagttcaacatcagccgctacagtcaacagcaactgatggaaaccagccatcgccatctgctgcacgcggaagaaggcacatggctgaatatcgacggtttccatatggggattggtggcgacgactcctggagcccgtcagtatcggcgtaaaccggtggctagtaataaaagatccttattttcattggatctgtgtgttggttttttgtgtgggtaccgtttgtagataagtagcatggcgggttaatcattaactacaaggaacccctagtgatggagttggccactccctctctgcgcgctcgctcgctcactgaggccgggcgaccaaaggtcgcccgacgcccgggctttgcccgggcggcctcagtgagcgagcgagcgcgcagctggcgtaatagcgaagaggcccgcaccgatcgcccttcccaacagttgcgcagcctgaatggcgaatggcgattccgttgcaatggctggcggtaatattgttctggatattaccagcaaggccgatagtttgagttcttctactcaggcaagtgatgttattactaatcaaagaagtattgcgacaacggttaatttgcgtgatggacagactcttttactcggtggcctcactgattataaaaacacttctcaggattctggcgtaccgttcctgtctaaaatccctttaatcggcctcctgtttagctcccgctctgattctaacgaggaaagcacgttatacgtgctcgtcaaagcaaccatagtacgcgccctgtagcggcgcattaagcgcggcgggtgtggtggttacgcgcagcgtgaccgctacacttgccagcgccctagcgcccgctcctttcgctttcttcccttcctttctcgccacgttcgccggctttccccgtcaagctctaaatcgggggctccctttagggttccgatttagtgctttacggcacctcgaccccaaaaaacttgattagggtgatggttcacgtagtgggccatcgccctgatagacggtttttcgccctttgacgttggagtccacgttctttaatagtggactcttgttccaaactggaacaacactcaaccctatctcggtctattcttttgatttataagggattttgccgatttcggcctattggttaaaaaatgagctgatttaacaaaaatttaacgcgaattttaacaaaatattaacgtttacaatttaaatatttgcttatacaatcttcctgtttttggggcttttctgattatcaaccggggtacatatgattgacatgctagttttacgattaccgttcatcgattctcttgtttgctccagactctcaggcaatgacctgatagcctttgtagagacctctcaaaaatagctaccctctccggcatgaatttatcagctagaacggttgaatatcatattgatggtgatttgactgtctccggcctttctcacccgtttgaatctttacctacacattactcaggcattgcatttaaaatatatgagggttctaaaaatttttatccttgcgttgaaataaaggcttctcccgcaaaagtattacagggtcataatgtttttggtacaaccgatttagctttatgctctgaggctttattgcttaattttgctaattctttgccttgcctgtatgatttattggatgttggaattcctgatgcggtattttctccttacgcatctgtgcggtatttcacaccgcatatggtgcactctcagtacaatctgctctgatgccgcatagttaagccagccccgacacccgccaacacccgctgacgcgccctgacgggcttgtctgctcccggcatccgcttacagacaagctgtgaccgtctccgggagctgcatgtgtcagaggttttcaccgtcatcaccgaaacgcgcgagacgaaagggcctcgtgatacgcctatttttataggttaatgtcatgataataatggtttcttagacgtcaggtggcacttttcggggaaatgtgcgcggaacccctatttgtttatttttctaaatacattcaaatatgtatccgctcatgagacaataaccctgataaatgcttcaataatattgaaaaaggaagagtatgagtattcaacatttccgtgtcgcccttattcccttttttgcggcattttgccttcctgtttttgctcacccagaaacgctggtgaaagtaaaagatgctgaagatcagttgggtgcacgagtgggttacatcgaactggatctcaacagcggtaagatccttgagagttttcgccccgaagaacgttttccaatgatgagcacttttaaagttctgctatgtggcgcggtattatcccgtattgacgccgggcaagagcaactcggtcgccgcatacactattctcagaatgacttggttgagtactcaccagtcacagaaaagcatcttacggatggcatgacagtaagagaattatgcagtgctgccataaccatgagtgataacactgcggccaacttacttctgacaacgatcggaggaccgaaggagctaaccgcttttttgcacaacatgggggatcatgtaactcgccttgatcgttgggaaccggagctgaatgaagccataccaaacgacgagcgtgacaccacgatgcctgtagcaatggcaacaacgttgcgcaaactattaactggcgaactacttactctagcttcccggcaacaattaatagactggatggaggcggataaagttgcaggaccacttctgcgctcggcccttccggctggctggtttattgctgataaatctggagccggtgagcgtgggtctcgcggtatcattgcagcactggggccagatggtaagccctcccgtatcgtagttatctacacgacggggagtcaggcaactatggatgaacgaaatagacagatcgctgagataggtgcctcactgattaagcattggtaactgtcagaccaagtttactcatatatactttagattgatttaaaacttcatttttaatttaaaaggatctaggtgaagatcctttttgataatctcatgaccaaaatcccttaacgtgagttttcgttccactgagcgtcagaccccgtagaaaagatcaaaggatcttcttgagatcctttttttctgcgcgtaatctgctgcttgcaaacaaaaaaaccaccgctaccagcggtggtttgtttgccggatcaagagctaccaactctttttccgaaggtaactggcttcagcagagcgcagataccaaatactgtccttctagtgtagccgtagttaggccaccacttcaagaactctgtagcaccgcctacatacctcgctctgctaatcctgttaccagtggctgctgccagtggcgataagtcgtgtcttaccgggttggactcaagacgatagttaccggataaggcgcagcggtcgggctgaacggggggttcgtgcacacagcccagcttggagcgaacgacctacaccgaactgagatacctacagcgtgagctatgagaaagcgccacgcttcccgaagggagaaaggcggacaggtatccggtaagcggcagggtcggaacaggagagcgcacgagggagcttccagggggaaacgcctggtatctttatagtcctgtcgggtttcgccacctctgacttgagcgtcgatttttgtgatgctcgtcaggggggcggagcctatggaaaaacgccagcaacgcggcctttttacggttcctggccttttgctggccttttgctcacatgttctttcctgcgttatcccctgattctgtggataaccgtattaccgcctttgagtgagctgataccgctcgccgcagccgaacgaccgagcgcagcgagtcagtgagcgaggaagcggaagagcgcccaatacgcaaaccgcctctccccgcgcgttggccgattcattaatg

SEQ ID NO: 42 - protein, 238 aa, synthetic construct
MVSKGEELFTGVVPILVELDGDVNGHKFSVSGEGEGDATYGKLTLKFICTTGKLPVPWPTLVTTLTYGVQCFSRYPDHMKQHDFFKSAMPEGYVQERTIFFKDDGNYKTRAEVKFEGDTLVNRIELKGIDFKEDGNILGHKLEYNYNSHNVYIMADKQKNGIKVNFKIRHNIEDGSVQLADHYQQNTPIGDGPVLLPDNHYLSTQSALSKDPNEKRDHMVLLEFVTAAGITLGMDELY

SEQ ID NO: 43 - protein, 287 aa, synthetic construct; identical to SEQ ID NO: 18

SEQ ID NO: 44 - protein, 7 aa, synthetic construct
PKKKRKV

SEQ ID NO: 45 - DNA, 8307 bp, synthetic construct
  source 1..8307: mol_type = other DNA
cagctgcgcgctcgctcgctcactgaggccgcccgggcaaagcccgggcgtcgggcgacctttggtcgcccggcctcagtgagcgagcgagcgcgcagagagggagtggccaactccatcactaggggttccttgtagttaatgattaacccgccatgctacttatctacaaactctagcatgctgcccatgtaaggaggcaaggcctggggacacccgagatgcctggttataattaacccagacatgtggctgcccccccccccccaacacctgctgcctctaaaaataaccctgcatgccatgttcccggcgaagggccagctgtcccccgccagctagactcagcacttagtttaggaaccagtgagcaagtcagcccttggggcagcccatacaaggccatggggctgggcaagctgcacgcctgggtccggggtgggcacggtgcccgggcaacgagctgaaagctcatctgctctcaggggcccctccctggggacagcccctcctggctagtcacaccctgtaggctcctctatataacccaggggcacaggggctgccctcattctaccaccacctccacagcacagacagacactcaggagccagccagcgtcgaggttaacgccaccatggtgagcaagggcgaggagctgttcaccggggtggtgcccatcctggtcgagctggacggcgacgtaaacggccacaagttcagcgtgtccggcgagggcgagggcgatgccacctacggcaagctgaccctgaagttcatctgcaccaccggcaagctgcccgtgccctggcccaccctcgtgaccaccctgacctacggcgtgcagtgcttcagccgctaccccgaccacatgaagcagcacgacttcttcaagtccgccatgcccgaaggctacgtccaggagcgcaccatcttcttcaaggacgacggcaactacaagacccgcgccgaggtgaagttcgagggcgacaccctggtgaaccgcatcgagctgaagggcatcgacttcaaggaggacggcaacatcctggggcacaagctggagtacaactacaacagccacaacgtctatatcatggccgacaagcagaagaacggcatcaaggtgaacttcaagatccgccacaacatcgaggacggcagcgtgcagctcgccgaccactaccagcagaacacccccatcggcgacggccccgtgctgctgcccgacaaccactacctgagcacccagtccgccctgagcaaagaccccaacgagaagcgcgatcacatggtcctgctggagttcgtgaccgccgccgggatcactctcggcatggacgagctgtactccaagtcattccagcagtcatctctcagtagggactcacagggtcatgggcgtgacctgtctgcggcaggaataggccttcttgctgctgctacccagtctttaagtatgccagcatctcttggaaggatgaaccagggtactgcacgccttgctagtttaatgaatcttggaatgagttcttcattgaatcaacaaggagctcatagtgcactgtcttctgctagtacttcttcccataatttgcagtctatatttaacattggaagtagaggtccactccctttatcttctcaacaccgtggagatgcagaccaggccagtaacattttggccagctttggtctgtctgctagagacttagatgaactgagtcgttatccagaggacaagattactcctgagaatttgccccaaatccttctacagcttaaaaggaggagaactgaagaaggccctaccttgagttatggtagagatggcagatctgctacacgggagccaccatacagagtacctagggatgattgggaagaaaaaaggcactttagaagagatagttttgatgatcgtggtcctagtctcaacccagtgcttgattatgaccatggaagtcgttctcaagaatctggttattatgacagaatggattatgaagatgacagattaagagatggagaaaggtgtagggatgattctttttttggtgagacctcgcataactatcataaatttgacagtgagtatgagagaatgggacgtggtcctggccccttacaagagagatctctctttgagaaaaagagaggcgctcctccaagtagcaatattgaagacttccatggactcttaccgaagggttatccccatctgtgctctatatgtgatttgccagttcattctaataaggagtggagtcaacatatcaatggagcaagtcacagtcgtcgatgccagcttcttcttgaaatctacccagaatggaatcctgacaatgatacaggacacacaatgggtgatccattcatgttgcagcagtctacaaatccagcaccaggaattctgggacctccacctccctcatttcatcttgggggaccagcagttggaccaagaggaaatctgggtgctggaaatggaaacctgcaaggacctagacacatgcagaaaggcagagtggaaactagcagagttgttcacatcatggattttcaacgagggaaaaacttgagataccagctattacagctggtagaaccatttggagtcatttcaaatcatctgattctaaataaaattaatgaggcatttattgaaatggcaaccacagaggatgctcaggccgcagtggattattacacaaccacaccagcgttagtatttggcaagccagtgagagttcatttatcccagaagtataaaagaataaagaaacctgaaggaaagccagatcagaagtttgatcaaaagcaagagcttggacgtgtgatacatctcagcaatttgccgcattctggctattctgatagtgctgttctcaagcttgctgagccttatgggaaaataaagaattacatattgatgaggatgaaaagtcaggcttttattgagatggagacaagagaagatgcaatggcaatggttgaccattgtttgaaaaaagccctttggtttcaggggagatgtgtgaaggttgacctgtctgagaaatataaaaaactggttctgaggattccaaacagaggcattgatttactgaaaaaagataaatcccgaaaaagatcttactctccagatggcaaagaatctccaagtgataagaaatccaaaactgatggttcccagaagactgagagttcaaccgaaggtaaagaacaagaagagaagtccggtgaagatggtgagaaagacacaaaggatgaccagacagagcaggaacctaatatgcttcttgaatctgaagatgagctacttgtagatgaagaagaagcagcagcactgctagaaagtggcagttcagtgggagacgagaccgatcttgctaatttaggtgatgtggcttctgatgggaaaaaggaaccatcagataaagctgtgaaaaaagatggaagtgcttcagcagcagcaaagaaaaagcttaaaaaggtggacaagatcgaggaacttgatcaagaaaacgaagcagcgttggaaaatggaattaaaaatgaggaaaacacagaaccaggtgctgaatcttctgagaacgctgatgatcccaacaaagatacaagtgaaaacgcagatggtcaaagtgatgagaacaaggacgactatacaatcccagatgagtatagaattggaccatatcagcccaatgttcctgttggtatagactatgtgatacctaaaacagggttttactgtaagctgtgttcactcttttatacaaatgaagaagttgcaaagaatactcattgcagcagccttcctcattatcagaaattaaagaaatttctgaataaattggcagaagaacgcagacagaagaaggaaacttaaaccggtgcgggccattaccaggccgaagcagcgttgttgcagtgcacggcagatacacttgctgatgcggtgctgattacgaccgctcacgcgtggcagcatcaggggaaaaccttatttatcagccggaaaacctaccggattgatggtagtggtcaaatggcgattaccgttgatgttgaagtggcgagcgatacaccgcatccggcgcggattggcctgaactgccagctggcgcaggtagcagagcgggtaaactggctcggattagggccgcaagaaaactatcccgaccgccttactgccgcctgttttgaccgctgggatctgccattgtcagacatgtataccccgtacgtcttcccgagcgaaaacggtctgcgctgcgggacgcgcgaattgaattatggcccacaccagtggcgcggcgacttccagttcaacatcagccgctacagtcaacagcaactgatggaaaccagccatcgccatctgctgcacgcggaagaaggcacatggctgaatatcgacggtttccatatggggattggtggcgacgactcctggagcccgtcagtatcggcgtaaaccggtggctagtaataaaagatccttattttcattggatctgtgtgttggttttttgtgtgggtaccgtttgtagataagtagcatggcgggttaatcattaactacaaggaacccctagtgatggagttggccactccctctctgcgcgctcgctcgctcactgaggccgggcgaccaaaggtcgcccgacgcccgggctttgcccgggcggcctcagtgagcgagcgagcgcgcagctggcgtaatagcgaagaggcccgcaccgatcgcccttcccaacagttgcgcagcctgaatggcgaatggcgattccgttgcaatggctggcggtaatattgttctggatattaccagcaaggccgatagtttgagttcttctactcaggcaagtgatgttattactaatcaaagaagtattgcgacaacggttaatttgcgtgatggacagactcttttactcggtggcctcactgattataaaaacacttctcaggattctggcgtaccgttcctgtctaaaatccctttaatcggcctcctgtttagctcccgctctgattctaacgaggaaagcacgttatacgtgctcgtcaaagcaaccatagtacgcgccctgtagcggcgcattaagcgcggcgggtgtggtggttacgcgcagcgtgaccgctacacttgccagcgccctagcgcccgctcctttcgctttcttcccttcctttctcgccacgttcgccggctttccccgtcaagctctaaatcgggggctccctttagggttccgatttagtgctttacggcacctcgaccccaaaaaacttgattagggtgatggttcacgtagtgggccatcgccctgatagacggtttttcgccctttgacgttggagtccacgttctttaatagtggactcttgttccaaactggaacaacactcaaccctatctcggtctattcttttgatttataagggattttgccgatttcggcctattggttaaaaaatgagctgatttaacaaaaatttaacgcgaattttaacaaaatattaacgtttacaatttaaatatttgcttatacaatcttcctgtttttggggcttttctgattatcaaccggggtacatatgattgacatgctagttttacgattaccgttcatcgattctcttgtttgctccagactctcaggcaatgacctgatagcctttgtagagacctctcaaaaatagctaccctctccggcatgaatttatcagctagaacggttgaatatcatattgatggtgatttgactgtctccggcctttctcacccgtttgaatctttacctacacattactcaggcattgcatttaaaatatatgagggttctaaaaatttttatccttgcgttgaaataaaggcttctcccgcaaaagtattacagggtcataatgtttttggtacaaccgatttagctttatgctctgaggctttattgcttaattttgctaattctttgccttgcctgtatgatttattggatgttggaattcctgatgcggtattttctccttacgcatctgtgcggtatttcacaccgcatatggtgcactctcagtacaatctgctctgatgccgcatagttaagccagccccgacacccgccaacacccgctgacgcgccctgacgggcttgtctgctcccggcatccgcttacagacaagctgtgaccgtctccgggagctgcatgtgtcagaggttttcaccgtcatcaccgaaacgcgcgagacgaaagggcctcgtgatacgcctatttttataggttaatgtcatgataataatggtttcttagacgtcaggtggcacttttcggggaaatgtgcgcggaacccctatttgtttatttttctaaatacattcaaatatgtatccgctcatgagacaataaccctgataaatgcttcaataatattgaaaaaggaagagtatgagtattcaacatttccgtgtcgcccttattcccttttttgcggcattttgccttcctgtttttgctcacccagaaacgctggtgaaagtaaaagatgctgaagatcagttgggtgcacgagtgggttacatcgaactggatctcaacagcggtaagatccttgagagttttcgccccgaagaacgttttccaatgatgagcacttttaaagttctgctatgtggcgcggtattatcccgtattgacgccgggcaagagcaactcggtcgccgcatacactattctcagaatgacttggttgagtactcaccagtcacagaaaagcatcttacggatggcatgacagtaagagaattatgcagtgctgccataaccatgagtgataacactgcggccaacttacttctgacaacgatcggaggaccgaaggagctaaccgcttttttgcacaacatgggggatcatgtaactcgccttgatcgttgggaaccggagctgaatgaagccataccaaacgacgagcgtgacaccacgatgcctgtagcaatggcaacaacgttgcgcaaactattaactggcgaactacttactctagcttcccggcaacaattaatagactggatggaggcggataaagttgcaggaccacttctgcgctcggcccttccggctggctggtttattgctgataaatctggagccggtgagcgtgggtctcgcggtatcattgcagcactggggccagatggtaagccctcccgtatcgtagttatctacacgacggggagtcaggcaactatggatgaacgaaatagacagatcgctgagataggtgcctcactgattaagcattggtaactgtcagaccaagtttactcatatatactttagattgatttaaaacttcatttttaatttaaaaggatctaggtgaagatcctttttgataatctcatgaccaaaatcccttaacgtgagttttcgttccactgagcgtcagaccccgtagaaaagatcaaaggatcttcttgagatcctttttttctgcgcgtaatctgctgcttgcaaacaaaaaaaccaccgctaccagcggtggtttgtttgccggatcaagagctaccaactctttttccgaaggtaactggcttcagcagagcgcagataccaaatactgtccttctagtgtagccgtagttaggccaccacttcaagaactctgtagcaccgcctacatacctcgctctgctaatcctgttaccagtggctgctgccagtggcgataagtcgtgtcttaccgggttggactcaagacgatagttaccggataaggcgcagcggtcgggctgaacggggggttcgtgcacacagcccagcttggagcgaacgacctacaccgaactgagatacctacagcgtgagctatgagaaagcgccacgcttcccgaagggagaaaggcggacaggtatccggtaagcggcagggtcggaacaggagagcgcacgagggagcttccagggggaaacgcctggtatctttatagtcctgtcgggtttcgccacctctgacttgagcgtcgatttttgtgatgctcgtcaggggggcggagcctatggaaaaacgccagcaacgcggcctttttacggttcctggccttttgctggccttttgctcacatgttctttcctgcgttatcccctgattctgtggataaccgtattaccgcctttgagtgagctgataccgctcgccgcagccgaacgaccgagcgcagcgagtcagtgagcgaggaagcggaagagcgcccaatacgcaaaccgcctctccccgcgcgttggccgattcattaatg

SEQ ID NO: 46 - protein, 238 aa, synthetic construct; identical to SEQ ID NO: 42

SEQ ID NO: 47 - protein, 846 aa, synthetic construct
SKSFQQSSLSRDSQGHGRDLSAAGIGLLAAATQSLSMPASLGRMNQGTARLASLMNLGMSSSLNQQGAHSALSSASTSSHNLQSIFNIGSRGPLPLSSQHRGDADQASNILASFGLSARDLDELSRYPEDKITPENLPQILLQLKRRRTEEGPTLSYGRDGRSATREPPYRVPRDDWEEKRHFRRDSFDDRGPSLNPVLDYDHGSRSQESGYYDRMDYEDDRLRDGERCRDDSFFGETSHNYHKFDSEYERMGRGPGPLQERSLFEKKRGAPPSSNIEDFHGLLPKGYPHLCSICDLPVHSNKEWSQHINGASHSRRCQLLLEIYPEWNPDNDTGHTMGDPFMLQQSTNPAPGILGPPPPSFHLGGPAVGPRGNLGAGNGNLQGPRHMQKGRVETSRVVHIMDFQRGKNLRYQLLQLVEPFGVISNHLILNKINEAFIEMATTEDAQAAVDYYTTTPALVFGKPVRVHLSQKYKRIKKPEGKPDQKFDQKQELGRVIHLSNLPHSGYSDSAVLKLAEPYGKIKNYILMRMKSQAFIEMETREDAMAMVDHCLKKALWFQGRCVKVDLSEKYKKLVLRIPNRGIDLLKKDKSRKRSYSPDGKESPSDKKSKTDGSQKTESSTEGKEQEEKSGEDGEKDTKDDQTEQEPNMLLESEDELLVDEEEAAALLESGSSVGDETDLANLGDVASDGKKEPSDKAVKKDGSASAAAKKKLKKVDKIEELDQENEAALENGIKNEENTEPGAESSENADDPNKDTSENADGQSDENKDDYTIPDEYRIGPYQPNVPVGIDYVIPKTGFYCKLCSLFYTNEEVAKNTHCSSLPHYQKLKKFLNKLAEERRQKKET

SEQ ID NO: 48 - DNA, 5458 bp, synthetic construct
  source 1..5458: mol_type = other DNA
acgttatcgactgcacggtgcaccaatgcttctggcgtcaggcagccatcggaagctgtggtatggctgtgcaggtcgtaaatcactgcataattcgtgtcgctcaaggcgcactcccgttctggataatgttttttgcgccgacatcataacggttctggcaaatattctgaaatgagctgttgacaattaatcatcggctcgtataatgtgtggaattgtgagcggataacaatttcacacaggaaacagtattcttgacaattaatcatcggctcgtataatgtgtggaattgtgagcggataacaatttcacacaggaaacagtattcatgtcccctatactaggttattggaaaattaagggccttgtgcaacccactcgacttcttttggaatatcttgaagaaaaatatgaagagcatttgtatgagcgcgatgaaggtgataaatggcgaaacaaaaagtttgaattgggtttggagtttcccaatcttccttattatattgatggtgatgttaaattaacacagtctatggccatcatacgttatatagctgacaagcacaacatgttgggtggttgtccaaaagagcgtgcagagatttcaatgcttgaaggagcggttttggatattagatacggtgtttcgagaattgcatatagtaaagactttgaaactctcaaagttgattttcttagcaagctacctgaaatgctgaaaatgttcgaagatcgtttatgtcataaaacatatttaaatggtgatcatgtaacccatcctgacttcatgttgtatgacgctcttgatgttgttttatacatggacccaatgtgcctggatgcgttcccaaaattagtttgttttaaaaaacgtattgaagctatcccacaaattgataagtacttgaaatccagcaagtatatagcatggcctttgcagggctggcaagccacgtttggtggtggcgaccatcctccaaaatcggatctggttccgcgtggatctcgtcgtgcatctgttggatccgaagaaggccctaccttgagttatggtagagatggcagatctgctacacgggagccaccatacagagtacctagggatgattgggaagaaaaaaggcactttagaagagatagttttgatgatcgtggtcctagtctcaacccagtgcttgattatgaccatggaagtcgttctcaagaatctggttattatgacagaatggattatgaagatgacagattaagagatggagaaaggtgtagggatgattctttttttggtgagacctcgcataactatcataaatttgacagtgagtatgagagaatgggacgtggtcctggccccttacaagagagatctctctttgagaaaaagagaggcgctcctccaagtagcaatattgaagacttccatggactcttaccgaagtaaccgggaattcatcgtgactgactgacgatctgcctcgcgcgtttcggtgatgacggtgaaaacctctgacacatgcagctcccggagacggtcacagcttgtctgtaagcggatgccgggagcagacaagcccgtcagggcgcgtcagcgggtgttggcgggtgtcggggcgcagccatgacccagtcacgtagcgatagcggagtgtataattcttgaagacgaaagggcctcgtgatacgcctatttttataggttaatgtcatgataataatggtttcttagacgtcaggtggcacttttcggggaaatgtgcgcggaacccctatttgtttatttttctaaatacattcaaatatgtatccgctcatgagacaataaccctgataaatgcttcaataatattgaaaaaggaagagtatgagtattcaacatttccgtgtcgcccttattcccttttttgcggcattttgccttcctgtttttgctcacccagaaacgctggtgaaagtaaaagatgctgaagatcagttgggtgcacgagtgggttacatcgaactggatctcaacagcggtaagatccttgagagttttcgccccgaagaacgttttccaatgatgagcacttttaaagttctgctatgtggcgcggtattatcccgtgttgacgccgggcaagagcaactcggtcgccgcatacactattctcagaatgacttggttgagtactcaccagtcacagaaaagcatcttacggatggcatgacagtaagagaattatgcagtgctgccataaccatgagtgataacactgcggccaacttacttctgacaacgatcggaggaccgaaggagctaaccgcttttttgcacaacatgggggatcatgtaactcgccttgatcgttgggaaccggagctgaatgaagccataccaaacgacgagcgtgacaccacgatgcctgcagcaatggcaacaacgttgcgcaaactattaactggcgaactacttactctagcttcccggcaacaattaatagactggatggaggcggataaagttgcaggaccacttctgcgctcggcccttccggctggctggtttattgctgataaatctggagccggtgagcgtgggtctcgcggtatcattgcagcactggggccagatggtaagccctcccgtatcgtagttatctacacgacggggagtcaggcaactatggatgaacgaaatagacagatcgctgagataggtgcctcactgattaagcattggtaactgtcagaccaagtttactcatatatactttagattgatttaaaacttcatttttaatttaaaaggatctaggtgaagatcctttttgataatctcatgaccaaaatcccttaacgtgagttttcgttccactgagcgtcagaccccgtagaaaagatcaaaggatcttcttgagatcctttttttctgcgcgtaatctgctgcttgcaaacaaaaaaaccaccgctaccagcggtggtttgtttgccggatcaagagctaccaactctttttccgaaggtaactggcttcagcagagcgcagataccaaatactgtccttctagtgtagccgtagttaggccaccacttcaagaactctgtagcaccgcctacatacctcgctctgctaatcctgttaccagtggctgctgccagtggcgataagtcgtgtcttaccgggttggactcaagacgatagttaccggataaggcgcagcggtcgggctgaacggggggttcgtgcacacagcccagcttggagcgaacgacctacaccgaactgagatacctacagcgtgagctatgagaaagcgccacgcttcccgaagggagaaaggcggacaggtatccggtaagcggcagggtcggaacaggagagcgcacgagggagcttccagggggaaacgcctggtatctttatagtcctgtcgggtttcgccacctctgacttgagcgtcgatttttgtgatgctcgtcaggggggcggagcctatggaaaaacgccagcaacgcggcctttttacggttcctggccttttgctggccttttgctcacatgttctttcctgcgttatcccctgattctgtggataaccgtattaccgcctttgagtgagctgataccgctcgccgcagccgaacgaccgagcgcagcgagtcagtgagcgaggaagcggaagagcgcctgatgcggtattttctccttacgcatctgtgcggtatttcacaccgcataaattccgacaccatcgaatggtgcaaaacctttcgcggtatggcatgatagcgcccggaagagagtcaattcagggtggtgaatgtgaaaccagtaacgttatacgatgtcgcagagtatgccggtgtctcttatcagaccgtttcccgcgtggtgaaccaggccagccacgtttctgcgaaaacgcgggaaaaagtggaagcggcgatggcggagctgaattacattcccaaccgcgtggcacaacaactggcgggcaaacagtcgttgctgattggcgttgccacctccagtctggccctgcacgcgccgtcgcaaattgtcgcggcgattaaatctcgcgccgatcaactgggtgccagcgtggtggtgtcgatggtagaacgaagcggcgtcgaagcctgtaaagcggcggtgcacaatcttctcgcgcaacgcgtcagtgggctgatcattaactatccgctggatgaccaggatgccattgctgtggaagctgcctgcactaatgttccggcgttatttcttgatgtctctgaccagacacccatcaacagtattattttctcccatgaagacggtacgcgactgggcgtggagcatctggtcgcattgggtcaccagcaaatcgcgctgttagcgggcccattaagttctgtctcggcgcgtctgcgtctggctggctggcataaatatctcactcgcaatcaaattcagccgatagcggaacgggaaggcgactggagtgccatgtccggttttcaacaaaccatgcaaatgctgaatgagggcatcgttcccactgcgatgctggttgccaacgatcagatggcgctgggcgcaatgcgcgccattaccgagtccgggctgcgcgttggtgcggatatctcggtagtgggatacgacgataccgaagacagctcatgttatatcccgccgttaaccaccatcaaacaggattttcgcctgctggggcaaaccagcgtggaccgcttgctgcaactctctcagggccaggcggtgaagggcaatcagctgttgcccgtctcactggtgaaaagaaaaaccaccctggcgcccaatacgcaaaccgcctctccccgcgcgttggccgattcattaatgcagctggcacgacaggtttcccgactggaaagcgggcagtgagcgcaacgcaattaatgtgagttagctcactcattaggcaccccaggctttacactttatgcttccggctcgtatgttgtgtggaattgtgagcggataacaatttcacacaggaaacagctatgaccatgattacggattcactggccgtcgttttacaacgtcgtgactgggaaaaccctggcgttacccaacttaatcgccttgcagcacatccccctttcgccagctggcgtaatagcgaagaggcccgcaccgatcgcccttcccaacagttgcgcagcctgaatggcgaatggcgctttgcctggtttccggcaccagaagcggtgccggaaagctggctggagtgcgatcttcctgaggccgatactgtcgtcgtcccctcaaactggcagatgcacggttacgatgcgcccatctacaccaacgtaacctatcccattacggtcaatccgccgtttgttcccacggagaatccgacgggttgttactcgctcacatttaatgttgatgaaagctggctacaggaaggccagacgcgaattatttttgatggcgttggaatt

SEQ ID NO: 49 - protein, 370 aa, synthetic construct
MSPILGYWKIKGLVQPTRLLLEYLEEKYEEHLYERDEGDKWRNKKFELGLEFPNLPYYIDGDVKLTQSMAIIRYIADKHNMLGGCPKERAEISMLEGAVLDIRYGVSRIAYSKDFETLKVDFLSKLPEMLKMFEDRLCHKTYLNGDHVTHPDFMLYDALDVVLYMDPMCLDAFPKLVCFKKRIEAIPQIDKYLKSSKYIAWPLQGWQATFGGGDHPPKSDLVPRGSRRASVGSEEGPTLSYGRDGRSATREPPYRVPRDDWEEKRHFRRDSFDDRGPSLNPVLDYDHGSRSQESGYYDRMDYEDDRLRDGERCRDDSFFGETSHNYHKFDSEYERMGRGPGPLQERSLFEKKRGAPPSSNIEDFHGLLPK

SEQ ID NO: 50 - DNA, 4777 bp, synthetic construct
  source 1..4777: mol_type = other DNA
atgcattagttattaatagtaatcaattacggggtcattagttcatagcccatatatggagttccgcgttacataacttacggtaaatggcccgcctggctgaccgcccaacgacccccgcccattgacgtcaataatgacgtatgttcccatagtaacgccaatagggactttccattgacgtcaatgggtggagtatttacggtaaactgcccacttggcagtacatcaagtgtatcatatgccaagtacgccccctattgacgtcaatgacggtaaatggcccgcctggcattatgcccagtacatgaccttatgggactttcctacttggcagtacatctacgtattagtcatcgctattaccatggtgatgcggttttggcagtacatcaatgggcgtggatagcggtttgactcacggggatttccaagtctccaccccattgacgtcaatgggagtttgttttggcaccaaaatcaacgggactttccaaaatgtcgtaacaactccgccccattgacgcaaatgggcggtaggcgtgtacggtgggaggtctatataagcagagctggtttagtgaaccgtcagatccgctagcgattacgccaagctcgaaattaaccctcactaaagggaacaaaagctggagctccaccgcggtggcggccgccaccatggattacaaggatgacgacgataagagcccgggcggatccgaagaaggccctaccttgagttatggtagagatggcagatctgctacacgggagccaccatacagagtacctagggatgattgggaagaaaaaaggcactttagaagagatagttttgatgatcgtggtcctagtctcaacccagtgcttgattatgaccatggaagtcgttctcaagaatctggttattatgacagaatggattatgaagatgacagattaagagatggagaaaggtgtagggatgattctttttttggtgagacctcgcataactatcataaatttgacagtgagtatgagagaatgggacgtggtcctggccccttacaagagagatctctctttgagaaaaagagaggcgctcctccaagtagcaatattgaagacttccatggactcttaccgaagaaggatcccaagaaaaaacgcaaggtggaagatcctaagaaaaagcggaaagtggaagacccaaaaaagaagagaaaggtagactgactcgagggggggcccggtaccttaattaattaaggtaccaggtaagtgtacccaattcgccctatagtgagtcgtattacaattcactcgatcgcccttcccaacagttgcgcagcctgaatggcgaatggagatccaatttttaagtgtataatgtgttaaactactgattctaattgtttgtgtattttagattcacagtcccaaggctcatttcaggcccctcagtcctcacagtctgttcatgatcataatcagccataccacatttgtagaggttttacttgctttaaaaaacctcccacacctccccctgaacctgaaacataaaatgaatgcaattgttgttgttaacttgtttattgcagcttataatggttacaaataaagcaatagcatcacaaatttcacaaataaagcatttttttcactgcattctagttgtggtttgtccaaactcatcaatgtatcttaacgcgtaaattgtaagcgttaatattttgttaaaattcgcgttaaatttttgttaaatcagctcattttttaaccaataggccgaaatcggcaaaatcccttataaatcaaaagaatagaccgagatagggttgagtgttgttccagtttggaacaagagtccactattaaagaacgtggactccaacgtcaaagggcgaaaaaccgtctatcagggcgatggcccactacgtgaaccatcaccctaatcaagttttttggggtcgaggtgccgtaaagcactaaatcggaaccctaaagggagcccccgatttagagcttgacggggaaagccggcgaacgtggcgagaaaggaagggaagaaagcgaaaggagcgggcgctagggcgctggcaagtgtagcggtcacgctgcgcgtaaccaccacacccgccgcgcttaatgcgccgctacagggcgcgtcaggtggcacttttcggggaaatgtgcgcggaacccctatttgtttatttttctaaatacattcaaatatgtatccgctcatgagacaataaccctgataaatgcttcaataatattgaaaaaggaagaatcctgaggcggaaagaaccagctgtggaatgtgtgtcagttagggtgtggaaagtccccaggctccccagcaggcagaagtatgcaaagcatgcatctcaattagtcagcaaccaggtgtggaaagtccccaggctccccagcaggcagaagtatgcaaagcatgcatctcaattagtcagcaaccatagtcccgcccctaactccgcccatcccgcccctaactccgcccagttccgcccattctccgccccatggctgactaattttttttatttatgcagaggccgaggccgcctcggcctctgagctattccagaagtagtgaggaggcttttttggaggcctaggcttttgcaaagatcgatcaagagacaggatgaggatcgtttcgcatgattgaacaagatggattgcacgcaggttctccggccgcttgggtggagaggctattcggctatgactgggcacaacagacaatcggctgctctgatgccgccgtgttccggctgtcagcgcaggggcgcccggttctttttgtcaagaccgacctgtccggtgccctgaatgaactgcaagacgaggcagcgcggctatcgtggctggccacgacgggcgttccttgcgcagctgtgctcgacgttgtcactgaagcgggaagggactggctgctattgggcgaagtgccggggcaggatctcctgtcatctcaccttgctcctgccgagaaagtatccatcatggctgatgcaatgcggcggctgcatacgcttgatccggctacctgcccattcgaccaccaagcgaaacatcgcatcgagcgagcacgtactcggatggaagccggtcttgtcgatcaggatgatctggacgaagaacatcaggggctcgcgccagccgaactgttcgccaggctcaaggcgagcatgcccgacggcgaggatctcgtcgtgacccatggcgatgcctgcttgccgaatatcatggtggaaaatggccgcttttctggattcatcgactgtggccggctgggtgtggcggaccgctatcaggacatagcgttggctacccgtgatattgctgaagaacttggcggcgaatgggctgaccgcttcctcgtgctttacggtatcgccgctcccgattcgcagcgcatcgccttctatcgccttcttgacgagttcttctgagcgggactctggggttcgaaatgaccgaccaagcgacgcccaacctgccatcacgagatttcgattccaccgccgccttctatgaaaggttgggcttcggaatcgttttccgggacgccggctggatgatcctccagcgcggggatctcatgctggagttcttcgcccaccctagggggaggctaactgaaacacggaaggagacaataccggaaggaacccgcgctatgacggcaataaaaagacagaataaaacgcacggtgttgggtcgtttgttcataaacgcggggttcggtcccagggctggcactctgtcgataccccaccgagaccccattggggccaatacgcccgcgtttcttccttttccccaccccaccccccaagttcgggtgaaggcccagggctcgcagccaacgtcggggcggcaggccctgccatagcctcaggttactcatatatactttagattgatttaaaacttcatttttaatttaaaaggatctaggtgaagatcctttttgataatctcatgaccaaaatcccttaacgtgagttttcgttccactgagcgtcagaccccgtagaaaagatcaaaggatcttcttgagatcctttttttctgcgcgtaatctgctgcttgcaaacaaaaaaaccaccgctaccagcggtggtttgtttgccggatcaagagctaccaactctttttccgaaggtaactggcttcagcagagcgcagataccaaatactgtccttctagtgtagccgtagttaggccaccacttcaagaactctgtagcaccgcctacatacctcgctctgctaatcctgttaccagtggctgctgccagtggcgataagtcgtgtcttaccgggttggactcaagacgatagttaccggataaggcgcagcggtcgggctgaacggggggttcgtgcacacagcccagcttggagcgaacgacctacaccgaactgagatacctacagcgtgagctatgagaaagcgccacgcttcccgaagggagaaaggcggacaggtatccggtaagcggcagggtcggaacaggagagcgcacgagggagcttccagggggaaacgcctggtatctttatagtcctgtcgggtttcgccacctctgacttgagcgtcgatttttgtgatgctcgtcaggggggcggagcctatggaaaaacgccagcaacgcggcctttttacggttcctggccttttgctggccttttgctcacatgttctttcctgcgttatcccctgattctgtggataaccgtattaccgcc

SEQ ID NO: 51 - protein, 179 aa, synthetic construct
MDYKDDDDKSPGGSEEGPTLSYGRDGRSATREPPYRVPRDDWEEKRHFRRDSFDDRGPSLNPVLDYDHGSRSQESGYYDRMDYEDDRLRDGERCRDDSFFGETSHNYHKFDSEYERMGRGPGPLQERSLFEKKRGAPPSSNIEDFHGLLPKKDPKKKRKVEDPKKKRKVEDPKKKRKVD

SEQ ID NO: 52 - DNA, 10464 bp, synthetic construct
  source 1..10464: mol_type = other DNA
gtcgacggatcgggagatctcccgatcccctatggtgcactctcagtacaatctgctctgatgccgcatagttaagccagtatctgctccctgcttgtgtgttggaggtcgctgagtagtgcgcgagcaaaatttaagctacaacaaggcaaggcttgaccgacaattgcatgaagaatctgcttagggttaggcgttttgcgctgcttcgcgatgtacgggccagatatacgcgttgacattgattattgactagttattaatagtaatcaattacggggtcattagttcatagcccatatatggagttccgcgttacataacttacggtaaatggcccgcctggctgaccgcccaacgacccccgcccattgacgtcaataatgacgtatgttcccatagtaacgccaatagggactttccattgacgtcaatgggtggagtatttacggtaaactgcccacttggcagtacatcaagtgtatcatatgccaagtacgccccctattgacgtcaatgacggtaaatggcccgcctggcattatgcccagtacatgaccttatgggactttcctacttggcagtacatctacgtattagtcatcgctattaccatggtgatgcggttttggcagtacatcaatgggcgtggatagcggtttgactcacggggatttccaagtctccaccccattgacgtcaatgggagtttgttttggcaccaaaatcaacgggactttccaaaatgtcgtaacaactccgccccattgacgcaaatgggcggtaggcgtgtacggtgggaggtctatataagcagcgcgttttgcctgtactgggtctctctggttagaccagatctgagcctgggagctctctggctaactagggaacccactgcttaagcctcaataaagcttgccttgagtgcttcaagtagtgtgtgcccgtctgttgtgtgactctggtaactagagatccctcagacccttttagtcagtgtggaaaatctctagcagtggcgcccgaacagggacttgaaagcgaaagggaaaccagaggagctctctcgacgcaggactcggcttgctgaagcgcgcacggcaagaggcgaggggcggcgactggtgagtacgccaaaaattttgactagcggaggctagaaggagagagatgggtgcgagagcgtcagtattaagcgggggagaattagatcgcgatgggaaaaaattcggttaaggccagggggaaagaaaaaatataaattaaaacatatagtatgggcaagcagggagctagaacgattcgcagttaatcctggcctgttagaaacatcagaaggctgtagacaaatactgggacagctacaaccatcccttcagacaggatcagaagaacttagatcattatataatacagtagcaaccctctattgtgtgcatcaaaggatagagataaaagacaccaaggaagctttagacaagatagaggaagagcaaaacaaaagtaagaccaccgcacagcaagcggccgctgatcttcagacctggaggaggagatatgagggacaattggagaagtgaattatataaatataaagtagtaaaaattgaaccattaggagtagcacccaccaaggcaaagagaagagtggtgcagagagaaaaaagagcagtgggaataggagctttgttccttgggttcttgggagcagcaggaagcactatgggcgcagcgtcaatgacgctgacggtacaggccagacaattattgtctggtatagtgcagcagcagaacaatttgctgagggctattgaggcgcaacagcatctgttgcaactcacagtctggggcatcaagcagctccaggcaagaatcctggctgtggaaagatacctaaaggatcaacagctcctggggatttggggttgctctggaaaactcatttgcaccactgctgtgccttggaatgctagttggagtaataaatctctggaacagatttggaatcacacgacctggatggagtgggacagagaaattaacaattacacaagcttaatacactccttaattgaagaatcgcaaaaccagcaagaaaagaatgaacaagaattattggaattagataaatgggcaagtttgtggaattggtttaacataacaaattggctgtggtatataaaattattcataatgatagtaggaggcttggtaggtttaagaatagtttttgctgtactttctatagtgaatagagttaggcagggatattcaccattatcgtttcagacccacctcccaaccccgaggggacccgacaggcccgaaggaatagaagaagaaggtggagagagagacagagacagatccattcgattagtgaacggatcggcactgcgtgcgccaattctgcagacaaatggcagtattcatccacaattttaaaagaaaaggggggattggggggtacagtgcaggggaaagaatagtagacataatagcaacagacatacaaactaaagaattacaaaaacaaattacaaaaattcaaaattttcgggtttattacagggacagcagagatccagtttggttaattaacccgtgtcggctccagatctggcctccgcgccgggttttggcgcctcccgcgggcgcccccctcctcacggcgagcgctgccacgtcagacgaagggcgcagcgagcgtcctgatccttccgcccggacgctcaggacagcggcccgctgctcataagactcggccttagaaccccagtatcagcagaaggacattttaggacgggacttgggtgactctagggcactggttttctttccagagagcggaacaggcgaggaaaagtagtcccttctcggcgattctgcggagggatctccgtggggcggtgaacgccgatgattatataaggacgcgccgggtgtggcacagctagttccgtcgcagccgggatttgggtcgcggttcttgtttgtggatcgctgtgatcgtcacttggtgagtagcgggctgctgggctggccggggctttcgtggccgccgggccgctcggtgggacggaagcgtgtggagagaccgccaagggctgtagtctgggtccgcgagcaaggttgccctgaactgggggttggggggagcgcagcaaaatggcggctgttcccgagtcttgaatggaagacgcttgtgaggcgggctgtgaggtcgttgaaacaaggtggggggcatggtgggcggcaagaacccaaggtcttgaggccttcgctaatgcgggaaagctcttattcgggtgagatgggctggggcaccatctggggaccctgacgtgaagtttgtcactgactggagaactcggtttgtcgtctgttgcgggggcggcagttatggcggtgccgttgggcagtgcacccgtacctttgggagcgcgcgccctcgtcgtgtcgtgacgtcacccgttctgttggcttataatgcagggtggggccacctgccggtaggtgtgcggtaggcttttctccgtcgcaggacgcagggttcgggcctagggtaggctctcctgaatcgacaggcgccggacctctggtgaggggagggataagtgaggcgtcagtttctttggtcggttttatgtacctatcttcttaagtagctgaagctccggttttgaactatgcgctcggggttggcgagtgtgttttgtgaagttttttaggcaccttttgaaatgtaatcatttgggtcaatatgtaattttcagtgttagactagtaaattgtccgctaaattctggccgtttttggcttttttgttagacgaagcttgggctgcaggtcgactctagaggatccccgggtaccggtcgccaccatggtgagcaagggcgaggagctgttcaccggggtggtgcccatcctggtcgagctggacggcgacgtaaacggccacaagttcagcgtgtccggcgagggcgagggcgatgccacctacggcaagctgaccctgaagttcatctgcaccaccggcaagctgcccgtgccctggcccaccctcgtgaccaccctgacctacggcgtgcagtgcttcagccgctaccccgaccacatgaagcagcacgacttcttcaagtccgccatgcccgaaggctacgtccaggagcgcaccatcttcttcaaggacgacggcaactacaagacccgcgccgaggtgaagttcgagggcgacaccctggtgaaccgcatcgagctgaagggcatcgacttcaaggaggacggcaacatcctggggcacaagctggagtacaactacaacagccacaacgtctatatcatggccgacaagcagaagaacggcatcaaggtgaacttcaagatccgccacaacatcgaggacggcagcgtgcagctcgccgaccactaccagcagaacacccccatcggcgacggccccgtgctgctgcccgacaaccactacctgagcacccagtccgccctgagcaaagaccccaacgagaagcgcgatcacatggtcctgctggagttcgtgaccgccgccgggatcactctcggcatggacgagctgtacaaggaagaaggccctaccttgagttatggtagagatggcagatctgctacacgggagccaccatacagagtacctagggatgattgggaagaaaaaaggcactttagaagagatagttttgatgatcgtggtcctagtctcaacccagtgcttgattatgaccatggaagtcgttctcaagaatctggttattatgacagaatggattatgaagatgacagattaagagatggagaaaggtgtagggatgattctttttttggtgagacctcgcataactatcataaatttgacagtgagtatgagagaatgggacgtggtcctggccccttacaagagagatctctctttgagaaaaagagaggcgctcctccaagtagcaatattgaagacttccatggactcttaccgaagggtagggatcccaagaaaaaacgcaaggtggaagatcctaagaaaaagcggaaagtggaagacccaaaaaagaagagaaaggtagactaatgtacaagtaaagcggccgcgactctagaattcgatatcaagcttatcgataatcaacctctggattacaaaatttgtgaaagattgactggtattcttaactatgttgctccttttacgctatgtggatacgctgctttaatgcctttgtatcatgctattgcttcccgtatggctttcattttctcctccttgtataaatcctggttgctgtctctttatgaggagttgtggcccgttgtcaggcaacgtggcgtggtgtgcactgtgtttgctgacgcaacccccactggttggggcattgccaccacctgtcagctcctttccgggactttcgctttccccctccctattgccacggcggaactcatcgccgcctgccttgcccgctgctggacaggggctcggctgttgggcactgacaattccgtggtgttgtcggggaaatcatcgtcctttccttggctgctcgcctgtgttgccacctggattctgcgcgggacgtccttctgctacgtcccttcggccctcaatccagcggaccttccttcccgcggcctgctgccggctctgcggcctcttccgcgtcttcgccttcgccctcagacgagtcggatctccctttgggccgcctccccgcatcgataccgtcgacctcgagacctagaaaaacatggagcaatcacaagtagcaatacagcagctaccaatgctgattgtgcctggctagaagcacaagaggaggaggaggtgggttttccagtcacacctcaggtacctttaagaccaatgacttacaaggcagctgtagatcttagccactttttaaaagaaaaggggggactggaagggctaattcactcccaacgaagacaagatatccttgatctgtggatctaccacacacaaggctacttccctgattggcagaactacacaccagggccagggatcagatatccactgacctttggatggtgctacaagctagtaccagttgagcaagagaaggtagaagaagccaatgaaggagagaacacccgcttgttacaccctgtgagcctgcatgggatggatgacccggagagagaagtattagagtggaggtttgacagccgcctagcatttcatcacatggcccgagagctgcatccggactgtactgggtctctctggttagaccagatctgagcctgggagctctctggctaactagggaacccactgcttaagcctcaataaagcttgccttgagtgcttcaagtagtgtgtgcccgtctgttgtgtgactctggtaactagagatccctcagacccttttagtcagtgtggaaaatctctagcagggcccgtttaaacccgctgatcagcctcgactgtgccttctagttgccagccatctgttgtttgcccctcccccgtgccttccttgaccctggaaggtgccactcccactgtcctttcctaataaaatgaggaaattgcatcgcattgtctgagtaggtgtcattctattctggggggtggggtggggcaggacagcaagggggaggattgggaagacaatagcaggcatgctggggatgcggtgggctctatggcttctgaggcggaaagaaccagctggggctctagggggtatccccacgcgccctgtagcggcgcattaagcgcggcgggtgtggtggttacgcgcagcgtgaccgctacacttgccagcgccctagcgcccgctcctttcgctttcttcccttcctttctcgccacgttcgccggctttccccgtcaagctctaaatcgggggctccctttagggttccgatttagtgctttacggcacctcgaccccaaaaaacttgattagggtgatggttcacgtagtgggccatcgccctgatagacggtttttcgccctttgacgttggagtccacgttctttaatagtggactcttgttccaaactggaacaacactcaaccctatctcggtctattcttttgatttataagggattttgccgatttcggcctattggttaaaaaatgagctgatttaacaaaaatttaacgcgaattaattctgtggaatgtgtgtcagttagggtgtggaaagtccccaggctccccagcaggcagaagtatgcaaagcatgcatctcaattagtcagcaaccaggtgtggaaagtccccaggctccccagcaggcagaagtatgcaaagcatgcatctcaattagtcagcaaccatagtcccgcccctaactccgcccatcccgcccctaactccgcccagttccgcccattctccgccccatggctgactaattttttttatttatgcagaggccgaggccgcctctgcctctgagctattccagaagtagtgaggaggcttttttggaggcctaggcttttgcaaaaagctcccgggagcttgtatatccattttcggatctgatcagcacgtgttgacaattaatcatcggcatagtatatcggcatagtataatacgacaaggtgaggaactaaaccatggccaagttgaccagtgccgttccggtgctcaccgcgcgcgacgtcgccggagcggtcgagttctggaccgaccggctcgggttctcccgggacttcgtggaggacgacttcgccggtgtggtccgggacgacgtgaccctgttcatcagcgcggtccaggaccaggtggtgccggacaacaccctggcctgggtgtgggtgcgcggcctggacgagctgtacgccgagtggtcggaggtcgtgtccacgaacttccgggacgcctccgggccggccatgaccgagatcggcgagcagccgtgggggcgggagttcgccctgcgcgacccggccggcaactgcgtgcacttcgtggccgaggagcaggactgacacgtgctacgagatttcgattccaccgccgccttctatgaaaggttgggcttcggaatcgttttccgggacgccggctggatgatcctccagcgcggggatctcatgctggagttcttcgcccaccccaacttgtttattgcagcttataatggttacaaataaagcaatagcatcacaaatttcacaaataaagcatttttttcactgcattctagttgtggtttgtccaaactcatcaatgtatcttatcatgtctgtataccgtcgacctctagctagagcttggcgtaatcatggtcatagctgtttcctgtgtgaaattgttatccgctcacaattccacacaacatacgagccggaagcataaagtgtaaagcctggggtgcctaatgagtgagctaactcacattaattgcgttgcgctcactgcccgctttccagtcgggaaacctgtcgtgccagctgcattaatgaatcggccaacgcgcggggagaggcggtttgcgtattgggcgctcttccgcttcctcgctcactgactcgctgcgctcggtcgttcggctgcggcgagcggtatcagctcactcaaaggcggtaatacggttatccacagaatcaggggataacgcaggaaagaacatgtgagcaaaaggccagcaaaaggccaggaaccgtaaaaaggccgcgttgctggcgtttttccataggctccgcccccctgacgagcatcacaaaaatcgacgctcaagtcagaggtggcgaaacccgacaggactataaagataccaggcgtttccccctggaagctccctcgtgcgctctcctgttccgaccctgccgcttaccggatacctgtccgcctttctcccttcgggaagcgtggcgctttctcatagctcacgctgtaggtatctcagttcggtgtaggtcgttcgctccaagctgggctgtgtgcacgaaccccccgttcagcccgaccgctgcgccttatccggtaactatcgtcttgagtccaacccggtaagacacgacttatcgccactggcagcagccactggtaacaggattagcagagcgaggtatgtaggcggtgctacagagttcttgaagtggtggcctaactacggctacactagaagaacagtatttggtatctgcgctctgctgaagccagttaccttcggaaaaagagttggtagctcttgatccggcaaacaaaccaccgctggtagcggtggtttttttgtttgcaagcagcagattacgcgcagaaaaaaaggatctcaagaagatcctttgatcttttctacggggtctgacgctcagtggaacgaaaactcacgttaagggattttggtcatgagattatcaaaaaggatcttcacctagatccttttaaattaaaaatgaagttttaaatcaatctaaagtatatatgagtaaacttggtctgacagttaccaatgcttaatcagtgaggcacctatctcagcgatctgtctatttcgttcatccatagttgcctgactccccgtcgtgtagataactacgatacgggagggcttaccatctggccccagtgctgcaatgataccgcgagacccacgctcaccggctccagatttatcagcaataaaccagccagccggaagggccgagcgcagaagtggtcctgcaactttatccgcctccatccagtctattaattgttgccgggaagctagagtaagtagttcgccagttaatagtttgcgcaacgttgttgccattgctacaggcatcgtggtgtcacgctcgtcgtttggtatggcttcattcagctccggttcccaacgatcaaggcgagttacatgatcccccatgttgtgcaaaaaagcggttagctccttcggtcctccgatcgttgtcagaagtaagttggccgcagtgttatcactcatggttatggcagcactgcataattctcttactgtcatgccatccgtaagatgcttttctgtgactggtgagtactcaaccaagtcattctgagaatagtgtatgcggcgaccgagttgctcttgcccggcgtcaatacgggataataccgcgccacatagcagaactttaaaagtgctcatcattggaaaacgttcttcggggcgaaaactctcaaggatcttaccgctgttgagatccagttcgatgtaacccactcgtgcacccaactgatcttcagcatcttttactttcaccagcgtttctgggtgagcaaaaacaggaaggcaaaatgccgcaaaaaagggaataagggcgacacggaaatgttgaatactcatactcttcctttttcaatattattgaagcatttatcagggttattgtctcatgagcggatacatatttgaatgtatttagaaaaataaacaaataggggttccgcgcacatttccccgaaaagtgccacctgac

SEQ ID NO: 53 - protein, 405 aa, synthetic construct
MVSKGEELFTGVVPILVELDGDVNGHKFSVSGEGEGDATYGKLTLKFICTTGKLPVPWPTLVTTLTYGVQCFSRYPDHMKQHDFFKSAMPEGYVQERTIFFKDDGNYKTRAEVKFEGDTLVNRIELKGIDFKEDGNILGHKLEYNYNSHNVYIMADKQKNGIKVNFKIRHNIEDGSVQLADHYQQNTPIGDGPVLLPDNHYLSTQSALSKDPNEKRDHMVLLEFVTAAGITLGMDELYKEEGPTLSYGRDGRSATREPPYRVPRDDWEEKRHFRRDSFDDRGPSLNPVLDYDHGSRSQESGYYDRMDYEDDRLRDGERCRDDSFFGETSHNYHKFDSEYERMGRGPGPLQERSLFEKKRGAPPSSNIEDFHGLLPKGRDPKKKRKVEDPKKKRKVEDPKKKRKVD

SEQ ID NO: 54 - DNA, 5493 bp, synthetic construct
  source 1..5493: mol_type = other DNA
acgttatcgactgcacggtgcaccaatgcttctggcgtcaggcagccatcggaagctgtggtatggctgtgcaggtcgtaaatcactgcataattcgtgtcgctcaaggcgcactcccgttctggataatgttttttgcgccgacatcataacggttctggcaaatattctgaaatgagctgttgacaattaatcatcggctcgtataatgtgtggaattgtgagcggataacaatttcacacaggaaacagtattcatgtcccctatactaggttattggaaaattaagggccttgtgcaacccactcgacttcttttggaatatcttgaagaaaaatatgaagagcatttgtatgagcgcgatgaaggtgataaatggcgaaacaaaaagtttgaattgggtttggagtttcccaatcttccttattatattgatggtgatgttaaattaacacagtctatggccatcatacgttatatagctgacaagcacaacatgttgggtggttgtccaaaagagcgtgcagagatttcaatgcttgaaggagcggttttggatattagatacggtgtttcgagaattgcatatagtaaagactttgaaactctcaaagttgattttcttagcaagctacctgaaatgctgaaaatgttcgaagatcgtttatgtcataaaacatatttaaatggtgatcatgtaacccatcctgacttcatgttgtatgacgctcttgatgttgttttatacatggacccaatgtgcctggatgcgttcccaaaattagtttgttttaaaaaacgtattgaagctatcccacaaattgataagtacttgaaatccagcaagtatatagcatggcctttgcagggctggcaagccacgtttggtggtggcgaccatcctccaaaatcggatctggttccgcgtggatctggccgcaaaaaacgccgccagcgccgccgcccgccgcagggcctgtttgaagcgattgaaggctttattgaaaacggctgggaaggcatgattgatggctggtatggcaacaacacccatgatctggtgggcgatgtgcgcctggcgggcgtgcagagcgtggcgagcagccgccgccataaacgctttgcgggcgtgggcgatcgcatgaaacagattgaagataaaattgaagaaattctgagcaaaatttatccgaaaaaaaaacgcaaagtgcatattgaaaacgaaattgcgcgcattaaaaaactgattggcgaacgcggcagcggcagcgaaagcggctattatgatcgcatggattatgaagatgatcgcctgcgcgatggcgaacgctgccgcgatgatagcttttttggcgaaaccagccataactatcataaatttgatagcgaatatgaacgcatgggccgcggcagcggcagcgcgctggcgccgtatattccgccgaaaaaaaaacgcaaagtgcatcatcatcatcatcattaagaattcatcgtgactgactgacgatctgcctcgcgcgtttcggtgatgacggtgaaaacctctgacacatgcagctcccggagacggtcacagcttgtctgtaagcggatgccgggagcagacaagcccgtcagggcgcgtcagcgggtgttggcgggtgtcggggcgcagccatgacccagtcacgtagcgatagcggagtgtataattcttgaagacgaaagggcctcgtgatacgcctatttttataggttaatgtcatgataataatggtttcttagacgtcaggtggcacttttcggggaaatgtgcgcggaacccctatttgtttatttttctaaatacattcaaatatgtatccgctcatgagacaataaccctgataaatgcttcaataatattgaaaaaggaagagtatgagtattcaacatttccgtgtcgcccttattcccttttttgcggcattttgccttcctgtttttgctcacccagaaacgctggtgaaagtaaaagatgctgaagatcagttgggtgcacgagtgggttacatcgaactggatctcaacagcggtaagatccttgagagttttcgccccgaagaacgttttccaatgatgagcacttttaaagttctgctatgtggcgcggtattatcccgtgttgacgccgggcaagagcaactcggtcgccgcatacactattctcagaatgacttggttgagtactcaccagtcacagaaaagcatcttacggatggcatgacagtaagagaattatgcagtgctgccataaccatgagtgataacactgcggccaacttacttctgacaacgatcggaggaccgaaggagctaaccgcttttttgcacaacatgggggatcatgtaactcgccttgatcgttgggaaccggagctgaatgaagccataccaaacgacgagcgtgacaccacgatgcctgcagcaatggcaacaacgttgcgcaaactattaactggcgaactacttactctagcttcccggcaacaattaatagactggatggaggcggataaagttgcaggaccacttctgcgctcggcccttccggctggctggtttattgctgataaatctggagccggtgagcgtgggtctcgcggtatcattgcagcactggggccagatggtaagccctcccgtatcgtagttatctacacgacggggagtcaggcaactatggatgaacgaaatagacagatcgctgagataggtgcctcactgattaagcattggtaactgtcagaccaagtttactcatatatactttagattgatttaaaacttcatttttaatttaaaaggatctaggtgaagatcctttttgataatctcatgaccaaaatcccttaacgtgagttttcgttccactgagcgtcagaccccgtagaaaagatcaaaggatcttcttgagatcctttttttctgcgcgtaatctgctgcttgcaaacaaaaaaaccaccgctaccagcggtggtttgtttgccggatcaagagctaccaactctttttccgaaggtaactggcttcagcagagcgcagataccaaatactgtccttctagtgtagccgtagttaggccaccacttcaagaactctgtagcaccgcctacatacctcgctctgctaatcctgttaccagtggctgctgccagtggcgataagtcgtgtcttaccgggttggactcaagacgatagttaccggataaggcgcagcggtcgggctgaacggggggttcgtgcacacagcccagcttggagcgaacgacctacaccgaactgagatacctacagcgtgagctatgagaaagcgccacgcttcccgaagggagaaaggcggacaggtatccggtaagcggcagggtcggaacaggagagcgcacgagggagcttccagggggaaacgcctggtatctttatagtcctgtcgggtttcgccacctctgacttgagcgtcgatttttgtgatgctcgtcaggggggcggagcctatggaaaaacgccagcaacgcggcctttttacggttcctggccttttgctggccttttgctcacatgttctttcctgcgttatcccctgattctgtggataaccgtattaccgcctttgagtgagctgataccgctcgccgcagccgaacgaccgagcgcagcgagtcagtgagcgaggaagcggaagagcgcctgatgcggtattttctccttacgcatctgtgcggtatttcacaccgcataaattccgacaccatcgaatggtgcaaaacctttcgcggtatggcatgatagcgcccggaagagagtcaattcagggtggtgaatgtgaaaccagtaacgttatacgatgtcgcagagtatgccggtgtctcttatcagaccgtttcccgcgtggtgaaccaggccagccacgtttctgcgaaaacgcgggaaaaagtggaagcggcgatggcggagctgaattacattcccaaccgcgtggcacaacaactggcgggcaaacagtcgttgctgattggcgttgccacctccagtctggccctgcacgcgccgtcgcaaattgtcgcggcgattaaatctcgcgccgatcaactgggtgccagcgtggtggtgtcgatggtagaacgaagcggcgtcgaagcctgtaaagcggcggtgcacaatcttctcgcgcaacgcgtcagtgggctgatcattaactatccgctggatgaccaggatgccattgctgtggaagctgcctgcactaatgttccggcgttatttcttgatgtctctgaccagacacccatcaacagtattattttctcccatgaagacggtacgcgactgggcgtggagcatctggtcgcattgggtcaccagcaaatcgcgctgttagcgggcccattaagttctgtctcggcgcgtctgcgtctggctggctggcataaatatctcactcgcaatcaaattcagccgatagcggaacgggaaggcgactggagtgccatgtccggttttcaacaaaccatgcaaatgctgaatgagggcatcgttcccactgcgatgctggttgccaacgatcagatggcgctgggcgcaatgcgcgccattaccgagtccgggctgcgcgttggtgcggatatctcggtagtgggatacgacgataccgaagacagctcatgttatatcccgccgttaaccaccatcaaacaggattttcgcctgctggggcaaaccagcgtggaccgcttgctgcaactctctcagggccaggcggtgaagggcaatcagctgttgcccgtctcactggtgaaaagaaaaaccaccctggcgcccaatacgcaaaccgcctctccccgcgcgttggccgattcattaatgcagctggcacgacaggtttcccgactggaaagcgggcagtgagcgcaacgcaattaatgtgagttagctcactcattaggcaccccaggctttacactttatgcttccggctcgtatgttgtgtggaattgtgagcggataacaatttcacacaggaaacagctatgaccatgattacggattcactggccgtcgttttacaacgtcgtgactgggaaaaccctggcgttacccaacttaatcgccttgcagcacatccccctttcgccagctggcgtaatagcgaagaggcccgcaccgatcgcccttcccaacagttgcgcagcctgaatggcgaatggcgctttgcctggtttccggcaccagaagcggtgccggaaagctggctggagtgcgatcttcctgaggccgatactgtcgtcgtcccctcaaactggcagatgcacggttacgatgcgcccatctacaccaacgtaacctatcccattacggtcaatccgccgtttgttcccacggagaatccgacgggttgttactcgctcacatttaatgttgatgaaagctggctacaggaaggccagacgcgaattatttttgatggcgttggaatt

SEQ ID NO: 55 - protein, 401 aa, synthetic construct
MSPILGYWKIKGLVQPTRLLLEYLEEKYEEHLYERDEGDKWRNKKFELGLEFPNLPYYIDGDVKLTQSMAIIRYIADKHNMLGGCPKERAEISMLEGAVLDIRYGVSRIAYSKDFETLKVDFLSKLPEMLKMFEDRLCHKTYLNGDHVTHPDFMLYDALDVVLYMDPMCLDAFPKLVCFKKRIEAIPQIDKYLKSSKYIAWPLQGWQATFGGGDHPPKSDLVPRGSGRKKRRQRRRPPQGLFEAIEGFIENGWEGMIDGWYGNNTHDLVGDVRLAGVQSVASSRRHKRFAGVGDRMKQIEDKIEEILSKIYHIENEIARIKKLIGERGSGSESGYYDRMDYEDDRLRDGERCRDDSFFGETSHNYHKFDSEYERMGRGSGSALAPYIPPKKKRKVHHHHHH

SEQ ID NO: 56 - protein, 176 aa, synthetic construct
MGRKKRRQRRRPPQGLFEAIEGFIENGWEGMIDGWYGNNTHDLVGDVRLAGVQSVASSRRHKRFAGVGDRMKQIEDKIEEILSKIYHIENEIARIKKLIGERGSGSESGYYDRMDYEDDRLRDGERCRDDSFFGETSHNYHKFDSEYERMGRGSGSALAPYIPPKKKRKVHHHHHH

SEQ ID NO: 57 - DNA, 5451 bp, synthetic construct
  source 1..5451: mol_type = other DNA
acgttatcgactgcacggtgcaccaatgcttctggcgtcaggcagccatcggaagctgtggtatggctgtgcaggtcgtaaatcactgcataattcgtgtcgctcaaggcgcactcccgttctggataatgttttttgcgccgacatcataacggttctggcaaatattctgaaatgagctgttgacaattaatcatcggctcgtataatgtgtggaattgtgagcggataacaatttcacacaggaaacagtattcatgtcccctatactaggttattggaaaattaagggccttgtgcaacccactcgacttcttttggaatatcttgaagaaaaatatgaagagcatttgtatgagcgcgatgaaggtgataaatggcgaaacaaaaagtttgaattgggtttggagtttcccaatcttccttattatattgatggtgatgttaaattaacacagtctatggccatcatacgttatatagctgacaagcacaacatgttgggtggttgtccaaaagagcgtgcagagatttcaatgcttgaaggagcggttttggatattagatacggtgtttcgagaattgcatatagtaaagactttgaaactctcaaagttgattttcttagcaagctacctgaaatgctgaaaatgttcgaagatcgtttatgtcataaaacatatttaaatggtgatcatgtaacccatcctgacttcatgttgtatgacgctcttgatgttgttttatacatggacccaatgtgcctggatgcgttcccaaaattagtttgttttaaaaaacgtattgaagctatcccacaaattgataagtacttgaaatccagcaagtatatagcatggcctttgcagggctggcaagccacgtttggtggtggcgaccatcctccaaaatcggatctggttccgcgtggatctggccgcaaaaaacgccgccagcgccgccgcccgccgcagggcctgtttgaagcgattgaaggctttattgaaaacggctgggaaggcatgattgatggctggtatggcaacaacacccatgatctggtgggcgatgtgcgcctggcgggcgtgcagagcgtggcgagcagccgccgccataaacgctttgcgggcgtgggcgatcgcatgaaacagattgaagataaaattgaagaaattctgagcaaaatttatcatattgaaaacgaaattgcgcgcattaaaaaactgattggcgaacgcggcagcggcagcgaaagcggctattatgatcgcatggattatgaagatgatcgcctgcgcgatggcgaacgctgccgcgatgatagcttttttggcgaaaccagccataactatcataaatttgatagcgaatatgaacgcatgggccgcggcagcggcagcccgaaaaaaaaacgcaaagtgcatcatcatcatcatcattaagaattcatcgtgactgactgacgatctgcctcgcgcgtttcggtgatgacggtgaaaacctctgacacatgcagctcccggagacggtcacagcttgtctgtaagcggatgccgggagcagacaagcccgtcagggcgcgtcagcgggtgttggcgggtgtcggggcgcagccatgacccagtcacgtagcgatagcggagtgtataattcttgaagacgaaagggcctcgtgatacgcctatttttataggttaatgtcatgataataatggtttcttagacgtcaggtggcacttttcggggaaatgtgcgcggaacccctatttgtttatttttctaaatacattcaaatatgtatccgctcatgagacaataaccctgataaatgcttcaataatattgaaaaaggaagagtatgagtattcaacatttccgtgtcgcccttattcccttttttgcggcattttgccttcctgtttttgctcacccagaaacgctggtgaaagtaaaagatgctgaagatcagttgggtgcacgagtgggttacatcgaactggatctcaacagcggtaagatccttgagagttttcgccccgaagaacgttttccaatgatgagcacttttaaagttctgctatgtggcgcggtattatcccgtgttgacgccgggcaagagcaactcggtcgccgcatacactattctcagaatgacttggttgagtactcaccagtcacagaaaagcatcttacggatggcatgacagtaagagaattatgcagtgctgccataaccatgagtgataacactgcggccaacttacttctgacaacgatcggaggaccgaaggagctaaccgcttttttgcacaacatgggggatcatgtaactcgccttgatcgttgggaaccggagctgaatgaagccataccaaacgacgagcgtgacaccacgatgcctgcagcaatggcaacaacgttgcgcaaactattaactggcgaactacttactctagcttcccggcaacaattaatagactggatggaggcggataaagttgcaggaccacttctgcgctcggcccttccggctggctggtttattgctgataaatctggagccggtgagcgtgggtctcgcggtatcattgcagcactggggccagatggtaagccctcccgtatcgtagttatctacacgacggggagtcaggcaactatggatgaacgaaatagacagatcgctgagataggtgcctcactgattaagcattggtaactgtcagaccaagtttactcatatatactttagattgatttaaaacttcatttttaatttaaaaggatctaggtgaagatcctttttgataatctcatgaccaaaatcccttaacgtgagttttcgttccactgagcgtcagaccccgtagaaaagatcaaaggatcttcttgagatcctttttttctgcgcgtaatctgctgcttgcaaacaaaaaaaccaccgctaccagcggtggtttgtttgccggatcaagagctaccaactctttttccgaaggtaactggcttcagcagagcgcagataccaaatactgtccttctagtgtagccgtagttaggccaccacttcaagaactctgtagcaccgcctacatacctcgctctgctaatcctgttaccagtggctgctgccagtggcgataagtcgtgtcttaccgggttggactcaagacgatagttaccggataaggcgcagcggtcgggctgaacggggggttcgtgcacacagcccagcttggagcgaacgacctacaccgaactgagatacctacagcgtgagctatgagaaagcgccacgcttcccgaagggagaaaggcggacaggtatccggtaagcggcagggtcggaacaggagagcgcacgagggagcttccagggggaaacgcctggtatctttatagtcctgtcgggtttcgccacctctgacttgagcgtcgatttttgtgatgctcgtcaggggggcggagcctatggaaaaacgccagcaacgcggcctttttacggttcctggccttttgctggccttttgctcacatgttctttcctgcgttatcccctgattctgtggataaccgtattaccgcctttgagtgagctgataccgctcgccgcagccgaacgaccgagcgcagcgagtcagtgagcgaggaagcggaagagcgcctgatgcggtattttctccttacgcatctgtgcggtatttcacaccgcataaattccgacaccatcgaatggtgcaaaacctttcgcggtatggcatgatagcgcccggaagagagtcaattcagggtggtgaatgtgaaaccagtaacgttatacgatgtcgcagagtatgccggtgtctcttatcagaccgtttcccgcgtggtgaaccaggccagccacgtttctgcgaaaacgcgggaaaaagtggaagcggcgatggcggagctgaattacattcccaaccgcgtggcacaacaactggcgggcaaacagtcgttgctgattggcgttgccacctccagtctggccctgcacgcgccgtcgcaaattgtcgcggcgattaaatctcgcgccgatcaactgggtgccagcgtggtggtgtcgatggtagaacgaagcggcgtcgaagcctgtaaagcggcggtgcacaatcttctcgcgcaacgcgtcagtgggctgatcattaactatccgctggatgaccaggatgccattgctgtggaagctgcctgcactaatgttccggcgttatttcttgatgtctctgaccagacacccatcaacagtattattttctcccatgaagacggtacgcgactgggcgtggagcatctggtcgcattgggtcaccagcaaatcgcgctgttagcgggcccattaagttctgtctcggcgcgtctgcgtctggctggctggcataaatatctcactcgcaatcaaattcagccgatagcggaacgggaaggcgactggagtgccatgtccggttttcaacaaaccatgcaaatgctgaatgagggcatcgttcccactgcgatgctggttgccaacgatcagatggcgctgggcgcaatgcgcgccattaccgagtccgggctgcgcgttggtgcggatatctcggtagtgggatacgacgataccgaagacagctcatgttatatcccgccgttaaccaccatcaaacaggattttcgcctgctggggcaaaccagcgtggaccgcttgctgcaactctctcagggccaggcggtgaagggcaatcagctgttgcccgtctcactggtgaaaagaaaaaccaccctggcgcccaatacgcaaaccgcctctccccgcgcgttggccgattcattaatgcagctggcacgacaggtttcccgactggaaagcgggcagtgagcgcaacgcaattaatgtgagttagctcactcattaggcaccccaggctttacactttatgcttccggctcgtatgttgtgtggaattgtgagcggataacaatttcacacaggaaacagctatgaccatgattacggattcactggccgtcgttttacaacgtcgtgactgggaaaaccctggcgttacccaacttaatcgccttgcagcacatccccctttcgccagctggcgtaatagcgaagaggcccgcaccgatcgcccttcccaacagttgcgcagcctgaatggcgaatggcgctttgcctggtttccggcaccagaagcggtgccggaaagctggctggagtgcgatcttcctgaggccgatactgtcgtcgtcccctcaaactggcagatgcacggttacgatgcgcccatctacaccaacgtaacctatcccattacggtcaatccgccgtttgttcccacggagaatccgacgggttgttactcgctcacatttaatgttgatgaaagctggctacaggaaggccagacgcgaattatttttgatggcgttggaatt

SEQ ID NO: 58 - protein, 394 aa, synthetic construct
MSPILGYWKIKGLVQPTRLLLEYLEEKYEEHLYERDEGDKWRNKKFELGLEFPNLPYYIDGDVKLTQSMAIIRYIADKHNMLGGCPKERAEISMLEGAVLDIRYGVSRIAYSKDFETLKVDFLSKLPEMLKMFEDRLCHKTYLNGDHVTHPDFMLYDALDVVLYMDPMCLDAFPKLVCFKKRIEAIPQIDKYLKSSKYIAWPLQGWQATFGGGDHPPKSDLVPRGSGRKKRRQRRRPPQGLFEAIEGFIENGWEGMIDGWYGNNTHDLVGDVRLAGVQSVASSRRHKRFAGVGDRMKQIEDKIEEILSKIYHIENEIARIKKLIGERGSGSESGYYDRMDYEDDRLRDGERCRDDSFFGETSHNYHKFDSEYERMGRGSGSPKKKRKVHHHHHH

SEQ ID NO: 59 - protein, 169 aa, synthetic construct
MGRKKRRQRRRPPQGLFEAIEGFIENGWEGMIDGWYGNNTHDLVGDVRLAGVQSVASSRRHKRFAGVGDRMKQIEDKIEEILSKIYHIENEIARIKKLIGERGSGSESGYYDRMDYEDDRLRDGERCRDDSFFGETSHNYHKFDSEYERMGRGSGSPKKKRKVHHHHHH

SEQ ID NO: 60 - DNA, 10154 bp, synthetic construct
  source 1..10154: mol_type = other DNA
gtcgacggatcgggagatctcccgatcccctatggtgcactctcagtacaatctgctctgatgccgcatagttaagccagtatctgctccctgcttgtgtgttggaggtcgctgagtagtgcgcgagcaaaatttaagctacaacaaggcaaggcttgaccgacaattgcatgaagaatctgcttagggttaggcgttttgcgctgcttcgcgatgtacgggccagatatacgcgttgacattgattattgactagttattaatagtaatcaattacggggtcattagttcatagcccatatatggagttccgcgttacataacttacggtaaatggcccgcctggctgaccgcccaacgacccccgcccattgacgtcaataatgacgtatgttcccatagtaacgccaatagggactttccattgacgtcaatgggtggagtatttacggtaaactgcccacttggcagtacatcaagtgtatcatatgccaagtacgccccctattgacgtcaatgacggtaaatggcccgcctggcattatgcccagtacatgaccttatgggactttcctacttggcagtacatctacgtattagtcatcgctattaccatggtgatgcggttttggcagtacatcaatgggcgtggatagcggtttgactcacggggatttccaagtctccaccccattgacgtcaatgggagtttgttttggcaccaaaatcaacgggactttccaaaatgtcgtaacaactccgccccattgacgcaaatgggcggtaggcgtgtacggtgggaggtctatataagcagcgcgttttgcctgtactgggtctctctggttagaccagatctgagcctgggagctctctggctaactagggaacccactgcttaagcctcaataaagcttgccttgagtgcttcaagtagtgtgtgcccgtctgttgtgtgactctggtaactagagatccctcagacccttttagtcagtgtggaaaatctctagcagtggcgcccgaacagggacttgaaagcgaaagggaaaccagaggagctctctcgacgcaggactcggcttgctgaagcgcgcacggcaagaggcgaggggcggcgactggtgagtacgccaaaaattttgactagcggaggctagaaggagagagatgggtgcgagagcgtcagtattaagcgggggagaattagatcgcgatgggaaaaaattcggttaaggccagggggaaagaaaaaatataaattaaaacatatagtatgggcaagcagggagctagaacgattcgcagttaatcctggcctgttagaaacatcagaaggctgtagacaaatactgggacagctacaaccatcccttcagacaggatcagaagaacttagatcattatataatacagtagcaaccctctattgtgtgcatcaaaggatagagataaaagacaccaaggaagctttagacaagatagaggaagagcaaaacaaaagtaagaccaccgcacagcaagcggccgctgatcttcagacctggaggaggagatatgagggacaattggagaagtgaattatataaatataaagtagtaaaaattgaaccattaggagtagcacccaccaaggcaaagagaagagtggtgcagagagaaaaaagagcagtgggaataggagctttgttccttgggttcttgggagcagcaggaagcactatgggcgcagcgtcaatgacgctgacggtacaggccagacaattattgtctggtatagtgcagcagcagaacaatttgctgagggctattgaggcgcaacagcatctgttgcaactcacagtctggggcatcaagcagctccaggcaagaatcctggctgtggaaagatacctaaaggatcaacagctcctggggatttggggttgctctggaaaactcatttgcaccactgctgtgccttggaatgctagttggagtaataaatctctggaacagatttggaatcacacgacctggatggagtgggacagagaaattaacaattacacaagcttaatacactccttaattgaagaatcgcaaaaccagcaagaaaagaatgaacaagaattattggaattagataaatgggcaagtttgtggaattggtttaacataacaaattggctgtggtatataaaattattcataatgatagtaggaggcttggtaggtttaagaatagtttttgctgtactttctatagtgaatagagttaggcagggatattcaccattatcgtttcagacccacctcccaaccccgaggggacccgacaggcccgaaggaatagaagaagaaggtggagagagagacagagacagatccattcgattagtgaacggatcggcactgcgtgcgccaattctgcagacaaatggcagtattcatccacaattttaaaagaaaaggggggattggggggtacagtgcaggggaaagaatagtagacataatagcaacagacatacaaactaaagaattacaaaaacaaattacaaaaattcaaaattttcgggtttattacagggacagcagagatccagtttggttaattaacccgtgtcggctccagatctggcctccgcgccgggttttggcgcctcccgcgggcgcccccctcctcacggcgagcgctgccacgtcagacgaagggcgcagcgagcgtcctgatccttccgcccggacgctcaggacagcggcccgctgctcataagactcggccttagaaccccagtatcagcagaaggacattttaggacgggacttgggtgactctagggcactggttttctttccagagagcggaacaggcgaggaaaagtagtcccttctcggcgattctgcggagggatctccgtggggcggtgaacgccgatgattatataaggacgcgccgggtgtggcacagctagttccgtcgcagccgggatttgggtcgcggttcttgtttgtggatcgctgtgatcgtcacttggtgagtagcgggctgctgggctggccggggctttcgtggccgccgggccgctcggtgggacggaagcgtgtggagagaccgccaagggctgtagtctgggtccgcgagcaaggttgccctgaactgggggttggggggagcgcagcaaaatggcggctgttcccgagtcttgaatggaagacgcttgtgaggcgggctgtgaggtcgttgaaacaaggtggggggcatggtgggcggcaagaacccaaggtcttgaggccttcgctaatgcgggaaagctcttattcgggtgagatgggctggggcaccatctggggaccctgacgtgaagtttgtcactgactggagaactcggtttgtcgtctgttgcgggggcggcagttatggcggtgccgttgggcagtgcacccgtacctttgggagcgcgcgccctcgtcgtgtcgtgacgtcacccgttctgttggcttataatgcagggtggggccacctgccggtaggtgtgcggtaggcttttctccgtcgcaggacgcagggttcgggcctagggtaggctctcctgaatcgacaggcgccggacctctggtgaggggagggataagtgaggcgtcagtttctttggtcggttttatgtacctatcttcttaagtagctgaagctccggttttgaactatgcgctcggggttggcgagtgtgttttgtgaagttttttaggcaccttttgaaatgtaatcatttgggtcaatatgtaattttcagtgttagactagtaaattgtccgctaaattctggccgtttttggcttttttgttagacgaagcttgggctgcaggtcgactctagaggatccccgggtaccggtcgccaccatggtgagcaagggcgaggagctgttcaccggggtggtgcccatcctggtcgagctggacggcgacgtaaacggccacaagttcagcgtgtccggcgagggcgagggcgatgccacctacggcaagctgaccctgaagttcatctgcaccaccggcaagctgcccgtgccctggcccaccctcgtgaccaccctgacctacggcgtgcagtgcttcagccgctaccccgaccacatgaagcagcacgacttcttcaagtccgccatgcccgaaggctacgtccaggagcgcaccatcttcttcaaggacgacggcaactacaagacccgcgccgaggtgaagttcgagggcgacaccctggtgaaccgcatcgagctgaagggcatcgacttcaaggaggacggcaacatcctggggcacaagctggagtacaactacaacagccacaacgtctatatcatggccgacaagcagaagaacggcatcaaggtgaacttcaagatccgccacaacatcgaggacggcagcgtgcagctcgccgaccactaccagcagaacacccccatcggcgacggccccgtgctgctgcccgacaaccactacctgagcacccagtccgccctgagcaaagaccccaacgagaagcgcgatcacatggtcctgctggagttcgtgaccgccgccgggatcactctcggcatggacgagctgtacaagggaggaggaggaggagaaagcggctattatgatcgcatggattatgaagatgatcgcctgcgcgatggcgaacgctgccgcgatgatagcttttttggcgaaaccagccataactatcataaatttgatagcgaatatgaacgcatgggccgcggcagcggcagcccgaaaaaaaaacgcaaagtgtaatgtacaagtaagctagctcgagctagaattaattcgatatcaagcttatcgataatcaacctctggattacaaaatttgtgaaagattgactggtattcttaactatgttgctccttttacgctatgtggatacgctgctttaatgcctttgtatcatgctattgcttcccgtatggctttcattttctcctccttgtataaatcctggttgctgtctctttatgaggagttgtggcccgttgtcaggcaacgtggcgtggtgtgcactgtgtttgctgacgcaacccccactggttggggcattgccaccacctgtcagctcctttccgggactttcgctttccccctccctattgccacggcggaactcatcgccgcctgccttgcccgctgctggacaggggctcggctgttgggcactgacaattccgtggtgttgtcggggaaatcatcgtcctttccttggctgctcgcctgtgttgccacctggattctgcgcgggacgtccttctgctacgtcccttcggccctcaatccagcggaccttccttcccgcggcctgctgccggctctgcggcctcttccgcgtcttcgccttcgccctcagacgagtcggatctccctttgggccgcctccccgcatcgataccgtcgacctcgagacctagaaaaacatggagcaatcacaagtagcaatacagcagctaccaatgctgattgtgcctggctagaagcacaagaggaggaggaggtgggttttccagtcacacctcaggtacctttaagaccaatgacttacaaggcagctgtagatcttagccactttttaaaagaaaaggggggactggaagggctaattcactcccaacgaagacaagatatccttgatctgtggatctaccacacacaaggctacttccctgattggcagaactacacaccagggccagggatcagatatccactgacctttggatggtgctacaagctagtaccagttgagcaagagaaggtagaagaagccaatgaaggagagaacacccgcttgttacaccctgtgagcctgcatgggatggatgacccggagagagaagtattagagtggaggtttgacagccgcctagcatttcatcacatggcccgagagctgcatccggactgtactgggtctctctggttagaccagatctgagcctgggagctctctggctaactagggaacccactgcttaagcctcaataaagcttgccttgagtgcttcaagtagtgtgtgcccgtctgttgtgtgactctggtaactagagatccctcagacccttttagtcagtgtggaaaatctctagcagggcccgtttaaacccgctgatcagcctcgactgtgccttctagttgccagccatctgttgtttgcccctcccccgtgccttccttgaccctggaaggtgccactcccactgtcctttcctaataaaatgaggaaattgcatcgcattgtctgagtaggtgtcattctattctggggggtggggtggggcaggacagcaagggggaggattgggaagacaatagcaggcatgctggggatgcggtgggctctatggcttctgaggcggaaagaaccagctggggctctagggggtatccccacgcgccctgtagcggcgcattaagcgcggcgggtgtggtggttacgcgcagcgtgaccgctacacttgccagcgccctagcgcccgctcctttcgctttcttcccttcctttctcgccacgttcgccggctttccccgtcaagctctaaatcgggggctccctttagggttccgatttagtgctttacggcacctcgaccccaaaaaacttgattagggtgatggttcacgtagtgggccatcgccctgatagacggtttttcgccctttgacgttggagtccacgttctttaatagtggactcttgttccaaactggaacaacactcaaccctatctcggtctattcttttgatttataagggattttgccgatttcggcctattggttaaaaaatgagctgatttaacaaaaatttaacgcgaattaattctgtggaatgtgtgtcagttagggtgtggaaagtccccaggctccccagcaggcagaagtatgcaaagcatgcatctcaattagtcagcaaccaggtgtggaaagtccccaggctccccagcaggcagaagtatgcaaagcatgcatctcaattagtcagcaaccatagtcccgcccctaactccgcccatcccgcccctaactccgcccagttccgcccattctccgccccatggctgactaattttttttatttatgcagaggccgaggccgcctctgcctctgagctattccagaagtagtgaggaggcttttttggaggcctaggcttttgcaaaaagctcccgggagcttgtatatccattttcggatctgatcagcacgtgttgacaattaatcatcggcatagtatatcggcatagtataatacgacaaggtgaggaactaaaccatggccaagttgaccagtgccgttccggtgctcaccgcgcgcgacgtcgccggagcggtcgagttctggaccgaccggctcgggttctcccgggacttcgtggaggacgacttcgccggtgtggtccgggacgacgtgaccctgttcatcagcgcggtccaggaccaggtggtgccggacaacaccctggcctgggtgtgggtgcgcggcctggacgagctgtacgccgagtggtcggaggtcgtgtccacgaacttccgggacgcctccgggccggccatgaccgagatcggcgagcagccgtgggggcgggagttcgccctgcgcgacccggccggcaactgcgtgcacttcgtggccgaggagcaggactgacacgtgctacgagatttcgattccaccgccgccttctatgaaaggttgggcttcggaatcgttttccgggacgccggctggatgatcctccagcgcggggatctcatgctggagttcttcgcccaccccaacttgtttattgcagcttataatggttacaaataaagcaatagcatcacaaatttcacaaataaagcatttttttcactgcattctagttgtggtttgtccaaactcatcaatgtatcttatcatgtctgtataccgtcgacctctagctagagcttggcgtaatcatggtcatagctgtttcctgtgtgaaattgttatccgctcacaattccacacaacatacgagccggaagcataaagtgtaaagcctggggtgcctaatgagtgagctaactcacattaattgcgttgcgctcactgcccgctttccagtcgggaaacctgtcgtgccagctgcattaatgaatcggccaacgcgcggggagaggcggtttgcgtattgggcgctcttccgcttcctcgctcactgactcgctgcgctcggtcgttcggctgcggcgagcggtatcagctcactcaaaggcggtaatacggttatccacagaatcaggggataacgcaggaaagaacatgtgagcaaaaggccagcaaaaggccaggaaccgtaaaaaggccgcgttgctggcgtttttccataggctccgcccccctgacgagcatcacaaaaatcgacgctcaagtcagaggtggcgaaacccgacaggactataaagataccaggcgtttccccctggaagctccctcgtgcgctctcctgttccgaccctgccgcttaccggatacctgtccgcctttctcccttcgggaagcgtggcgctttctcatagctcacgctgtaggtatctcagttcggtgtaggtcgttcgctccaagctgggctgtgtgcacgaaccccccgttcagcccgaccgctgcgccttatccggtaactatcgtcttgagtccaacccggtaagacacgacttatcgccactggcagcagccactggtaacaggattagcagagcgaggtatgtaggcggtgctacagagttcttgaagtggtggcctaactacggctacactagaagaacagtatttggtatctgcgctctgctgaagccagttaccttcggaaaaagagttggtagctcttgatccggcaaacaaaccaccgctggtagcggtggtttttttgtttgcaagcagcagattacgcgcagaaaaaaaggatctcaagaagatcctttgatcttttctacggggtctgacgctcagtggaacgaaaactcacgttaagggattttggtcatgagattatcaaaaaggatcttcacctagatccttttaaattaaaaatgaagttttaaatcaatctaaagtatatatgagtaaacttggtctgacagttaccaatgcttaatcagtgaggcacctatctcagcgatctgtctatttcgttcatccatagttgcctgactccccgtcgtgtagataactacgatacgggagggcttaccatctggccccagtgctgcaatgataccgcgagacccacgctcaccggctccagatttatcagcaataaaccagccagccggaagggccgagcgcagaagtggtcctgcaactttatccgcctccatccagtctattaattgttgccgggaagctagagtaagtagttcgccagttaatagtttgcgcaacgttgttgccattgctacaggcatcgtggtgtcacgctcgtcgtttggtatggcttcattcagctccggttcccaacgatcaaggcgagttacatgatcccccatgttgtgcaaaaaagcggttagctccttcggtcctccgatcgttgtcagaagtaagttggccgcagtgttatcactcatggttatggcagcactgcataattctcttactgtcatgccatccgtaagatgcttttctgtgactggtgagtactcaaccaagtcattctgagaatagtgtatgcggcgaccgagttgctcttgcccggcgtcaatacgggataataccgcgccacatagcagaactttaaaagtgctcatcattggaaaacgttcttcggggcgaaaactctcaaggatcttaccgctgttgagatccagttcgatgtaacccactcgtgcacccaactgatcttcagcatcttttactttcaccagcgtttctgggtgagcaaaaacaggaaggcaaaatgccgcaaaaaagggaataagggcgacacggaaatgttgaatactcatactcttcctttttcaatattattgaagcatttatcagggttattgtctcatgagcggatacatatttgaatgtatttagaaaaataaacaaataggggttccgcgcacatttccccgaaaagtgccacctgac

SEQ ID NO: 61 - protein, 301 aa, synthetic construct
MVSKGEELFTGVVPILVELDGDVNGHKFSVSGEGEGDATYGKLTLKFICTTGKLPVPWPTLVTTLTYGVQCFSRYPDHMKQHDFFKSAMPEGYVQERTIFFKDDGNYKTRAEVKFEGDTLVNRIELKGIDFKEDGNILGHKLEYNYNSHNVYIMADKQKNGIKVNFKIRHNIEDGSVQLADHYQQNTPIGDGPVLLPDNHYLSTQSALSKDPNEKRDHMVLLEFVTAAGITLGMDELYKGGGGGESGYYDRMDYEDDRLRDGERCRDDSFFGETSHNYHKFDSEYERMGRGSGSPKKKRKV

SEQ ID NO: 62 - DNA, 8712 bp, synthetic construct
  source 1..8712: mol_type = other DNA
aaatttcacaaataaagcatttttttcactgcattctagttgtggtttgtccaaactcatcaatgtatcttatcatgtctggctctagctatcccgcccctaactccgcccagttccgcccattctccgccccatggctgactaattttttttatttatgcagaggccgaggccgcctcggcctctgagctattccagaagtagtgaggaggcttttttggaggcctaggcttttgcgtcgagacgtacccaattcgccctatagtgagtcgtattacgcgcgctcactggccgtcgttttacaacgtcgtgactgggaaaaccctggcgttacccaacttaatcgccttgcagcacatccccctttcgccagctggcgtaatagcgaagaggcccgcaccgatcgcccttcccaacagttgcgcagcctgaatggcgaatggcgcgacgcgccctgtagcggcgcattaagcgcggcgggtgtggtggttacgcgcagcgtgaccgctacacttgccagcgccctagcgcccgctcctttcgctttcttcccttcctttctcgccacgttcgccggctttccccgtcaagctctaaatcgggggctccctttagggttccgatttagtgctttacggcacctcgaccccaaaaaacttgattagggtgatggttcacgtagtgggccatcgccctgatagacggtttttcgccctttgacgttggagtccacgttctttaatagtggactcttgttccaaactggaacaacactcaaccctatctcggtctattcttttgatttataagggattttgccgatttcggcctattggttaaaaaatgagctgatttaacaaaaatttaacgcgaattttaacaaaatattaacgtttacaatttcccaggtggcacttttcggggaaatgtgcgcggaacccctatttgtttatttttctaaatacattcaaatatgtatccgctcatgagacaataaccctgataaatgcttcaataatattgaaaaaggaagagtatgagtattcaacatttccgtgtcgcccttattcccttttttgcggcattttgccttcctgtttttgctcacccagaaacgctggtgaaagtaaaagatgctgaagatcagttgggtgcacgagtgggttacatcgaactggatctcaacagcggtaagatccttgagagttttcgccccgaagaacgttttccaatgatgagcacttttaaagttctgctatgtggcgcggtattatcccgtattgacgccgggcaagagcaactcggtcgccgcatacactattctcagaatgacttggttgagtactcaccagtcacagaaaagcatcttacggatggcatgacagtaagagaattatgcagtgctgccataaccatgagtgataacactgcggccaacttacttctgacaacgatcggaggaccgaaggagctaaccgcttttttgcacaacatgggggatcatgtaactcgccttgatcgttgggaaccggagctgaatgaagccataccaaacgacgagcgtgacaccacgatgcctgtagcaatggcaacaacgttgcgcaaactattaactggcgaactacttactctagcttcccggcaacaattaatagactggatggaggcggataaagttgcaggaccacttctgcgctcggcccttccggctggctggtttattgctgataaatctggagccggtgagcgtgggtctcgcggtatcattgcagcactggggccagatggtaagccctcccgtatcgtagttatctacacgacggggagtcaggcaactatggatgaacgaaatagacagatcgctgagataggtgcctcactgattaagcattggtaactgtcagaccaagtttactcatatatactttagattgatttaaaacttcatttttaatttaaaaggatctaggtgaagatcctttttgataatctcatgaccaaaatcccttaacgtgagttttcgttccactgagcgtcagaccccgtagaaaagatcaaaggatcttcttgagatcctttttttctgcgcgtaatctgctgcttgcaaacaaaaaaaccaccgctaccagcggtggtttgtttgccggatcaagagctaccaactctttttccgaaggtaactggcttcagcagagcgcagataccaaatactgtccttctagtgtagccgtagttaggccaccacttcaagaactctgtagcaccgcctacatacctcgctctgctaatcctgttaccagtggctgctgccagtggcgataagtcgtgtcttaccgggttggactcaagacgatagttaccggataaggcgcagcggtcgggctgaacggggggttcgtgcacacagcccagcttggagcgaacgacctacaccgaactgagatacctacagcgtgagctatgagaaagcgccacgcttcccgaagggagaaaggcggacaggtatccggtaagcggcagggtcggaacaggagagcgcacgagggagcttccagggggaaacgcctggtatctttatagtcctgtcgggtttcgccacctctgacttgagcgtcgatttttgtgatgctcgtcaggggggcggagcctatggaaaaacgccagcaacgcggcctttttacggttcctggccttttgctggccttttgctcacatgttctttcctgcgttatcccctgattctgtggataaccgtattaccgcctttgagtgagctgataccgctcgccgcagccgaacgaccgagcgcagcgagtcagtgagcgaggaagcggaagagcgcccaatacgcaaaccgcctctccccgcgcgttggccgattcattaatgcagctggcacgacaggtttcccgactggaaagcgggcagtgagcgcaacgcaattaatgtgagttagctcactcattaggcaccccaggctttacactttatgcttccggctcgtatgttgtgtggaattgtgagcggataacaatttcacacaggaaacagctatgaccatgattacgccaagcgcgcaattaaccctcactaaagggaacaaaagctggagctgcaagcttggccattgcatacgttgtatccatatcataatatgtacatttatattggctcatgtccaacattaccgccatgttgacattgattattgactagttattaatagtaatcaattacggggtcattagttcatagcccatatatggagttccgcgttacataacttacggtaaatggcccgcctggctgaccgcccaacgacccccgcccattgacgtcaataatgacgtatgttcccatagtaacgccaatagggactttccattgacgtcaatgggtggagtatttacggtaaactgcccacttggcagtacatcaagtgtatcatatgccaagtacgccccctattgacgtcaatgacggtaaatggcccgcctggcattatgcccagtacatgaccttatgggactttcctacttggcagtacatctacgtattagtcatcgctattaccatggtgatgcggttttggcagtacatcaatgggcgtggatagcggtttgactcacggggatttccaagtctccaccccattgacgtcaatgggagtttgttttggcaccaaaatcaacgggactttccaaaatgtcgtaacaactccgccccattgacgcaaatgggcggtaggcgtgtacggtgggaggtctatataagcagagctcgtttagtgaaccggggtctctctggttagaccagatctgagcctgggagctctctggctaactagggaacccactgcttaagcctcaataaagcttgccttgagtgcttcaagtagtgtgtgcccgtctgttgtgtgactctggtaactagagatccctcagacccttttagtcagtgtggaaaatctctagcagtggcgcccgaacagggacctgaaagcgaaagggaaaccagagctctctcgacgcaggactcggcttgctgaagcgcgcacggcaagaggcgaggggcggcgactggtgagtacgccaaaaattttgactagcggaggctagaaggagagagatgggtgcgagagcgtcagtattaagcgggggagaattagatcgcgatgggaaaaaattcggttaaggccagggggaaagaaaaaatataaattaaaacatatagtatgggcaagcagggagctagaacgattcgcagttaatcctggcctgttagaaacatcagaaggctgtagacaaatactgggacagctacaaccatcccttcagacaggatcagaagaacttagatcattatataatacagtagcaaccctctattgtgtgcatcaaaggatagagataaaagacaccaaggaagctttagacaagatagaggaagagcaaaacaaaagtaagaccaccgcacagcaagcggccgctgatcttcagacctggaggaggagatatgagggacaattggagaagtgaattatataaatataaagtagtaaaaattgaaccattaggagtagcacccaccaaggcaaagagaagagtggtgcagagagaaaaaagagcagtgggaataggagctttgttccttgggttcttgggagcagcaggaagcactatgggcgcagcctcaatgacgctgacggtacaggccagacaattattgtctggtatagtgcagcagcagaacaatttgctgagggctattgaggcgcaacagcatctgttgcaactcacagtctggggcatcaagcagctccaggcaagaatcctggctgtggaaagatacctaaaggatcaacagctcctggggatttggggttgctctggaaaactcatttgcaccactgctgtgccttggaatgctagttggagtaataaatctctggaacagattggaatcacacgacctggatggagtgggacagagaaattaacaattacacaagcttaatacactccttaattgaagaatcgcaaaaccagcaagaaaagaatgaacaagaattattggaattagataaatgggcaagtttgtggaattggtttaacataacaaattggctgtggtatataaaattattcataatgatagtaggaggcttggtaggtttaagaatagtttttgctgtactttctatagtgaatagagttaggcagggatattcaccattatcgtttcagacccacctcccaaccccgaggggacccgacaggcccgaaggaatagaagaagaaggtggagagagagacagagacagatccattcgattagtgaacggatctcgacggtatcggttaacttttaaaagaaaaggggggattggggggtacagtgcaggggaaagaatagtagacataatagcaacagacatacaaactaaagaattacaaaaacaaattacaaaaattcaaaattttatcgatcacgagactagcctcgagaagcttgattatatactagtatgaaaccccacctgtaggtttggcaagctagctgcagtaacgccattttgcaaggcatggaaaaataccaaaccaagaatagagaagttcagatcaagggcgggtacatgaaaatagctaacgttgggccaaacaggatatctgcggtgagcagtttcggccccggcccggggccaagaacagatggtcaccgcagtttcggccccggcccgaggccaagaacagatggtccccagatatggcccaaccctcagcagtttcttaagacccatcagatgtttccaggctcccccaaggacctgaaatgaccctgcgccttatttgaattaaccaatcagcctgcttctcgcttctgttcgcgcgcttctgcttcccgagctctataaaagagctcacaacccctcactcggcttaattaaaagctttatataatcagcatcacaagtttgtacaaaaaagcaggctccatggattacaaggatgacgacgataagagcccgggcggatccgaatctggttattatgacagaatggattatgaagatgacagattaagagatggagaaaggtgtagggatgattctttttttggtgagacctcgcataactatcataaatttgacagtgagtatgagagaatgggacgtggaagcggaagcgccctggccccctacatccccgaagacccaaaaaagaagagaaaggtagactaagacccagctttcttgtacaaagtggtgatgctctagaatgcatgcatgccgtacgatcgccgcctcaggcctgagttcgaagtatacgtcgacaatcaacctctggattacaaaatttgtgaaagattgactggtattcttaactatgttgctccttttacgctatgtggatacgctgctttaatgcctttgtatcatgctattgcttcccgtatggctttcattttctcctccttgtataaatcctggttgctgtctctttatgaggagttgtggcccgttgtcaggcaacgtggcgtggtgtgcactgtgtttgctgacgcaacccccactggttggggcattgccaccacctgtcagctcctttccgggactttcgctttccccctccctattgccacggcggaactcatcgccgcctgccttgcccgctgctggacaggggctcggctgttgggcactgacaattccgtggtgttgtcggggaagctgacgtcctttccatggctgctcgcctgtgttgccacctggattctgcgcgggacgtcttctgctacgtcccttcggcctcaatcagcggacttccttcccgcggcctgctgccggctctgcggcctcttccgcgtcttcgccttcgccctcagacgagtcggatctccctttgggccgcctccccgcctggaattcctgcagcccgggggatcaaggatctgcgatcgctccggtgcccgtcagtgggcagagcgcacatcgcccacagtccccgagaagttggggggaggggtcggcaattgaacgggtgcctagagaaggtggcgcggggtaaactgggaaagtgatgtcgtgtactggctccgcctttttcccgagggtgggggagaaccgtatataagtgcagtagtcgccgtgaacgttctttttcgcaacgggtttgccgccagaacacagctgaagcttcgaggggctcgcatctctccttcacgcgcccgccgccctacctgaggccgccatccacgccggttgagtcgcgttctgccgcctcccgcctgtggtgcctcctgaactgcgtccgccgtctaggtaagtttaaagctcaggtcgagaccgggcctttgtccggcgctcccttggagcctacctagactcagccggctctccacgctttgcctgaccctgcttgctcaactctacgtctttgtttcgttttctgttctgcgccgttacagatccaagctgtgaccggcgcctacgatccaccggtcgccaccatgagcgagctgattaaggagaacatgcacatgaagctgtacatggagggcaccgtggacaaccatcacttcaagtgcacatccgagggcgaaggcaagccctacgagggcacccagaccatgagaatcaaggtggtcgagggcggccctctccccttcgccttcgacatcctggctactagcttcctctacggcagcaagaccttcatcaaccacacccagggcatccccgacttcttcaagcagtccttccctgagggcttcacatgggagagagtcaccacatacgaagacgggggcgtgctgaccgctacccaggacaccagcctccaggacggctgcctcatctacaacgtcaagatcagaggggtgaacttcacatccaacggccctgtgatgcagaagaaaacactcggctgggaggccttcaccgagacgctgtaccccgctgacggcggcctggaaggcagaaacgacatggccctgaagctcgtgggcgggagccatctgatcgcaaacatcaagaccacatatagatccaagaaacccgctaagaacctcaagatgcctggcgtctactatgtggactacagactggaaagaatcaaggaggccaacaacgagacctacgtcgagcagcacgaggtggcagtggccagatactgcgacctccctagcaaactggggcacaagcttaattaaagcggccgcgtcgagagatgggggaggctaactgagctagcttagtcatgcaccgggctgcaggaattcgagctcggtacctttaagaccaatgacttacaaggcagctgtagatcttagccactttttaaaagaaaaggggggactggaagggctaattcactcccaacgaagacaagatctgctttttgcttgtactgggtctctctggttagaccagatctgagcctgggagctctctggctaactagggaacccactgcttaagcctcaataaagcttgccttgagtgcttcaagtagtgtgtgcccgtctgttgtgtgactctggtaactagagatccctcagacccttttagtcagtgtggaaaatctctagcagtagtagttcatgtcatcttattattcagtatttataacttgcaaagaaatgaatatcagagagtgagaggaacttgtttattgcagcttataatggttacaaataaagcaatagcatcac

SEQ ID NO: 63 - protein, 81 aa, synthetic construct
MDYKDDDDKSPGGSESGYYDRMDYEDDRLRDGERCRDDSFFGETSHNYHKFDSEYERMGRGSGSALAPYIPEDPKKKRKVD

SEQ ID NO: 64 - DNA, 8685 bp, synthetic construct
  source 1..8685: mol_type = other DNA
aaatttcacaaataaagcatttttttcactgcattctagttgtggtttgtccaaactcatcaatgtatcttatcatgtctggctctagctatcccgcccctaactccgcccagttccgcccattctccgccccatggctgactaattttttttatttatgcagaggccgaggccgcctcggcctctgagctattccagaagtagtgaggaggcttttttggaggcctaggcttttgcgtcgagacgtacccaattcgccctatagtgagtcgtattacgcgcgctcactggccgtcgttttacaacgtcgtgactgggaaaaccctggcgttacccaacttaatcgccttgcagcacatccccctttcgccagctggcgtaatagcgaagaggcccgcaccgatcgcccttcccaacagttgcgcagcctgaatggcgaatggcgcgacgcgccctgtagcggcgcattaagcgcggcgggtgtggtggttacgcgcagcgtgaccgctacacttgccagcgccctagcgcccgctcctttcgctttcttcccttcctttctcgccacgttcgccggctttccccgtcaagctctaaatcgggggctccctttagggttccgatttagtgctttacggcacctcgaccccaaaaaacttgattagggtgatggttcacgtagtgggccatcgccctgatagacggtttttcgccctttgacgttggagtccacgttctttaatagtggactcttgttccaaactggaacaacactcaaccctatctcggtctattcttttgatttataagggattttgccgatttcggcctattggttaaaaaatgagctgatttaacaaaaatttaacgcgaattttaacaaaatattaacgtttacaatttcccaggtggcacttttcggggaaatgtgcgcggaacccctatttgtttatttttctaaatacattcaaatatgtatccgctcatgagacaataaccctgataaatgcttcaataatattgaaaaaggaagagtatgagtattcaacatttccgtgtcgcccttattcccttttttgcggcattttgccttcctgtttttgctcacccagaaacgctggtgaaagtaaaagatgctgaagatcagttgggtgcacgagtgggttacatcgaactggatctcaacagcggtaagatccttgagagttttcgccccgaagaacgttttccaatgatgagcacttttaaagttctgctatgtggcgcggtattatcccgtattgacgccgggcaagagcaactcggtcgccgcatacactattctcagaatgacttggttgagtactcaccagtcacagaaaagcatcttacggatggcatgacagtaagagaattatgcagtgctgccataaccatgagtgataacactgcggccaacttacttctgacaacgatcggaggaccgaaggagctaaccgcttttttgcacaacatgggggatcatgtaactcgccttgatcgttgggaaccggagctgaatgaagccataccaaacgacgagcgtgacaccacgatgcctgtagcaatggcaacaacgttgcgcaaactattaactggcgaactacttactctagcttcccggcaacaattaatagactggatggaggcggataaagttgcaggaccacttctgcgctcggcccttccggctggctggtttattgctgataaatctggagccggtgagcgtgggtctcgcggtatcattgcagcactggggccagatggtaagccctcccgtatcgtagttatctacacgacggggagtcaggcaactatggatgaacgaaatagacagatcgctgagataggtgcctcactgattaagcattggtaactgtcagaccaagtttactcatatatactttagattgatttaaaacttcatttttaatttaaaaggatctaggtgaagatcctttttgataatctcatgaccaaaatcccttaacgtgagttttcgttccactgagcgtcagaccccgtagaaaagatcaaaggatcttcttgagatcctttttttctgcgcgtaatctgctgcttgcaaacaaaaaaaccaccgctaccagcggtggtttgtttgccggatcaagagctaccaactctttttccgaaggtaactggcttcagcagagcgcagataccaaatactgtccttctagtgtagccgtagttaggccaccacttcaagaactctgtagcaccgcctacatacctcgctctgctaatcctgttaccagtggctgctgccagtggcgataagtcgtgtcttaccgggttggactcaagacgatagttaccggataaggcgcagcggtcgggctgaacggggggttcgtgcacacagcccagcttggagcgaacgacctacaccgaactgagatacctacagcgtgagctatgagaaagcgccacgcttcccgaagggagaaaggcggacaggtatccggtaagcggcagggtcggaacaggagagcgcacgagggagcttccagggggaaacgcctggtatctttatagtcctgtcgggtttcgccacctctgacttgagcgtcgatttttgtgatgctcgtcaggggggcggagcctatggaaaaacgccagcaacgcggcctttttacggttcctggccttttgctggccttttgctcacatgttctttcctgcgttatcccctgattctgtggataaccgtattaccgcctttgagtgagctgataccgctcgccgcagccgaacgaccgagcgcagcgagtcagtgagcgaggaagcggaagagcgcccaatacgcaaaccgcctctccccgcgcgttggccgattcattaatgcagctggcacgacaggtttcccgactggaaagcgggcagtgagcgcaacgcaattaatgtgagttagctcactcattaggcaccccaggctttacactttatgcttccggctcgtatgttgtgtggaattgtgagcggataacaatttcacacaggaaacagctatgaccatgattacgccaagcgcgcaattaaccctcactaaagggaacaaaagctggagctgcaagcttggccattgcatacgttgtatccatatcataatatgtacatttatattggctcatgtccaacattaccgccatgttgacattgattattgactagttattaatagtaatcaattacggggtcattagttcatagcccatatatggagttccgcgttacataacttacggtaaatggcccgcctggctgaccgcccaacgacccccgcccattgacgtcaataatgacgtatgttcccatagtaacgccaatagggactttccattgacgtcaatgggtggagtatttacggtaaactgcccacttggcagtacatcaagtgtatcatatgccaagtacgccccctattgacgtcaatgacggtaaatggcccgcctggcattatgcccagtacatgaccttatgggactttcctacttggcagtacatctacgtattagtcatcgctattaccatggtgatgcggttttggcagtacatcaatgggcgtggatagcggtttgactcacggggatttccaagtctccaccccattgacgtcaatgggagtttgttttggcaccaaaatcaacgggactttccaaaatgtcgtaacaactccgccccattgacgcaaatgggcggtaggcgtgtacggtgggaggtctatataagcagagctcgtttagtgaaccggggtctctctggttagaccagatctgagcctgggagctctctggctaactagggaacccactgcttaagcctcaataaagcttgccttgagtgcttcaagtagtgtgtgcccgtctgttgtgtgactctggtaactagagatccctcagacccttttagtcagtgtggaaaatctctagcagtggcgcccgaacagggacctgaaagcgaaagggaaaccagagctctctcgacgcaggactcggcttgctgaagcgcgcacggcaagaggcgaggggcggcgactggtgagtacgccaaaaattttgactagcggaggctagaaggagagagatgggtgcgagagcgtcagtattaagcgggggagaattagatcgcgatgggaaaaaattcggttaaggccagggggaaagaaaaaatataaattaaaacatatagtatgggcaagcagggagctagaacgattcgcagttaatcctggcctgttagaaacatcagaaggctgtagacaaatactgggacagctacaaccatcccttcagacaggatcagaagaacttagatcattatataatacagtagcaaccctctattgtgtgcatcaaaggatagagataaaagacaccaaggaagctttagacaagatagaggaagagcaaaacaaaagtaagaccaccgcacagcaagcggccgctgatcttcagacctggaggaggagatatgagggacaattggagaagtgaattatataaatataaagtagtaaaaattgaaccattaggagtagcacccaccaaggcaaagagaagagtggtgcagagagaaaaaagagcagtgggaataggagctttgttccttgggttcttgggagcagcaggaagcactatgggcgcagcctcaatgacgctgacggtacaggccagacaattattgtctggtatagtgcagcagcagaacaatttgctgagggctattgaggcgcaacagcatctgttgcaactcacagtctggggcatcaagcagctccaggcaagaatcctggctgtggaaagatacctaaaggatcaacagctcctggggatttggggttgctctggaaaactcatttgcaccactgctgtgccttggaatgctagttggagtaataaatctctggaacagattggaatcacacgacctggatggagtgggacagagaaattaacaattacacaagcttaatacactccttaattgaagaatcgcaaaaccagcaagaaaagaatgaacaagaattattggaattagataaatgggcaagtttgtggaattggtttaacataacaaattggctgtggtatataaaattattcataatgatagtaggaggcttggtaggtttaagaatagtttttgctgtactttctatagtgaatagagttaggcagggatattcaccattatcgtttcagacccacctcccaaccccgaggggacccgacaggcccgaaggaatagaagaagaaggtggagagagagacagagacagatccattcgattagtgaacggatctcgacggtatcggttaacttttaaaagaaaaggggggattggggggtacagtgcaggggaaagaatagtagacataatagcaacagacatacaaactaaagaattacaaaaacaaattacaaaaattcaaaattttatcgatcacgagactagcctcgagaagcttgattatatactagtatgaaaccccacctgtaggtttggcaagctagctgcagtaacgccattttgcaaggcatggaaaaataccaaaccaagaatagagaagttcagatcaagggcgggtacatgaaaatagctaacgttgggccaaacaggatatctgcggtgagcagtttcggccccggcccggggccaagaacagatggtcaccgcagtttcggccccggcccgaggccaagaacagatggtccccagatatggcccaaccctcagcagtttcttaagacccatcagatgtttccaggctcccccaaggacctgaaatgaccctgcgccttatttgaattaaccaatcagcctgcttctcgcttctgttcgcgcgcttctgcttcccgagctctataaaagagctcacaacccctcactcggcttaattaaaagctttatataatcagcatcacaagtttgtacaaaaaagcaggctccatggattacaaggatgacgacgataagagcccgggcggatccgaatctggttattatgacagaatggattatgaagatgacagattaagagatggagaaaggtgtagggatgattctttttttggtgagacctcgcataactatcataaatttgacagtgagtatgagagaatgggacgtggaagcggaagcccaaaaaagaagagaaaggtagactaagacccagctttcttgtacaaagtggtgatgctctagaatgcatgcatgccgtacgatcgccgcctcaggcctgagttcgaagtatacgtcgacaatcaacctctggattacaaaatttgtgaaagattgactggtattcttaactatgttgctccttttacgctatgtggatacgctgctttaatgcctttgtatcatgctattgcttcccgtatggctttcattttctcctccttgtataaatcctggttgctgtctctttatgaggagttgtggcccgttgtcaggcaacgtggcgtggtgtgcactgtgtttgctgacgcaacccccactggttggggcattgccaccacctgtcagctcctttccgggactttcgctttccccctccctattgccacggcggaactcatcgccgcctgccttgcccgctgctggacaggggctcggctgttgggcactgacaattccgtggtgttgtcggggaagctgacgtcctttccatggctgctcgcctgtgttgccacctggattctgcgcgggacgtcttctgctacgtcccttcggcctcaatcagcggacttccttcccgcggcctgctgccggctctgcggcctcttccgcgtcttcgccttcgccctcagacgagtcggatctccctttgggccgcctccccgcctggaattcctgcagcccgggggatcaaggatctgcgatcgctccggtgcccgtcagtgggcagagcgcacatcgcccacagtccccgagaagttggggggaggggtcggcaattgaacgggtgcctagagaaggtggcgcggggtaaactgggaaagtgatgtcgtgtactggctccgcctttttcccgagggtgggggagaaccgtatataagtgcagtagtcgccgtgaacgttctttttcgcaacgggtttgccgccagaacacagctgaagcttcgaggggctcgcatctctccttcacgcgcccgccgccctacctgaggccgccatccacgccggttgagtcgcgttctgccgcctcccgcctgtggtgcctcctgaactgcgtccgccgtctaggtaagtttaaagctcaggtcgagaccgggcctttgtccggcgctcccttggagcctacctagactcagccggctctccacgctttgcctgaccctgcttgctcaactctacgtctttgtttcgttttctgttctgcgccgttacagatccaagctgtgaccggcgcctacgatccaccggtcgccaccatgagcgagctgattaaggagaacatgcacatgaagctgtacatggagggcaccgtggacaaccatcacttcaagtgcacatccgagggcgaaggcaagccctacgagggcacccagaccatgagaatcaaggtggtcgagggcggccctctccccttcgccttcgacatcctggctactagcttcctctacggcagcaagaccttcatcaaccacacccagggcatccccgacttcttcaagcagtccttccctgagggcttcacatgggagagagtcaccacatacgaagacgggggcgtgctgaccgctacccaggacaccagcctccaggacggctgcctcatctacaacgtcaagatcagaggggtgaacttcacatccaacggccctgtgatgcagaagaaaacactcggctgggaggccttcaccgagacgctgtaccccgctgacggcggcctggaaggcagaaacgacatggccctgaagctcgtgggcgggagccatctgatcgcaaacatcaagaccacatatagatccaagaaacccgctaagaacctcaagatgcctggcgtctactatgtggactacagactggaaagaatcaaggaggccaacaacgagacctacgtcgagcagcacgaggtggcagtggccagatactgcgacctccctagcaaactggggcacaagcttaattaaagcggccgcgtcgagagatgggggaggctaactgagctagcttagtcatgcaccgggctgcaggaattcgagctcggtacctttaagaccaatgacttacaaggcagctgtagatcttagccactttttaaaagaaaaggggggactggaagggctaattcactcccaacgaagacaagatctgctttttgcttgtactgggtctctctggttagaccagatctgagcctgggagctctctggctaactagggaacccactgcttaagcctcaataaagcttgccttgagtgcttcaagtagtgtgtgcccgtctgttgtgtgactctggtaactagagatccctcagacccttttagtcagtgtggaaaatctctagcagtagtagttcatgtcatcttattattcagtatttataacttgcaaagaaatgaatatcagagagtgagaggaacttgtttattgcagcttataatggttacaaataaagcaatagcatcac

SEQ ID NO: 65 - protein, 72 aa, synthetic construct
MDYKDDDDKSPGGSESGYYDRMDYEDDRLRDGERCRDDSFFGETSHNYHKFDSEYERMGRGSGSPKKKRKVD

SEQ ID NO: 66 - DNA, 39 bp, synthetic construct
  source 1..39: mol_type = other DNA
catggactcttaccgaagtaatatccccatctgtgctct

SEQ ID NO: 67 - DNA, 39 bp, synthetic construct
  source 1..39: mol_type = other DNA
agagcacagatggggatattacttcggtaagagtccatg

SEQ ID NO: 68 - DNA, 39 bp, synthetic construct
  source 1..39: mol_type = other DNA
cgtcgatgccagcttctttaagaaatctacccagaatgg

SEQ ID NO: 69 - DNA, 39 bp, synthetic construct
  source 1..39: mol_type = other DNA
ccattctgggtagatttcttaaagaagctggcatcgacg

SEQ ID NO: 70 - DNA, 39 bp, synthetic construct
  source 1..39: mol_type = other DNA
gactatgtgataccttaaacagggttttactgtaagctg

SEQ ID NO: 71 - DNA, 39 bp, synthetic construct
  source 1..39: mol_type = other DNA
cagcttacagtaaaaccctgtttaaggtatcacatagtc

SEQ ID NO: 72 - DNA, 34 bp, synthetic construct
  source 1..34: mol_type = other DNA
aaaggatcctatccccatctgtgctctatatgtg

SEQ ID NO: 73 - DNA, 27 bp, synthetic construct
  source 1..27: mol_type = other DNA
aaactcgagttaagtttccttcttctg

SEQ ID NO: 74 - DNA, 52 bp, synthetic construct
  source 1..52: mol_type = other DNA
ggggacaagtttgtacaaaaaagcaggctccgccctcccgacaccctcggac

SEQ ID NO: 75 - DNA, 51 bp, synthetic construct
  source 1..51: mol_type = other DNA
ggggaccactttgtacaagaaagctgggtctaaagctcctccagcagagcc

SEQ ID NO: 76 - DNA, 52 bp, synthetic construct; identical to SEQ ID NO: 74
  source 1..52: mol_type = other DNA

SEQ ID NO: 77 - DNA, 49 bp, synthetic construct
  source 1..49: mol_type = other DNA
ggggaccactttgtacaagaaagctgggtctagacctgcgcgggcgccc

SEQ ID NO: 78 - DNA, 22 bp, synthetic construct
  source 1..22: mol_type = other DNA
atcaatggagcaagtcacagtc

SEQ ID NO: 79 - DNA, 21 bp, synthetic construct
  source 1..21: mol_type = other DNA
tgcaacatgaatggatcaccc

SEQ ID NO: 80 - DNA, 21 bp, synthetic construct
  source 1..21: mol_type = other DNA
ctcagactctcgtccgaatcc

SEQ ID NO: 81 - DNA, 22 bp, synthetic construct
  source 1..22: mol_type = other DNA
cagaagcaagatagctggcatc

SEQ ID NO: 82 - DNA, 20 bp, synthetic construct
  source 1..20: mol_type = other DNA
gagaaggcggcttacctgag

SEQ ID NO: 83 - DNA, 20 bp, synthetic construct
  source 1..20: mol_type = other DNA
cgaaggcccgctttaagaga

SEQ ID NO: 84 - DNA, 21 bp, synthetic construct
  source 1..21: mol_type = other DNA
ggcatgtggcgtcatagtaga

SEQ ID NO: 85 - DNA, 21 bp, synthetic construct
  source 1..21: mol_type = other DNA
cacggagttagctctgtgact

SEQ ID NO: 86 - DNA, 17 bp, synthetic construct
  source 1..17: mol_type = other DNA
cgtgtgctgggctcctc

SEQ ID NO: 87 - DNA, 20 bp, synthetic construct
  source 1..20: mol_type = other DNA
aaagctttgtctccgtcggt

SEQ ID NO: 88 - DNA, 20 bp, synthetic construct
  source 1..20: mol_type = other DNA
ctgcgagtacctccatggtc

SEQ ID NO: 89 - DNA, 20 bp, synthetic construct
  source 1..20: mol_type = other DNA
agagagaaagccaactccgc

SEQ ID NO: 90 - DNA, 20 bp, synthetic construct
  source 1..20: mol_type = other DNA
tgctgacgtgtttcttgtcc

SEQ ID NO: 91 - DNA, 20 bp, synthetic construct
  source 1..20: mol_type = other DNA
ttgcactgcctttcattctg

SEQ ID NO: 92 - DNA, 20 bp, synthetic construct
  source 1..20: mol_type = other DNA
ccgtgacccagttcgacaac

SEQ ID NO: 93 - DNA, 19 bp, synthetic construct
  source 1..19: mol_type = other DNA
cggcagtttagtgagcggt

SEQ ID NO: 94 - DNA, 20 bp, synthetic construct
  source 1..20: mol_type = other DNA
gcttttcgagtcagtgctgc

SEQ ID NO: 95 - DNA, 21 bp, synthetic construct
  source 1..21: mol_type = other DNA
ggggagaataactcagggttg

SEQ ID NO: 96 - DNA, 20 bp, synthetic construct
  source 1..20: mol_type = other DNA
ttgattttgcccgtacccgt

SEQ ID NO: 97 - DNA, 20 bp, synthetic construct
  source 1..20: mol_type = other DNA
ggatccggaagcattccctt

SEQ ID NO: 98 - DNA, 20 bp, synthetic construct
  source 1..20: mol_type = other DNA
gcgcaacctctcctagaaac

SEQ ID NO: 99 - DNA, 20 bp, synthetic construct
  source 1..20: mol_type = other DNA
agcagagcccggtattcttc

SEQ ID NO: 100 - DNA, 18 bp, synthetic construct
  source 1..18: mol_type = other DNA
cccaggtaccagcagacc

SEQ ID NO: 101 - DNA, 24 bp, synthetic construct
  source 1..24: mol_type = other DNA
tccaggagatgtaactctaatcca

SEQ ID NO: 102 - DNA, 20 bp, synthetic construct
  source 1..20: mol_type = other DNA
gcgttcacctcttttccaag

SEQ ID NO: 103 - DNA, 20 bp, synthetic construct
  source 1..20: mol_type = other DNA
gccatgtggatttctcgttt

SEQ ID NO: 104 - DNA, 20 bp, synthetic construct
  source 1..20: mol_type = other DNA
cccacatcaaggaactggag

SEQ ID NO: 105 - DNA, 20 bp, synthetic construct
  source 1..20: mol_type = other DNA
tgttggcatccaaggtcata

SEQ ID NO: 106 - DNA, 20 bp, synthetic construct
  source 1..20: mol_type = other DNA
acccatcactggactggtgt

SEQ ID NO: 107 - DNA, 20 bp, synthetic construct
  source 1..20: mol_type = other DNA
cacatcctcaaagagcctga

SEQ ID NO: 108 - DNA, 21 bp, synthetic construct
  source 1..21: mol_type = other DNA
ggagctgtgttttggtgacct

SEQ ID NO: 109 - DNA, 21 bp, synthetic construct
  source 1..21: mol_type = other DNA
gtagttcatgcagatggggca

SEQ ID NO: 110 - DNA, 21 bp, synthetic construct
  source 1..21: mol_type = other DNA
gggaaactggcttcaaagcta

SEQ ID NO: 111 - DNA, 19 bp, synthetic construct
  source 1..19: mol_type = other DNA
tgatggccgtgtctgcatt

SEQ ID NO: 112 - DNA, 20 bp, synthetic construct
  source 1..20: mol_type = other DNA
tggaaatcaagtggcaaaaa

SEQ ID NO: 113 - DNA, 18 bp, synthetic construct
  source 1..18: mol_type = other DNA
ctgcatgtggacgtggac

SEQ ID NO: 114 - DNA, 21 bp, synthetic construct
  source 1..21: mol_type = other DNA
agcaagagcacaacaatttgg

SEQ ID NO: 115 - DNA, 19 bp, synthetic construct
  source 1..19: mol_type = other DNA
ccctgttcgtcccgtatca

SEQ ID NO: 116 - DNA, 17 bp, synthetic construct
  source 1..17: mol_type = other DNA
gctgctgtggggtttcc

SEQ ID NO: 117 - DNA, 17 bp, synthetic construct
  source 1..17: mol_type = other DNA
aaggcaccccagtgccc

SEQ ID NO: 118 - DNA, 24 bp, synthetic construct
  source 1..24: mol_type = other DNA
cagctctgttaactcactcatctt

SEQ ID NO: 119 - DNA, 21 bp, synthetic construct
  source 1..21: mol_type = other DNA
gagctggaggtgctttttccc

SEQ ID NO: 120 - DNA, 18 bp, synthetic construct
  source 1..18: mol_type = other DNA
gcaatgcttcaacgagac

SEQ ID NO: 121 - DNA, 19 bp, synthetic construct
  source 1..19: mol_type = other DNA
tgtccttcttaaactccgc

SEQ ID NO: 122 - DNA, 24 bp, synthetic construct
  source 1..24: mol_type = other DNA
ggaagttttcagacaaacggattt

SEQ ID NO: 123 - DNA, 19 bp, synthetic construct
  source 1..19: mol_type = other DNA
accggtccaggctgatctc

SEQ ID NO: 124 - DNA, 20 bp, synthetic construct
  source 1..20: mol_type = other DNA
agctgtgcttgctctacctg

SEQ ID NO: 125 - DNA, 19 bp, synthetic construct
  source 1..19: mol_type = other DNA
gagcaacagccgcttgtcc

SEQ ID NO: 126 - DNA, 22 bp, synthetic construct
  source 1..22: mol_type = other DNA
tcgccgaccactaccagcagaa

SEQ ID NO: 127 - DNA, 23 bp, synthetic construct
  source 1..23: mol_type = other DNA
ctggaatgacttggagtacagct

SEQ ID NO: 128 - DNA, 20 bp, synthetic construct
  source 1..20: mol_type = other DNA
ggatgacgacgataagagcc

SEQ ID NO: 129 - DNA, 21 bp, synthetic construct
  source 1..21: mol_type = other DNA
tagcagacagaccaaagctgg